European Patent Specification EP 4 033 248 B1, published April 10, 2024. Title: SYSTEM AND METHOD FOR ANALYSIS OF BIOLOGICAL DATA. Applicant: MEMED DIAGNOSTICS LTD. The sequence listing filed with the application follows.

SEQUENCE LISTING (42 sequences)

SEQ ID NO: 1 - DNA, 1953 bp, Homo sapiens
acagaacccagaaaaacaactcattcgctttcatttcctcactgactataaaagaatagagaaggaagggcttcagtgaccggctgcctggctgacttacagcagtcagactctgacaggatcatggctatgatggaggtccaggggggacccagcctgggacagacctgcgtgctgatcgtgatcttcacagtgctcctgcagtctctctgtgtggctgtaacttacgtgtactttaccaacgagctgaagcagatgcaggacaagtactccaaaagtggcattgcttgtttcttaaaagaagatgacagttattgggaccccaatgacgaagagagtatgaacagcccctgctggcaagtcaagtggcaactccgtcagctcgttagaaagatgattttgagaacctctgaggaaaccatttctacagttcaagaaaagcaacaaaatatttctcccctagtgagagaaagaggtcctcagagagtagcagctcacataactgggaccagaggaagaagcaacacattgtcttctccaaactccaagaatgaaaaggctctgggccgcaaaataaactcctgggaatcatcaaggagtgggcattcattcctgagcaacttgcacttgaggaatggtgaactggtcatccatgaaaaagggttttactacatctattcccaaacatactttcgatttcaggaggaaataaaagaaaacacaaagaacgacaaacaaatggtccaatatatttacaaatacacaagttatcctgaccctatattgttgatgaaaagtgctagaaatagttgttggtctaaagatgcagaatatggactctattccatctatcaagggggaatatttgagcttaaggaaaatgacagaatttttgtttctgtaacaaatgagcacttgatagacatggaccatgaagccagtttttttggggcctttttagttggctaactgacctggaaagaaaaagcaataacctcaaagtgactattcagttttcaggatgatacactatgaagatgtttcaaaaaatctgaccaaaacaaacaaacagaaaacagaaaacaaaaaaacctctatgcaatctgagtagagcagccacaaccaaaaaattctacaacacacactgttctgaaagtgactcacttatcccaagagaatgaaattgctgaaagatctttcaggactctacctcatatcagtttgctagcagaaatctagaagactgtcagcttccaaacattaatgcaatggttaacatcttctgtctttataatctactccttgtaaagactgtagaagaaagagcaacaatccatctctcaagtagtgtatcacagtagtagcctccaggtttccttaagggacaacatccttaagtcaaaagagagaagaggcaccactaaaagatcgcagtttgcctggtgcagtggctcacacctgtaatcccaacattttgggaacccaaggtgggtagatcacgagatcaagagatcaagaccatagtgaccaacatagtgaaaccccatctctactgaaagtacaaaaattagctgggtgtgttggcacatgcctgtagtcccagctacttgagaggctgaggcaagagaattgtttgaacccgggaggcagaggttgcagtgtggtgagatcatgccactacactccagcctggcgacagagcgagacttggtttcaaaaaaaaaaaaaaaaaaaacttcagtaagtacgtgttatttttttcaataaaattctattacagtatgtcatgtttgctgtagtgctcatatttattgttgtttttgttttagtactcacttgtttcataatatcaagattactaaaaatgggggaaaagacttctaatctttttttcataatatctttgacacatattacagaagaaataaatttcttacttttaatttaatatga

SEQ ID NO: 2 - DNA, 1805 bp, Homo sapiens
acagaacccagaaaaacaactcattcgctttcatttcctcactgactataaaagaatagagaaggaagggcttcagtgaccggctgcctggctgacttacagcagtcagactctgacaggatcatggctatgatggaggtccaggggggacccagcctgggacagacctgcgtgctgatcgtgatcttcacagtgctcctgcagtctctctgtgtggctgtaacttacgtgtactttaccaacgagctgaagcagatgcaggacaagtactccaaaagtggcattgcttgtttcttaaaagaagatgacagttattgggaccccaatgacgaagagagtatgaacagcccctgctggcaagtcaagtggcaactccgtcagctcgttagaaagactccaagaatgaaaaggctctgggccgcaaaataaactcctgggaatcatcaaggagtgggcattcattcctgagcaacttgcacttgaggaatggtgaactggtcatccatgaaaaagggttttactacatctattcccaaacatactttcgatttcaggaggaaataaaagaaaacacaaagaacgacaaacaaatggtccaatatatttacaaatacacaagttatcctgaccctatattgttgatgaaaagtgctagaaatagttgttggtctaaagatgcagaatatggactctattccatctatcaagggggaatatttgagcttaaggaaaatgacagaatttttgtttctgtaacaaatgagcacttgatagacatggaccatgaagccagtttttttggggcctttttagttggctaactgacctggaaagaaaaagcaataacctcaaagtgactattcagttttcaggatgatacactatgaagatgtttcaaaaaatctgaccaaaacaaacaaacagaaaacagaaaacaaaaaaacctctatgcaatctgagtagagcagccacaaccaaaaaattctacaacacacactgttctgaaagtgactcacttatcccaagagaatgaaattgctgaaagatctttcaggactctacctcatatcagtttgctagcagaaatctagaagactgtcagcttccaaacattaatgcaatggttaacatcttctgtctttataatctactccttgtaaagactgtagaagaaagagcaacaatccatctctcaagtagtgtatcacagtagtagcctccaggtttccttaagggacaacatccttaagtcaaaagagagaagaggcaccactaaaagatcgcagtttgcctggtgcagtggctcacacctgtaatcccaacattttgggaacccaaggtgggtagatcacgagatcaagagatcaagaccatagtgaccaacatagtgaaaccccatctctactgaaagtacaaaaattagctgggtgtgttggcacatgcctgtagtcccagctacttgagaggctgaggcaagagaattgtttgaacccgggaggcagaggttgcagtgtggtgagatcatgccactacactccagcctggcgacagagcgagacttggtttcaaaaaaaaaaaaaaaaaaaacttcagtaagtacgtgttatttttttcaataaaattctattacagtatgtcatgtttgctgtagtgctcatatttattgttgtttttgttttagtactcacttgtttcataatatcaagattactaaaaatgggggaaaagacttctaatctttttttcataatatctttgacacatattacagaagaaataaatttcttacttttaatttaatatga

SEQ ID NO: 3 - DNA, 1334 bp, Homo sapiens
atttcctcactgactataaaagaatagagaaggaagggcttcagtgaccggctgcctggctgacttacagcagtcagactctgacaggatcatggctatgatggaggtccaggggggacccagcctgggacagacctgcgtgctgatcgtgatcttcacagtgctcctgcagtctctctgtgtggctgtaacttacgtgtactttaccaacgagctgaagcagtttgcagaaaatgattgccagagactaatgtctgggcagcagacagggtcattgctgccatcttgaagtctaccttgctgagtctaccctgctgacctcaagccccatcaaggactggttgaccctggcctagacaaccaccgtgtttgtaacagcaccaagagcagtcaccatggaaatccacttttcagaaccaagggcttctggagctgaagaacaggcacccagtgcaagagctttcttttcagaggcacgcaaatgaaaataatccccacacgctaccttctgcccccaatgcccaagtgtggttagttagagaatatagcctcagcctatgatatgctgcaggaaactcatattttgaagtggaaaggatgggaggaggcgggggagacgtatcgtattaattatcattcttggaataaccacagcacctcacgtcaacccgccatgtgtctagtcaccagcattggccaagttctataggagaaactaccaaaattcatgatgcaagaaacatgtgagggtggagagagtgactggggcttcctctctggatttctattgttcagaaatcaatatttatgcataaaaaggtctagaaagagaaacaccaaaatgacaatgtgatctctagatggtatgattatgggtactttttttcctttttatttttctatattttacaaattttctacagggaatgttataaaaatatccatgctatccatgtataattttcatacagatttaaagaacacagcatttttatatagtcttatgagaaaacaaccatactcaaaattatgcacacacacagtctgatctcacccctgtaaacaagagatatcatccaaaggttaagtaggaggtgagaatatagctgctattagtggttgttttgttttgtttttgtgatttacttatttagtttttggagggttttttttttcttttagaaaagtgttctttacttttccatgcttccctgcttgcctgtgtatcctgaatgtatccaggctttataaactcctgggtaataatgtagctacattaacttgttaacctcccatccacttatacccaggaccttactcaattttccaggttc

SEQ ID NO: 4 - protein, 281 aa, Homo sapiens [sequence omitted]

SEQ ID NO: 5 - protein, 101 aa, Homo sapiens
MAMMEVQGGPSLGQTCVLIVIFTVLLQSLCVAVTYVYFTNELKQMQDKYSKSGIACFLKEDDSYWDPNDEESMNSPCWQVKWQLRQLVRKTPRMKRLWAAK

SEQ ID NO: 6 - protein, 65 aa, Homo sapiens
MAMMEVQGGPSLGQTCVLIVIFTVLLQSLCVAVTYVYFTNELKQFAENDCQRLMSGQQTGSLLPS

SEQ ID NO: 7 - protein, 223 aa, Homo sapiens
QDHGYDGGPGGTQPGTDLRADRDLHSAPAVSLCGCNLRVLYQRAEAEKQQNISPLVRERGPQRVAAHITGTRGRSNTLSSPNSKNEKALGRKINSWESSRSGHSFLSNLHLRNGELVIHEKGFYYIYSQTYFRFQEEIKENTKNDKQMVQYIYKYTSYPDPILLMKSARNSCWSKDAEYGLYSIYQGGIFELKENDRIFVSVTNEHLIDMDHEASFFGAFLVG

SEQ ID NO: 8 - protein, 178 aa, Homo sapiens
KEKQQNISPLVRERGPQRVAAHITGTRGRSNTLSSPNSKNEKALGRKINSWESSRSGHSFLSNLHLRNGELVIHEKGFYYIYSQTYFRFQEEIKENTKNDKQMVQYIYKYTSYPDPILLMKSARNSCWSKDAEYGLYSIYQGGIFELKENDRIFVSVTNEHLIDMDHEASFFGAFLVG

SEQ ID NO: 9 - DNA, 2421 bp, Homo sapiens
caccctcatgagccccgggtacgtttaactattgagggccaggaaattgccttcctcctggacactggcgcagccttctcagggttaatctcctgtcctggatgactgtcttcaaggtccgttaccacccgaggaatcctgggacagcctataaccaggtatttctcccacatcctcagttgtaattgagagactttaatcttttcacatgccttttttgttattcctgaaagtcccacacccttattaaggagggatatattagccaaggctggagctattatctacatgaatatggggaaaaagttacccatttgctgtcccctacttgaggagggaatcaaccctgaagtctgggcattggaaggacaatttggaagggcaaaaaatgcctgcccagtccaaatcaggttaaaagatcccaccacttttccgtatcaaaggcaatatcccttaaggcctgaagctcataaaggattatagaatattgttaaacatttaaaagctcaaggcttagtgaggaaatgcagcagtccctgcaacaccccagttctaggagtacaaaaaccaaacagtcagtggagactagtgcaagatcttagactcattaatgaggcagtaattcctctatatccagttgtacccaacccctataccctgctctctcaaataccaggggaagcagaatggttcacggttctggacctcaaggatgccttcttctttattcccctgcactctgactcccagtttctctttgcttttgaggatcccacagaccacacgtcccaacttacacagatggtcttgccccaagggtttagggatagccctcatctgtttggtcaggcactggcccaagatctataggccacttctcaagtccaggcactctggtccttcaatatgtggatgatttacttttggctaccagtttggaagcctcgtgccagcaggctactctggatctcttgaactttctggctaatcaagggtacaaggtgtctaggtcgaaggcccagctttgcctacagcaggttaaatatctaagcctaatcttagccaaagggaccagggccctcagcaaggaatgaatacagcctatactggcttatcctcaccctaagacattaaaacagttgcggggattccttggaattactggcttttgctgactatggatctccagatacagcgagacagccaggcccctctatactctaatcaaggaaacccagagggcaaatactcatctagtcgaaagggaaccagaggcagaaacagccttcaaaagcttaaagcaggctctagtacaagctccagctttaagccttcccacaggacagaacttctctttatacatcacagagagagccaagatagctcttggagtccttagactcgtgggacaaccccacaaccagtggcatacctaagtaaggaaattgatgtagtagcaaaaggctggcctcactgtttaagggtagttgcagcagcggccgtcttagcgtcagaggctatcagaataatacaaggaaaggatctcactgtctggactactcatgatgtaaatggcatactaggtgccaaaggaagtttatggctatcagacaaccgcctcttagatgccaggcactactccttgagggactggtgcttaaaatatgcacgtgcgtggccctcaaccctgccacttttctcccagaggatggggaaccaattgagcatgactgccaacaaattatagtccagacttatgccgcccgagatgatctcttagaagtccccttaactaatcctgaccttaacctatataccgacggaagttcatttgtggagaatgggatacgaagggcaggttacgccatagtgatgtaaccacacttgaaagcaagcctcttcccccagggaccagtgcccagttagcagaactagtggcacttacccgagccttagaactgggaaagggaaaaagaataaatgtgtatacagataacaagtatgcttatctaatcctacatgcccatgctgcaatatggaaagaatgggagttcctaacctctgggaacccccgctggatgccacagggaagttatggagttattgcacatggtgcaggaacccaaagaggtgggagtcttacactaccaaggccatcaaaatgggaaggagaggggagaacagcagcataagcggctggcagaggtagggaaagaccagcaagaaggaaagagagaaagagaaagtcagagaaagagacagagagaggaagagacagagagacagaacgttaaagagggtgtcagaaacagagacaaacaaaaggagtcagaaagaaggacagacacagaaagtcaaagagagagttaaaaagagaggaagagacaaagaagtcgaagagagaaagagagagatggaagt

SEQ ID NO: 10 - DNA, 2421 bp, Homo sapiens
ctttgcagataaatatggcacactagccccacgttttctgagacattcctcaattgcttagacatattctgagcctacagcagaggaacctccagtctcagcaccatgaatcaaactgccattctgatttgctgccttatctttctgactctaagtggcattcaaggtaaggaacatcaaaggatacttaatttgtaaaatgagaaataggaataggtataaattctaaaaatacagaaataatgtatttgtaaaagtttcactgcatgcttataaataagagggaaataaatagagattccctcagatcataaaacttatatgaattgaagtgagagaaacaaatagaataagagaaagagaaggaaaaagggaaggaggacagaagagatggggaagagggaggatagagagagaaaatgtgagggaatgcggacagagatgagatacagatacttccttacctaactaagctcaatgaaccacatgaactgtgcttaagggtttgactttataatcaacaagctgcaattcttttcttccagataatcaactctttaatcatttacagttgtgttatgatgtgatccattcctcctcagattaagtgactatttgctgatatggggatataggttctgctaaataccaccagtctacattaaatgcctaaaatgaacactgtgctaaccttctctgctgttcctcttttcctacaggagtacctctctctagaactgtacgctgtacctgcatcagcattagtaatcaacctgttaatccaaggtctttagaaaaacttgaaattattcctgcaagccaattttgtccacgtgttgagatcatgtgagtgaaatcccatctgattatcacttccctggttgtaattatatactgtattaaatatgtaatgataataaaaaaagatcagtaaagggtttgtgatgattctaaaactaatgtacagcaaacaaaaacatgcagagtgaaacttaaatgtctgacttcagaactgcgtatgccatctgttttattgacccaacacagttttaaatattttcatccctatttatttctacagtgctacaatgaaaaagaagggtgagaagagatgtctgaatccagaatcgaaggccatcaagaatttactgaaagcagttagcaaggaaaggtaggtttgctgttgcctgcagaagaattgctctttaggaaacggcaatcttgggagtcagaaatacttgcattgtggtttgctgtgcaatcgctggtttaaaagtatgttaccaccacgccctcccctacctccatttatttaaatgctgaggcaccatcttgtgtgataagtatcagaagttaccctgattaccagtcaaccttgaagtacagctataactatctaagcaaaactgacaacattttccccaagtctttcatggttgaaaaaagcaacccctataatccataatgaatgcatagcagcaggaaagctcagttatctattctatgaactcggtactttccaaacacaacccaatctgaagccagagtcagactatcacacttttatatcccctttctcttcttacaggtctaaaagatctccttaaaaccagaggggagcaaaatcgatgcagtgcttccaaggatggaccacacagaggctgcctctcccatcacttccctacatggagtatatgtcaagccataattgttcttagtttgcagttacactaaaaggtgaccaatgatggtcaccaaatcagctgctactactcctgtaggaaggttaatgttcatcatcctaagctattcagtaataactctaccctggcactataatgtaagctctactgaggtgctatgttcttagtggatgttctgaccctgcttcaaatatttccctcacctttcccatcttccaagggtactaaggaatctttctgctttggggtttatcagaattctcagaatctcaaataactaaaaggtatgcaatcaaatctgctttttaaagaatgctctttacttcatggacttccactgccatcctcccaaggggcccaaattctttcagtggctacctacatacaattccaaacacatacaggaaggtagaaatatctgaaaatgtatgtgtaagtattcttatttaatgaaagactgtacaaagtagaagtcttagatgtatatatttcctatattgttttcagtgtacatggaataacatgtaattaagtactatgtatcaatgagtaacaggaaaattttaaaaatacagatagatatatgctctgcatgttacataagataaatgtgctgaatggttttcaaaataaaaatgaggtactctcctggaaatattaagaaagactatctaaatgttgaaagatcaaaaggttaataaagtaattataactaaga

SEQ ID NO: 11 - DNA, 2421 bp, Homo sapiens
agatgacttttttctatttatatttaataagatgatgaacccttcttgcattcccgaaataaacctcaactgttacagtgttttattcttttaatatgtacgaagtacatgttaagcaagttatttcctaagcagccccacaaactgggcactactaccatcctgctctgcccctccctcactctacttcagccacttcagccacaatggcctctcctcactgcccctctgatgcaccaagcttgttctcacctcaggaatgtgcaacacctgccagacttgctgttccccggagcctccatccccagatatcctcatatatcatcctcctcttcatttgtgtctctgcttacatatgacctatttacagaagcctttcctgtctaccccccatgaaatagaaatcgcattccaatcttgtctctaccccaatgctgtttcattttgtctgtagcaattgtcatcatctcatatatattcacatgtggaaaatacacaaaatgtttaacttcttttaatttacattccatttccccatgaattgaagctccatgacagcggagatttttctctgctttccctgttgctcacttcccagcaccaagagcaggcctggcacatgggaagtacttactatttattgaatggatgaatgaacaaatgaatgaatggatacttattttacacataagaaaactgaagcttatagaaattaagtaactaaaatcacacagaagcacagctgaaactaaaacctacgtctaactttcaattcctgacccttaaccattaaaacaaatgacaggtgactttaggccactgaaaatgctcatataatcttatgaattctaaagcacaagttaatcacaccattgattgaaagtctgaggaatactgtatagacaagcccctgtacaaggtaagcaaaagaatcagaggatggcctccaaagaattccctggacattatgggaattacattgttagccttcctactgatacccataagcctcacagcaagcatcatgaagctgtgaccttcatctgcacatgcccttgtatacccaaaagataaaactggatgcttcagggccgaatggccaataaacacgtgtttattactggcatgggcagacacacatactgaaagtaccatttcccagcggactagccatattatgatcagtacagacactaaagatttagctttgaaaaaactatttgctcttccaaagctgaagaatcttctgtgatttcaacaggcaagttacagtcaggtattcttaatgttcttttcctcctctctcactgggatactttctttccttcagacaacgtcaagcgaaaaacaaaatttcacaaatctccatttctgacactaaacagtacagtatctttattttttttataatttaatcaaaccctgtattttagaactgtggggctgatccaacattgcaatgtgtcacatttaattccatcaatgtaaagcataatgagcaaagattaaggtagtgaggcataactaaatgttttgaacctgtgaatttcaaaagcaaggcccatttgtgttattttctaaatagtaaataaaatcattttccaacatttcactatcaaattacagtaatttttccaccagtacacacttgaggaaagccacaaaaagacttttccaacagttcattctgttattgctcataaccttctaaatacttctcctcattggcttctattcaaaggtaaatggaaagcagtaaaatttatggaaaatatattcaactgcttaaaatacatcaaccaaaaaaaagattttagagctgtattatgagttgtgaaattgcattgccttcacttacctttcagtttcactggtaggtaacaaaactgacagactggtcaagttccaaaacatcccctatatagagcctgactcttccatctcaaattctcaccttggtcaaggccagagtaaacacctgtccttcacatttttacacaacatcactttgtatgctacaaatataagctttcataccagggaggaagcaaattccaggacactggaaacatttctgctctcttaaaccagtctgttgattgttcccttgactttctcagctgtcaggatagtgaaaggaggaaaactgcaaaactgtaaagtataacctgataagtttgccctttaagcttttcacacagagagaggtaaaataaaactcaagtctaaggtttaaaattgagctatgaatattatattctagcactagacaaaaatgttgcaagattttaataaaataagattattaaaatcaatttttacatttcatgggccaaggagagacatcaaagaatgtttaactaacattttaaagatactatactttataaagttaagaagaaaaatgacaactgcaccagt

SEQ ID NO: 12 - DNA, 1227 bp, Homo sapiens
ctttgcagataaatatggcacactagccccacgttttctgagacattcctcaattgcttagacatattctgagcctacagcagaggaacctccagtctcagcaccatgaatcaaactgccattctgatttgctgccttatctttctgactctaagtggcattcaaggagtacctctctctagaactgtacgctgtacctgcatcagcattagtaatcaacctgttaatccaaggtctttagaaaaacttgaaattattcctgcaagccaattttgtccacgtgttgagatcattgctacaatgaaaaagaagggtgagaagagatgtctgaatccagaatcgaaggccatcaagaatttactgaaagcagttagcaaggaaaggtctaaaagatctccttaaaaccagaggggagcaaaatcgatgcagtgcttccaaggatggaccacacagaggctgcctctcccatcacttccctacatggagtatatgtcaagccataattgttcttagtttgcagttacactaaaaggtgaccaatgatggtcaccaaatcagctgctactactcctgtaggaaggttaatgttcatcatcctaagctattcagtaataactctaccctggcactataatgtaagctctactgaggtgctatgttcttagtggatgttctgaccctgcttcaaatatttccctcacctttcccatcttccaagggtactaaggaatctttctgctttggggtttatcagaattctcagaatctcaaataactaaaaggtatgcaatcaaatctgctttttaaagaatgctctttacttcatggacttccactgccatcctcccaaggggcccaaattctttcagtggctacctacatacaattccaaacacatacaggaaggtagaaatatctgaaaatgtatgtgtaagtattcttatttaatgaaagactgtacaaagtagaagtcttagatgtatatatttcctatattgttttcagtgtacatggaataacatgtaattaagtactatgtatcaatgagtaacaggaaaattttaaaaatacagatagatatatgctctgcatgttacataagataaatgtgctgaatggttttcaaaataaaaatgaggtactctcctggaaatattaagaaagactatctaaatgttgaaagatcaaaaggttaataaagtaattataactaagaaaaaaaaaaaa

SEQ ID NO: 13 - protein, 98 aa, Homo sapiens
MNQTAILICCLIFLTLSGIQGVPLSRTVRCTCISISNQPVNPRSLEKLEIIPASQFCPRVEIIATMKKKGEKRCLNPESKAIKNLLKAVSKERSKRSP

SEQ ID NO: 14 - DNA, 2301 bp, Homo sapiens
aaggcaagagatctaggacttctagcccctgaactttcagccgaatacatcttttccaaaggagtgaattcaggcccttgtatcactggcagcaggacgtgaccatggagaagctgttgtgtttcttggtcttgaccagcctctctcatgcttttggccagacaggtaagggccaccccaggctatgggagagatttgatctgaggtatgggggtggggtctaagactgcatgaacagtctcaaaaaaaaaaaaaaaagactgtatgaacagaacagtggagcatccttcatggtgtgtgtgtgtgtgtgtgtgtgtgtgtgtgtgtgtgtggtgtgtaactggagaaggggtcagtctgtttctcaatcttaaattctatacgtaagtgaggggatagatctgtgtgatctgagaaacctctcacatttgcttgtttttctggctcacagacatgtcgaggaaggcttttgtgtttcccaaagagtcggatacttcctatgtatccctcaaagcaccgttaacgaagcctctcaaagccttcactgtgtgcctccacttctacacggaactgtcctcgacccgtgggtacagtattttctcgtatgccaccaagagacaagacaatgagattctcatattttggtctaaggatataggatacagttttacagtgggtgggtctgaaatattattcgaggttcctgaagtcacagtagctccagtacacatttgtacaagctgggagtccgcctcagggatcgtggagttctgggtagatgggaagcccagggtgaggaagagtctgaagaagggatacactgtgggggcagaagcaagcatcatcttggggcaggagcaggattccttcggtgggaactttgaaggaagccagtccctggtgggagacattggaaatgtgaacatgtgggactttgtgctgtcaccagatgagattaacaccatctatcttggcgggcccttcagtcctaatgtcctgaactggcgggcactgaagtatgaagtgcaaggcgaagtgttcaccaaaccccagctgtggccctgaggcccagctgtgggtcctgaaggtacctcccggttttttacaccgcatgggccccacgtctctgtctctggtacctcccgcttttttacactgcatggttcccacgtctctgtctctgggcctttgttcccctatatgcattgcaggcctgctccaccctcctcagcgcctgagaatggaggtaaagtgtctggtctgggagctcgttaactatgctgggaaacggtccaaaagaatcagaatttgaggtgttttgttttcatttttatttcaagttggacagatcttggagataatttcttacctcacatagatgagaaaactaacacccagaaaggagaaatgatgttataaaaaactcataaggcaagagctgagaaggaagcgctgatcttctatttaattccccacccatgacccccagaaagcaggagggcattgcccacattcacagggctcttcagtctcagaatcaggacactggccaggtgtctggtttgggtccagagtgctcatcatcatgtcatagaactgctgggcccaggtctcctgaaatgggaagcccagcaataccacgcagtccctccactttctcaaagcacactggaaaggccattagaattgccccagcagagcagatctgctttttttccagagcaaaatgaagcactaggtataaatatgttgttactgccaagaacttaaatgactggtttttgtttgcttgcagtgctttcttaattttatggctcttctgggaaactcctccccttttccacacgaaccttgtggggctgtgaattctttcttcatccccgcattcccaatatacccaggccacaagagtggacgtgaaccacagggtgtcctgtcagaggagcccatctcccatctccccagctccctatctggaggatagttggatagttacgtgttcctagcaggaccaactacagtcttcccaaggattgagttatggactttgggagtgagacatcttcttgctgctggatttccaagctgagaggacgtgaacctgggaccaccagtagccatcttgtttgccacatggagagagactgtgaggacagaagccaaactggaagtggaggagccaagggattgacaaacaacagagccttgaccacgtggagtctctgaatcagccttgtctggaaccagatctacacctggactgcccaggtctataagccaataaagcccctgtttacttga

SEQ ID NO: 15 - DNA, 2301 bp, Homo sapiens
aggaattgaactcagctctgccccaagcggacctaatagacatctacagaactctccaccccaaatcaacagaatatacatttttttcagcaccacaccacacctattccaaaattgatcacatagttggcagtaaagctctcctcagcaaatgtaaaggaacagaaattataacaaactatctctcagaccacagtgcaatcaaattagaactcagaattaagaatctcactcaaaaccgcacaactacatggaaactgaacaacctgcttctgaatgactactgggtacataatgaaatgaaggcagaaataaagatgttctttgaaatgaacaagaacaaacacacaacataccagaatctctgggacgcattcaaagcagtgtgtagagggaaatttatagcactaaatgcccacaagagaaagcaggaaacatccaaaattgacatcctaacatcacagttaaaagaactagaaaagcaagagcaaacacattcaaaagctagcagaaggcaagagataactaaaatcagagcagaactgaaggaaatagagacacaaaaacccttcaaaaaattaatgaatccaggagctggttttttgaaaggatcaacaaaatagatagaccactagcaagactaataaagaaaaaaagagagaagaatcaaatagacacaataaaaaaatgataaaggggatatcaccaccgatcccacggaaatacaaactaccatcagagaatactacaaacacctctacgcaaataaactagaaaatcaagaagaaatggataaattcctcgacacatacactctcccaagactaaaccaggaagaagttgaatctctgaatagaccaataacaggatatgaaattgtggcaataatcaataccttaccaacaaaaaagagtccaggaccagatggattcacagccgaattctaccagaggtacaaggaggaactggtaccattccttctgaaactattccaatcaatagaaaaagagggaatcctccctaactcattttatgaggccagcatcattctgataccaaagccgggcagagacacaaccaaaaaagagaattttagaccaatcaatatccttgatgaacattgatgcaaaaatcctcaataaaatactgccaaaccaaatccagcagcacatcaaaaagcttatccaccatgatcaagtgggcttcatccctgggatgcaaggctggttcaatatacgcaaatcaataaatgtaatccagcatataaacagagccaaagacaaaaaccacatgattatctcaatagatgcagaaaagacctttgacaaaattcaacaacccttcatgctcaaaactctcaataaattaggtattgatgggacgtatttcaaaataataagagctatctatgacaaacccacagccaatatcatactgaatgggcaaaaactggaagtattcactttgaaaactggcacaagacagggatgccctctctcaccactcctattcaacatagtgttggaagttctggccagggcaattaggcaggagaaggaaataaagggtattcaattaggaaaagaggaagtcaaattgtccctgtttgcagacgacatgattgtatatctagaaaaccccattgtctcagcccaaaatctccttaagcagataagcaacttcagcaaaatctcaggatacaaaatcaatgtacaaaaatcacaagcattcttatacaccaacaacagacaaacagagagccaaatcatgagtgaaatcccattcacaattgctttaaagagaataaaatacctaggaatccaacttacaagggatgtgaaggacctcttcaaggagaactacaaaccactgctcaatgaaataaaagaggataaaaacaaatggaagaacattccatgctcatgggtaggaagaatcaatatcatgaaaatggccatactgcccaaggtaatttacagattcaatgccatccccatcaagctaccaatgcctttcttcacagaattggaaaaaactatttttagttcatatggaaccaaaaaagagcccgcattgccaagtcaatcctaagccaaaagaacaaagctggaggcatcacactacctgacttcaaactatactacaaggctacagtaaccaaaacagcatggtactggaaccaaaacagagatatagatcaatggaacagaacagagccctcaaaattaatgccacatatctacaactatctgatctttgacaaacctgagaaaaaccagcaatggggaaaggattccccat

SEQ ID NO: 16 - DNA, 2024 bp, Homo sapiens
aaggcaagagatctaggacttctagcccctgaactttcagccgaatacatcttttccaaaggagtgaattcaggcccttgtatcactggcagcaggacgtgaccatggagaagctgttgtgtttcttggtcttgaccagcctctctcatgcttttggccagacagacatgtcgaggaaggcttttgtgtttcccaaagagtcggatacttcctatgtatccctcaaagcaccgttaacgaagcctctcaaagccttcactgtgtgcctccacttctacacggaactgtcctcgacccgtgggtacagtattttctcgtatgccaccaagagacaagacaatgagattctcatattttggtctaaggatataggatacagttttacagtgggtgggtctgaaatattattcgaggttcctgaagtcacagtagctccagtacacatttgtacaagctgggagtccgcctcagggatcgtggagttctgggtagatgggaagcccagggtgaggaagagtctgaagaagggatacactgtgggggcagaagcaagcatcatcttggggcaggagcaggattccttcggtgggaactttgaaggaagccagtccctggtgggagacattggaaatgtgaacatgtgggactttgtgctgtcaccagatgagattaacaccatctatcttggcgggcccttcagtcctaatgtcctgaactggcgggcactgaagtatgaagtgcaaggcgaagtgttcaccaaaccccagctgtggccctgaggcccagctgtgggtcctgaaggtacctcccggttttttacaccgcatgggccccacgtctctgtctctggtacctcccgcttttttacactgcatggttcccacgtctctgtctctgggcctttgttcccctatatgcattgcaggcctgctccaccctcctcagcgcctgagaatggaggtaaagtgtctggtctgggagctcgttaactatgctgggaaacggtccaaaagaatcagaatttgaggtgttttgttttcatttttatttcaagttggacagatcttggagataatttcttacctcacatagatgagaaaactaacacccagaaaggagaaatgatgttataaaaaactcataaggcaagagctgagaaggaagcgctgatcttctatttaattccccacccatgacccccagaaagcaggagggcattgcccacattcacagggctcttcagtctcagaatcaggacactggccaggtgtctggtttgggtccagagtgctcatcatcatgtcatagaactgctgggcccaggtctcctgaaatgggaagcccagcaataccacgcagtccctccactttctcaaagcacactggaaaggccattagaattgccccagcagagcagatctgctttttttccagagcaaaatgaagcactaggtataaatatgttgttactgccaagaacttaaatgactggtttttgtttgcttgcagtgctttcttaattttatggctcttctgggaaactcctccccttttccacacgaaccttgtggggctgtgaattctttcttcatccccgcattcccaatatacccaggccacaagagtggacgtgaaccacagggtgtcctgtcagaggagcccatctcccatctccccagctccctatctggaggatagttggatagttacgtgttcctagcaggaccaactacagtcttcccaaggattgagttatggactttgggagtgagacatcttcttgctgctggatttccaagctgagaggacgtgaacctgggaccaccagtagccatcttgtttgccacatggagagagactgtgaggacagaagccaaactggaagtggaggagccaagggattgacaaacaacagagccttgaccacgtggagtctctgaatcagccttgtctggaaccagatctacacctggactgcccaggtctataagccaataaagcccctgtttacttgaaaaaaaaaa

SEQ ID NO: 17 - protein, 224 aa, Homo sapiens
MEKLLCFLVLTSLSHAFGQTDMSRKAFVFPKESDTSYVSLKAPLTKPLKAFTVCLHFYTELSSTRGYSIFSYATKRQDNEILIFWSKDIGYSFTVGGSEILFEVPEVTVAPVHICTSWESASGIVEFWVDGKPRVRKSLKKGYTVGAEASIILGQEQDSFGGNFEGSQSLVGDIGNVNMWDFVLSPDEINTIYLGGPFSPNVLNWRALKYEVQGEVFTKPQLWP

SEQ ID NO: 18 - DNA, 26803 bp, Homo sapiens
cttgctctgtcacccaggctggagtgcagtgctgtgatcatggttcactgcagccttgaactcctgggctctggcaatcctcctgcctgagccttctgagtagctgagactatagatatgggccaccacacctggctaatttttaattttttttagtagagatgaagtcttgctatgttgaccaggcttgtgggagttcagtcaggctggtggaaaaaattttaaagatagttataagaaatagacacaaaccttcttgtaaggctggagagggtttacattgcttcagtaacagatttggctgaaagcagcctaatcctctctacctttagctgatagcaaaaatgaaaataacaagggaatgtgaggaagtttatctaaatagcttgcttactcatgtggtcctaaaaccaaactttgatcaacctcaggtgcataattgctctctactcagggggtgagcaatgttaattaccctctagtggtgtttactcgagacctttgtcatttaatctgtattaaataaatgtgaactttgctagcttattgaggtgatgctccagatgcagagcagagccccttagccagactgacaggcaaaatatctgtgtcagtgtatgtctctcatccatcactggttcagggtctgcgggctggattcctgcacaggctggtcttgaactcctgggctcaagcaatcctcccgcctgagccttctgagtagctgagactacagatatgggccaccacacctggctatttttaacattttttagtagagatgaagtcttgctgtgttgcccaggctggtcttaaactcctgggctcaagagctcctcctgccttggcctcccaaagtgctgggagtacaggcatgagtcatggtgcccagacggacatttttttaaaaataaaggaatactcctgaaacgctgaagtcttctttgtacccctctgtgataacatgaatagcctcttaatgacaccaaggagcaagacaagttagtcccaaagtagctcacatagatgatgataaaggaatgaggggtgggtgtgatctatgcaaaaaacccttactctttaatgggttgctgtttctaacataattgcaacagtaccctacattgctataatgcattatagttttcaaagtgcttttgtggcctccataatagagaggttgtgaggtaagcttcaaccacggctgccctactacccaagagtggacacacaatgatgaataggtcaatttctgcctcttagtttcttagctagggaggggcacttactggaacagcacagaaaacagagtctttggcccagttggagaatctttatcaggttatgctacttcaagctttcctcctgttaaatgtgagaggaataaatccctgttccttggatcagtgtgactctgaaacagctggaggagagacagctttaggcaggttgaaacagagagctccagcatatgtactttttttttttttttgagatggagtctcgctctgtctcccaggctggagtgcagtggctcgatcttggctcactgcaagctctgcctcccaggttcatgccattctcccgcctcagcctccctagtagctgggactacaggctcccgccaccacgcccggctaatttttttgtatttttagtagagacagggtttcaccatgttggccaggccagtcttgaactcctgacctgaggtgatccacctgcctcagtctcccaaagtgctgggattacaggcgtgagccactgaacttggccaagtgcactacttttaaaagttaaagtattatgcagccatgagggaatattgtgcaagaagaaagcttttacaagaaaaacttgaaacattggtatttttgcctcctttttaacaactagagtcgttttgggagttgtttcttgtcgaagaaacaacccatgtttattttcccagtatggcaggaccatgtaggaaagcaaaattacccctcaggagaggaaattctctgacactctataaggctccataaccctcctctgaactgtggccaacaagattgggtagcactttttaaggtagtttaagaaaaataggctgtgcatggtggtttatgcctgtaatcccagcactttgggaggccgaggtgagtggatcacctgaggtcaggagtttgagaccagcctgaccaatatggtgaaaccccatctctactgaaaatacaaaaattagccgggtgtggtggcgggcacctgtagtcccagctactcgggaggctgaggcaggagaattgcttgaacctgggaggcggaggttgcagtgagccgagactgtgccactgcactccagcctgggtgacagagcaggactccatctcaaaaaaaaaaaaaaaaaaaagaaagaaagaaaaatatatagtgagcccaataaagctgtataatctaaatcaaacatgacttgcatgcctggagactttgcactagaaaaatatttctacctaaaaaatcaaattttattttctttctcacaaatattcaatctgctttcatctcagttcttcctaccttgtcaaacctctccccacatttcctattctttttctctccagcctgatatctctcattatactgcttaagagaaatgttatgttactattcttttctcccagaactgtttctctggttctttaaggtgtctgagtacacactgtgccttcttccttttagccctctcttctccttgttccctgagccttacctttatgaccttagaacttcaagttcccactacaattttaaatatagactattttgcttttcctcctactagggagcttaaattgcctctaattacactgttttcccgagtccttcctctcctttgcaatttagatatagcacagaagcacattttgcttgactgtcctctgaactgtcatgctgttttgatgtggttctattgtccaagagtcttggttaaataatagcccagcatcccacctgtgtttaaaagaactgcttcacaggcaaatcaaaaagcccatggatccgaagtcacaatgggcgttgctattcaaacagcaccagattgctattcaacgcttggttgaaaaataaatttcagtttcattcacctaatatatttccttctattttgtaggatggtatgctcttacttcaatttggacttgttcacaattgaacgttaacatagccttatagattagcctgttttcattggtccagagtattctccaaataaagcagggtctgtgcattttaagcaactcccctgaacaatttcatgggcattctcaaatttgagaactacctgaaaagctgtgttggagaaaagaacaaccaatgaatgtggcaggacagaatattgaacattaacttcccttttcctcttctcccatctgttctcttccattatccctacccgtccgctcagtctcgttattcaggcaacagttattttgccattatttcctcaagaaaggaacaaaagtaaacacaattgctttctgattttttttttttttttgcattttaaaatggactttgaaaccataagcaaagaggtgtttaagagtctttccaaagccaaaaatgaaggttttgaaatttcaaagtcactgccttgaagagactcgaggtttggagtgtgtacagtatgtcggagctggacttttctccttcctgagactagataacggtctgaatccaagacagttttcatgatttcagaggaagtggtcaagtggtctgtgaggtagaccttctgcttaagagcagtcaggaggccgggtgccgtggctcacgcctgtaatcccagcactttgggagaccgaggtgggcggatcacctgaggtcaggagttcaagacaagcctgaccaacatgcagaaaccctgtctctactaaaaatacaaaaaattggccgggcacggtggcacatgcactccagcctgggcaacaatagtgaaactccatctcaaaaaaaaaacaaaaaaaagagaagaaaagaaaagaaaaggagcagtcaggatgtgtgcctccaaagctgaggtagacaaaaagataccagagttctagaggcctgccaggcacagcagcagcagcagaaggaaggtgtgggcgagaacagggcagccaggcgtgtgccacctcccagacacaattattgggaatggagggcaagtggtgatgggagaaaatcttgacttaattgatgtcaagattaaagaaatgccacctggtggcatttaagttcacacataggtaaagaaagttatgcatttactgtgaaagtcatcccactatttagtagaaacaggagatctggattctggtcaagagtctcttttgccaactgtggcaccactgagcagcggcacagcttttgtgaatcctgggttcttcattattaaaatggggacattagcgttgggttgagtataagaaatggacatttttgcaggtcaaaaatggttgaatatttgcattttcatatgattcaaccgaatacttacttcacaggcataaggaaaaaaatagaataacatactaacaactgtccctggagtaagtacttaacaaatacatgatttataaagaagatatgtgaaagatatttgtaagtacatgatttatagaaagatatgaaagtatgtaaacccttgtggtctaatggtcacagaataatctgagcttaatatccctgctccctaccatacagaaggcaaaatgcctattaggggttttctttcttcaccctctccttctttttcctcctcctcttgactcctcctcatcctcctctttcttcttccccttattaatgtctaaaaaggggctgagcatggtggctcatgcctgtaatcctagcactctgggaagctgcggcaggtggatcacctgaggccaggagtttgaaaccagcctggtcaacatggcaaaaccccatccctactaaaaatacaaaaattacccaggtgtggtggcaggcacctgtaattccaactacccgggaggctgaggcaggagaatcgcttaaacccgggaggcagaggttgcagtgagccaagattgtgccactgttgtccatcctgggtgacagagggagactctgtctcaagataaataataataataataataatttctaaaaaggtaatacattttcatagttcaaaaaccaaaaggtataaaaggaaatacagtaaaaaatttcctatcatatcactgtctagagtactattccttatatattttcctgatttttgagtattttaaaatgtgagtgttggatatgagtgttggatttaaaaagttttatgataatttgtgtatatttgtgtgtgtgtgtgtgtgtgtgtgtgtgtatagtagtccaagactatcagtttatgaataataagaggagacccatggaaaaccagtccctttgaccaagttcactcagataatcagcagcagggcttggacattaattacagttatccaacatcctttgaggtctcacatgacaaattacaaatatggagtgtaaatgtaacccactttgctaggcaaaaaaagccctgtttttttaaaaaatatatatttttggcttatgggcaacagaagccagggagacgtacagtcaaacctcatttctcatggctttcatatctgcaaattctcctactcattaaaagttatttataactcccgaatcaatacccacagcacttttgtgatcattggcagacatgtgcagaaaagaaaaaaaaattgagttgttgattgcacacattcccagctgaatttcaacaaagcaacactctgccttcccacttcagctttcttactatatgtgtgtcctttttctgtttatttagtaccatgtttttcacactttcgttctttttggtggtgattttgctgtttaaaatggccaacaagtgtagtgctaagtgctgcgtagggttcttaagcacaagaaggctatgatgtgccttatggagaaaatacgtgtgttggatcagtttcactcaagcatgagttatggcgctattagctgtgagttcaatgttaacaaatcaacaatatatgctaaagtgtctttaaacagaaacacacataaaacaaggttatatgtttggttggcaaaaatgttataaccagaagcttgcagaaacctaaccctgtatttcccttaagagcaatggttcattattcactaattcaatgtttacagcaactttataaactataactaccatgaataatgagaattgactatgttttagatcataatacctgaagtgaagttttccatcatggtttttagttcttagagtccatttaagttttttaaaaatatgatagctatcctatcacatcccacattcttgagattaaaaaattaatcttttatttggtacagaaaaggctcctgcgtgcatttttggaggggctggaccgctgaggaagtcatggttggctcaagtggtttaaatgcattgctaatttcatagcctctgaaccacttatgaaacaatactgatgatatgtcagtagctatgtttgcagctccttcaggaatgcttatatcttttactgctggtaaagaagaaatttatagtaatagattttttttttttttagatagagtctcactctgtcgcctaggctggattacagcggcttgatcacggtttactgcagcctggatctcccaggctctcctactgtagcctccccagtaactagggcccccacacaggcatcaccacacccagctcatttttttatgttttatagagacagggtcttactatgttttccaggctggtctcaaacttctgggctcaagcaatcctcctactttggcctcccaaagtgctgaaattacaggcatgaaccactgcacctggtttatggtcatcttaagtagagacttatgagtgcgtatcattgtatcaccaatctgagactcaattttatctttctgttaatagacaatgcagtttttctgttaattacaatgaaaatcaagggttgcttagcaagtttttactcataactccaagttttgtgacttatagtgagaaatgggtataattctttgtgatttgttaaaatgcagtatttcgaggagggataacatataaaatttaacagtttcctatcattatttttatccttttgaaccactgtatactacagatagacaaaggcagctttggccacttactcctcagtgtgactaagttgaccagatgttttccagaccacaggttctgtcaagagacagtgtggagagaaatgggtaggcaggtatggaaagaagagtcagaaacagatagtgagctaatctctacaaatggctcgttatggcctgagctgtgttctcctccccgcaaaaagatatgttggagtcgtaatccccagtacctcagaatgtggccttatttggagattcgatatttacagaggtaagcaagttaaaatgagatcactatagtgggtcctaattcaatacgactggtatccttacaaaaaaggggaaatttaaccacagatacagacacacacatagggagagtgctagtgaaggtgaagtcagagattggaatgatgtagcagaagcctaggaatgccaaagattgccagcaaaccaccagaagctgggagagccacatggaacagattctccttcacagtcccctgaaagaaccaactctcctgacacctcgatttcagacttctagcctccagagctggggtcaatgagcttctctcattaagccatcatccagtgtatggtactttgttacagcagtcttagcaaatgcatggttcctcactggaaccatgaatttccatgcatttatttcatttaaataataaaacggatcccctttgtggcttgtagttctgttccatttcaaaaatccagaaaaaagatttgttcagaagctagaaatgatgaactggatcttgcccaaggtcataaaaccacaaaaccctttacagagcacaaaagtctgatttttcaaagcttctctcaaaagatgggtcactccttagtcatttaggccactgacaactgccctggactctttatttatttatttatttatttatttatttaatttttttgagacagagtcttgctttgtcgcccaggctggagtgcagtggcgtgatctgagctcactgcaagccctgcctcccgggttgacgccattctcctgcctcagcctcccaagtagctgggactacaggcacccgccaccacgcccggctaattttttgtattttgtttagtagagacagggtttcaccatgttagccaggatggtctcgaggtcctgaccttgtgatccacccgccttggcctcccaaagtgctgggattacaggcgtgagccactgcgcctggcctggactcttacatataataagcttgacttatcgtacaacttataattgatgctttcacgtcatgggaagatcaaattaatgcagagagcgactacgtttctggtgggagagcagcaggggtcttgagaggaacagcagtgttgactgtttcgctacctactctgggtgctgattacatctttctttcgtgcaggcaaatccacttggagctattttgggctcactgtgggcatcattctttgtatactctgctcctttcccccatagtttctctattgatgggggattactaaagaatgaagaaaagaacaaaatgaaagtggcttttgaaaaattttaaatgactgtcactatgtaacatattcattatttcatgtctccactggacattttggagatgtgagccttgcaatacctacatgaatgcttctatgattatgattattgttttgctcttcgcctaacaacttgccaagtattgtcaacctcagtgtgtgagatggggtccactcaaacatcagggccgaagtcaggtagttcagttaagtgaatttgataccaggaactagttacaaaggagttggaagggctggaaagccaaactggagaagaaggggaaccccagagtaacaatagcaggaagcctctaccgtctacctctagaactggggaggagctgagttaacagagtcctggagccattgctggggaagaagaaccccaactgcagaggaaaagtggccattgtgaagaaggtgatggtggagaagtcgtctgaatcaaaggggagaggatatgttggctcctttatctttttatctttcattgtcctaattccttctgggcatggttaaatgagcccaggaaatgcagttggcaggaatcagcttcctgtgacatagacagagtaagagaaggacaaaaataatgaatctgagagcaagcaggcaaatgaccagcacattaagcctagcacacagtatgttatacgggatttggggtagcaaaagatgaaggcaggtcagagaagccacaactaggggatgggcaaggtcaatgaggtatgacgggtattgtatacaggaagagggtcataaacaggagtggagtcaatacaggagactaacatatacacatcataaatattagtagagaagcataaaatagtctcctggagatcagggaaacaggaaattataggttttcaggataattcagccatatccaggaaacacacacagtgaagtaacaaagagtcaataggcttagagtggtacaattcattatgcacatgtaggaattcattccaaataataggctgaaatgtagacatgagaatccaaaaaagatgttttcttagtttttgccaatatcttagctacgttttttttggttcaacaaagtaagttaacagtcatatctgcttggaaattgtatttaggccaggtgcagtgtctcacgcctgtaatcccagcacttggggtggctgaggcaggaggatcccttgagcccaggagttagaggctgcagtgagcgacaactacaccactgcattccagtctgggtgacagaacaaaaacttattaaaaaaagaaaaaaaaaaggtcgggcgcggtggctcacgcctgtaatcccagcactttgggaggtcgaggtgggcggatcacgagtcaagagatggagaccatcttggtcaacatggtgaaaccccatctctactaaaaatacaaaaattagctgggcatggtggcatgcacctgtagtcccacctattcaggaggctgaggcaggagaatcgcttgaacccgggaagcggaggttgcagtgagctgagattgcaccactgcactccatcctgtcgagactctgtctcaaaaagaaaaaaaaggaaaagaaactattgaaatagctgatattagtttgcttacttgtcgttactctttttcatgatggattataaagaaaagttataactatttgaattttctgctgatttgaagtctctataaacagtacattcctttttggtacacagagggcacttatctgcaagaaaggcaaagaaaatggaaaagttaatgaaagaggaatcatccaatccacgaacagaatgaaaccacatacacagtgaagaaacttgtcttacattttcttccttatattacttatcattcatggtagtgactactttggggcttgagtaaagcttctctaatttattccatgtagcatcatatgtgaaaaagacaaatagatactttagacatgataataacactttattttttatttatttgtttattttgagacagagttttgctcttgttgcccaggctggagtgcaatggtgcaatctcagctcactgcaacctctgcctcctgggttcaagcgactctcctgactcagcctcccaagtagctgggattacaggcacgcatcaccacgcccagctaattttttgtaattttagtagagacagggtttctccgtgttggccgggctggcctcaaactcctgacctcaggtgatccacccaccttggtctcccgaagtgctgggattataggtgtgagccaccatgcctggcccataacaccttatttaaaaataatctgtctggatccatacaacttgtctggataactaaattggaaattattccttgttttaaagtaattcaattgaaaatttttaaatttttttgttaatcaagcactttttggtggaatctaaattaacacatgtaggagatgcctgtttcactaattacacaggcatcttgcagtaattaatgtctgggaggaaggaatgtcttttgcttactctcttcttcttcacaaaaatgtgaattttggaaagcaataatggaagcatgtagaattatagaaatacaaatgtatataactatcacaaaaaaatgaggccaaaggactattcagatataattaggctatggtagctgtaattatctaggaaattaataaaattcattcacctagaaattattagtgagcatcaaatatgtgtcagcactaggctagggtctcagaacgtacagataaatcatagttctggcttcagggagttatatagattagagataaaacctaactacaggggctgggcacggtagctcatacctgtaatcccaccactttgggaggccgaggcgggtggatcgcctgaggtcaaggagtttgagaccagcctggccaacatgataaaatcctgtcactactaaaaatacaaaagttagccgggaggtagtatgtgcacctgtaatcccagctactcgggaggctgaggcaggagaatctcttgagcctgcggtggaggttgtggtgagctgagatcacgacactgcactccaatctgggcgagagagtgagaccctatctcaaaaccccaaacaaaacaaacaaaaaaaccaaacctaactacagggctatgagagatgactactggcaaggagccacaggtagaacaaaggggatgtgtccccaggcaaagggtagtcagcaagcctgcaacctcagggttcccggatctgagcctctggctcttggctaggcaggccccaagcgttggcctcctgccatggcaagctccagcctggtctcccaccttgagctaacattcatatgttgtagacacagccacgcttcctgcttacctgtcacttccagttctcgaaggcacccttttcaaatgaaaatccgccccttttcacatcaaacagctcatctggtcctgtggattacatttctcagaaatgcctctgaacattcgcctcctctccacccccactgcctctgctacagtgcaggtgctcgccatttctgatttgttctgtcacacactcgtttatcaggtctctccatctcctgttttgacatgctgtaaagcaatttgccactggaaaaaagggctctctttttttttttgagacggagtctcgctctgctgcccaggctggagtgcaatggcatgatctcggctcactgcaacctctgcctcccaagttcaagtgattctcctgcctcagcctccctaaagtctgggattacaggtgcacgccaccaagcccggctaatttttgtatttttagtagacgtggggtttcaccatattggccaagctggtctcgaactcctgacctcaggtgatccacccgcctcggcctcccaaagtgctgggatttcaggtgtgaggcatcgtgcccggcctctctttccaaagtatgttattatttttcccaagaccctttgacggatcctcatttcctacacacagtggttctcaaacttggatgtactccagaattacataggaaattcttcatttttttagacgaggtcttgctatgtttctcaggttggtctcaaactcttgacctcgtgtgatcctccggccgcagtctcccaagtagctgagattataggcgtgccactgagcccagctggaaatttttttaaaacacagattcctctgaatcaaaatttctagaagtgaggtctgagcaatctgtatttttaacaagttatccagatggctctttactgtcagtctggttccagctgagggagttttagaattacaaggcaaagtccaaacttagcacacaaagtcattcacatcaactcttcccctgtacacaccctatgtcatagccagagttgtaacccatttcttaaacacccagggttcttttaagtctctgtgtcattgtatgttattttctctagaattgcctttaacctcctttccaccctggaaagcattccctaagccatctttgaagctttctttgatctctaacttagagtcctcctctccttctaaagccctgtgttaatcacttgtcatggtgtactttaatttttacttgcctgtttctctttacggtactttgacttcaaagggtggggctgcaaattagtcatctccttagagtccagccttgttcctagttcctaactggcacttaatataaacgaatgaatgaatggacaaatgaagagaatgctagttatgataaagaattggccgtgtatgagactacttctctttatgaactaaataattatatgcctttcaataaaatactagtacacgtagctagcacaagctcatcagcatttgagatgatatggaaaccaaaataaacaaatgctaccacaaaaacataatgactgctttccccagtgcaggactgatggaatcatcaaacattgagattaatgtaatgtttggcagatgtccagtgtttttatttttcatttgcctttgtgttcatttatggactaacaatataataaacacacacatactcacagtacatcttttttttttttttttttgcaaagcccagttttcttcatcgcatatctttgttttcttcaagtatccccttacttaatgttggtagtattttttttaatgaaatataaatccctaaccaccaagcaagaaatgagactcttaattgcatcagtttacagtgcaatgtgagtgtaaatagtgtaaattgaatttttaatggacttttttttttcccgtttttgcttgccttacattcattatccctccctgggtaataaacatttatttttccctttgtaaccactcctccccttctgtccatgtggttctttttagtggagctggtggtagggatgtggcatgagattcaagcttggccacctggagtcactgtgttgtgctccagaaggacacctgatccaagtcagccagtaagagtgagccccaggatttttgcttggaccactgaggaaaagtgtactctgccctgtggctgatcaaccattaggatataagccattgttgtagctgtgtgagtcaagctacctgagaatgaggacaacacagtggcaagcaacaccaagagagaaaaagaggcagattctgatgacatttttgagcctttgcatccagctatgcctgaatccaatttatcccctggaatttacacttacttgagctccacccacttgaaagaaaacatttctttttattcttagcctgatttgaatttggcctctctcatttactacccaaagtgtcttgaccactagaatattatgccagactttacagcatcattgaatttgccactttccagaagagttgtgtgaattttcaatgtagcttttaccttctatgagtatctagagatatatttaagtagaagtactccactagtttgttgtgagatcttaagtcacttaatttctctgtaccctagttccctcatttgctagacctagggagctataatgttccttctgcaaaattcttattttgtgaaatattctagaatgtctaactgatacactgctagaacaactgactgctatttaagaagagttgactgctatttaaggatcataattctctaggcataagtgctgtgacggcacagcgtgtgcatcggggctgaggggtggggtggagcagaaagtaggaggagaaagtttgataaacttccttttggataaattgaaaacagtcaaataatttataatttcttatattatcattattagcttcttctataattaggagacttgttccaaaatgtgagaattgtcacaagttgtcaaattcatcaaaggaagaaaatggatgtctcacaaaaaagtatgctcagtccaatttcttctcgtcacactggaacaaactgaacagttttacacagagatgagaagcctggacatttttcaaatatgttttgaagagaatggcaatgcctgagacagaagtaggaaaaagcaatgaatatttaaaaatctgagctggtgtaaaactagaaatagttttagtaagaacaatgtgatgtgctacactaagtgaaatgtatacattgggccacattataatcaaaaataagaatgtacttttattcatcttttatttaaacaataatcaaggtggcgggcgcggtggctcatgcctgtaatcccagcactttgggaggccaaggtgggtggatcatgaggtcaggagttcaagaccagcctggacaacgtggtgaaaccccgtctctactaaaaatacaaaaattagctgggtggggtggcatatgcctgtaataccagctgctcggggggctgaggcaggagaatcgcttgaacttgggaagtggaggttgcagtcagccaagattgtgccattgcgctccagcctgggtgacagagcaagagactctgtctcaaaaggaaaaaagaaaaaaaaaaaatcaaggtaccatttgtaccatttcctggaatttctccaaagtggcaaggtcacatgtttatacattagactcccagtttaacacacagcagacaataactttttttttttttttttgagatggagtctcgctctgtcacccaggctggagtgcagtggcacaatcttggctgactgcaacctccgcttcccgagttcaagcgattctcctgcctcagcctcccgagtagctgggattacaggcatatgccaccatgcccagctaatttttgtatttttagtggagatggggtttcaccacattgtccaggctggtctcaaactcctgacctcataatccagccacctcagcctcccgaagtgctggtccacccttccttcttttctcccttccatccttctcccttttattccatttttctaaatattagaccatagtacaaatcaaaagtcacaaactgataggctgcaatgtagatacagctgggaaaatgttttgtttgcagaacactggggaaatttaacatgaaaaactggaagatctcaatccacatggccacatggtaatattattaatgttgcaggggctttccaattcaacatgtcctctgcatccctactatttatactgccactcatccacctttctgtattactggcctatcacctatacacgtttgagtttatattcttctggctttacttagcaacttaccttttatatttaacattacaacatggtattatcaattagtattcgattcagttgcatataaccaaaaatgccaaattatactggcttaaacactaaggatttatttttctgtcatataaaacaagtctggaggtgggtagtccagggctaatatgacactccagtgtcacaaggtacctgggctccttctatttatcttttttttttttttttttgagacggagtcttgctctgtagcccaggctggagtgcagtggtgcgatctgggctcactgcaagcttcgcctcccgggttcacaccattctcctgcctcagcctccggagtagctgggactacaggcgcccgccaccacgcccggctaatttttttgttatttttaatagagacgaggtttacaccgtgttagccaggatggtctcgatctcctgacctcgtgatccactcatctcggcctcccaaagtgctgggattagaggcgtgagccaccgcgcctggccctatttatcttttataggacatggcttccagtctcaagttcagtttgtcacccataatggccaaagagcagtagtcaccttacctgtttcaggcaggaagggcagagggcaagaaacaaaatggtgctcctcctgattgagtcagcgttctttaaagatgttttccagatgttccacccagccgcgtttttttttttttgagagacagggtcttgctcttgtcacccaggctggagtacagtggcatgatcatggctcactgaggcctcaatctcccaggctcaagcgatccttccattttagcctcccaagtagctggaagtagctgggaccacaggcacatgccaccataccctgctaactttttcattttgtgtagagacaaggtgtcactgtgttctccaggctggtctgcagtttccaactcctgagtgcaagtgatcctcctgctttggcctcccaaagggctgggattacaggtgtgagccactgtgtctggccaagctacttctacttatatctcattggtcataacttgatcacacagccacatccagctacaatggagattgagaaatgtagtcttttggctgggtacacagcatctgaataaaatccaggcattgttactaaggaagaaggagtaagtgtcaatctctgctccataactctctaggttaatacacacagatggaggagattgctagttgcccctcaagatccagccttgccttctgggctaagaaagcccctgagatttacctggccatagtggcactgggaacaaacaatgtatttctaaatcttctgattttaaaatctttcagaatcacgatttctccgacatcagtatttttatgtctttagaattcaacaaaatgaaattcctaagtctaatatatgtgaatattaagttttagcagatactgctacataactttccagaagggtgtggcaattcacatctccaccagtgatcagcatgttcattttccatacagctctggatattttgtctattttaaaatatcttcttctaatctataatttaaaaatgtaacttagtaggaatttaattgttcatgtaaccaaatcttcccattaatggctatgggtttcttcttttacttcagaaagtcctccccaccttcagagtatataaacatttttttctaaattcccttctaatttcttataatttatagttttatttttgttatttgattcatttattctctcaacagatatttattgagcacttattatacgtcaggctctcttcaaactctggtgagagtattttctaactgggagagacaaccctagttgataagaaacaaacaaaccaataagtaaataagacatttcccccagataattaatacttggtgacgggggaagacagtgagacaggctactttacactggcaggtcaggaaaggcttctctgaggaggcaagtgattcaggattaattgatgactggtggagaagtccggggagtggacacaggtgggaacagcctggtgggtgtgaacagcaacaagaaggttaatgtggcttcatggaacagggtgaagatgagacaagctgaacactgaggtgggcaccagaacatggagggctttgtaggtcccaataaggagtatggattttattgtatactggagatttgtcatccatctagaatctgtttttatatataagaaaaggtgtatatgtttgcgcaagtgtgtgtgtgtgtgtttgggggggcggggtgggggcagacagggcgtaacttttctttaaattagagtcaaaatttaattaaactattcattctttacaggcagtgaggggattaggatcttatcccacagaatctcacctcatttcaaatgttgtacagatattatctgagatatattttcaggccgggtgcggtggctcacgcctgtaatctcagcactttgggaagccgaggcgggtggatcatttgaggtcaggagttcaagaccatcctggccaacatggtgaaaccccatctctactaaaaatacaaaaattagccgggtgtggtggtacacgtctataatcccagctacttgagaggctgaggcaggagaatcgcttgaatccaggaggtggagcttgcagtgagccgagaaaacgccactgcactccagcctgggcgacagggcaagactctgtctcaaaaaaaaaaacgaaaaaagaaatatattttcaatgaaatcaagcatataatgactatttttatcccagcatcttggcttcttcaggctgctataacaaagcatccctagtggagcatccctaatctgaaaatccaaaatccaaaacgttccaaaatctgaaaccttctgaacactgacatgacaccacaaatggaaaattctacatgtaaatacacgtaaatacaaactttgtttcatgcacaaattaaaaatattgtataaaattaccttcaggctatgcatataaggcatatatgaaatataaatgaattttgtgtttacccatgggtctcatccccaagatgtttcattttgtatatgtgcatactcccaaatctgaaaaaatccaaaatcttaaatatctgtagtcctaagcattttagataagggatattcaatcccttatccataaacaatttatttataaacaacacaaatttaggctttgtaaaaaatagaaatttggccgggtgtggtggctcacgcttgtaatcccagcactttgggaggccgaggcaggcacatcacttgagctcaggagtttgagaccagcctggtcaacatggtgaaaccttgtctctaccaaaaatacaaaaattagcagggcttcgtggcatgcgcctgttgtcccagctactcgggaggctgaggcaggagaattgcttgaacccggaaggcagaggttgcagtgagccaagattgagccactgcactccagcctgggggacaagtgagactccacctcaaaaaacaaacaatcaaacacaatataaatttatttctcatagttctgcaagctgagaagtccaagatcaagatgtgagcagatccacctttggtgaagggctgctttccatttgatagatggctgtcttcttgtgtcctcacatggtggaaagggtgaggcagttttttgaggtctcttttaaaagagaactaatcccattcatgtgggggtctgccctcatgacctaatcactttccaaaggccccacttcctaataccatcaccctgggggttaaattttcaacacacaaattggttggagagtgagcgaacatagacattcagtctatagcccccagggatgtagccactgaataaaataatctagaacttcatctagaggcagtttataagtcacataagaaaaccagttttacttatagtcacataaaacttttgataaaaaacaaccctagttgataagccatttgtttactggacttggctctgaagaaatgacttttggctaatcctcaaaatgaaatctactcacagagggcaagatctgccaccagtgaagatgtttaaaacaatgtgctgtaggctttgaaggcaagtctaaagaagagcttctaaaaatattttgcacaatggtagcattaaaagagtaggcacatgggccccaagataacatctgtgaagaggaggaccagtgtgtgtttccttttgtatgtttaagtactaagtcagtgattactttataattaaaccatattcctcttgatctgtccataataaggtcactctgtaatttataataggcttcttaccaaattcaagctttacaacaaccctataggttaaatattcctgtgaattttatagatgaagaaacagagtaagtgaaagagttcatactcaattcaagtctcttgagtctaaaatcagtgctctctctacataagaagttagttgctaagatcacacaacttgagaagagagaagacagttttcacagtccctcccctctgaccactaggctgcttggggtacttttacaacttacctgctctgaattaaggctctctgtgaatctgattcatctgccaatttgcaaacagtcagccctgtagtacgtacctaagttgatttttaaaatactatttctcatcttaaaataatggaaattgagtgacataaatttcctggacactttttaagatccaaagacaatttgctaatttgtcgttacaattaaagagccccccaaaaggcgtaagaactggattttgacttggacttctgttccttagtttctttaacatattgggggccgggagtggtggctcacacctgtaatcccagcactttgggaggccgaggcgggcagatcacgaggtcaggagattgagaccatcctggctaacacagtgaaaccccgtctctacaaaaaatacaaaaaaaaaaaaaaaaaattagccgggtatggtggcgggcgcctgtagtcccagctactcaggaggctgaggtaggagaatggcatgaacccaggaggcagagcttgcagtgagccgagatcgcactacactgcactccagcctgggcgacagagcaagattccatctcaaaaaaaaaaagaaaaagatattgggaaaactcacttaaactctatgggcttctgtaccactaaggcttctcaaatttgatgcaagtaatgggaacttgctgtggctaacttgagccacaggagaaggatactgcaagactcacaaatgcttgaaagtttcggaacaggtttggaaatgggtaagaaccaaggaccgggttgacctgaactgaaaggaaattgaggtgctattagggacaaatatgaaatgaaggatgaactgtctctgacatcctttgcttctgtgtttggagatgagtaagcagggagtgggtgcatatgcaaacagggtggtcagaaatgctttggccggatgtgtgactgaaggctatgtgcagctgaggaaggctgggccaccacagtagcagagaggctgaccaatttggcatgcagcaagcaggaagtagaagggatcttaagcaagcaaagtgtttgggtagacaagattatgaggaatgagcaccaatgacatttccaacaagcactgaaagcttccaaatgcttctaacagttactgcctgtacaaacacaggacagtcttgactatgtgagactgtgacagtttcctcatgcctatgaaatgagagacagtacttagcactgacatgagcttcatatttgaaggcagcaaactactgaaccacatgtagcttccgaaatcaaaagatgcaaactggcagaccacaggtcagatatgacatgcagaaaaaaattagttactatcttagcctagtttgtgctgcttacagaatatcagagactgggtactttatagagaacacaaattatttttcatagttttagaggctgggaagtccaagatcaaagggccatcatctcgtgaaggcgtccctgctgtgtcaaaacatggtggaaggcatcacatgggcaaaagagagagagggaagcgggggcaaactcctttttatcaggcacccagtcctgtgattcattcatgaagacagtgtcctcctggcctaatcacctcttaaagctcccacctctcagcactgttgcactggaaattatatttctcacacatgaactttggggaacacattcaaaccattacagttaccaaagataaaaatgcagatttcagatttctcttggggaagaaaaaaggctctggcaataccagggctgtatttccacatggcaacagttgtctgttgccttctgttgggttgtgggctctcacattgccataccctcctcatggcccccttcactcataacagtacctgcctagacctcgaagcactagtttccaaccctgcttgagttaactacttccatgacaactgtgcaaggccagagtgtgggcagctaccttgagggccaccggcatgggctgcccaagtgaccgagggcactaacctctgctctcgaaacttctttggtaggatctcttcactcctgacttactacttgtaactgctggaaacaaccatttattctacccctactaaaccacatctgtcttttctgtcagagccaatcttcaagcatatgcttcctcaaaagactttaattaccaggtagtagaagcggcagcaaagagtccccatctagcatcttctaaaatgtagtggagaaaccaacgacaacgaatctgagacaaccagttgtttgacttctctgaaaacaacctctaaaaaaagccttctctcgtgaatagctgcagacatgctgggcactaattgatgatgatgccctttagtgagtctcctctgcacatacctgattccatttggatgctggccctcacatacttctatctgcgaactccggaacacagaatatcatacaatgtatgattcaatctggactctgctggagccattctctacaaagcagacacaactttttcttgcctaaatcctttcaagttgctttatttttatttttaaactaattaccataaatctaatttatcaagctgcttttaagataaactttaaaatgcttagagcagtctacaaattcttgcactgtttcactcttccttatctctcagtcttcatctcccattgcatcttctctgactctttcatatggatcttctttcaatttgtggaagaagccaagcttgttcctgcctcaggtccttgacacttgctgttcactctcctgggagactcttccccccatcttagcttttaaataccagctggtcagactccttacctgccttccaccttcctctcattctcccactcctcgccttcatttctcagagtcctccgctctcttctttctattgctcttaacacaatttgtctgttttccgctaatctgtaaactctacaagagcacttaactattttgcatcccaccgaatattcggagtcagcacagaccccgtcataatagagtaggtaagcaatgcttacctgtcaaatgaatgaatgaaacacccgattcatcccccaagccagcttaatacattagatgatcttatggactgaataagacatccctccttttaaagaatatttttgttttagcttcacatcagcaaaccccgaacggttcatcctaagataagcctggtagagaggaaagatactaaccttctagggtcctaaagtggaactaggaacttattagatatgcacattctcaggcattatttccgatagcccagtcagagaattctgggggtatggcccagcaatctgttttaacaaacctttcaggtaattctgatacacactaaagtttgaaaggtttctttaaggctttccagttttcttttcttttttggagggatgggggggggtctccccatgttgcccaggctggtctcgaactcctagcctcaagctatcctatcctcccacctcggccttccaaagcattgaaattacaggcatgacccactgcggctcgcctccgtttctaacttaaaaaaattttctttggaggggagccttaatcctttctattatcctgctagtagaatcttactactcctgagggtaatctttgtcataatccaaaagccttgaataaaggcctatttgtatagttatgcagaatatattcctgggaggtttgccttcctaggagcacaggtcggccctgggaggtgggggttggggggcagggctgcattctaaagtcctgtaacaacgcacaagtacaactgaatagaactcggaacaaaggcatcagggccacggtgcaagtctttgttcatccgttccccgactgctcaccctgtctgataccgctcttttccacccagaaaagcagccactcaagttttaagaatggatgtatgccgcggacgttttcgattaggccgttttctctcaggcactggaggatattcgtggctgcaggaggcgcttccaccctttcctcaacctagcaaagaagtaactgaaactaacccaagggttacaaccgaaaagccccttccagcttcagaagcagaactggaagctcggatagacttctccgcctctacactcctggaaaacccgcagtggatttcaccaacttcaggatcggagcccaggcaggcgaacgtaccttattgcgcatgctcgctagcccctcccgctcggagcggaagggggagcgctgggggcctgggcctggcctggccggggcgtcggcaccggcggccatcttggcttcccggggaaaggcggcgtgaggggaagaagttgtagggtgggggcaggagtgaggaggagggaagagagagggggaggaggccgcggcggggcagggcggggactgcctgcctgcctgggttgcggaagtgatagccgccgaccgagcctgctgctttcttgctactgcttcggcttcccggctaccccccggacggtgaaggcggcccagctgtggatggtcagatagcccttgtctcccgccgccaatctctggcccctagcagcacggagcagacggcggcagcagcagcagcaggcgaggaggaagatggcgggacggctgccggcctgtgtggtggactgtggcacggggtaagggggcttacgggcgggggtggggaaactgaggcggaggaaggaagatggcgggggagggaggaggccgggaaatgaatggtgcggcgaggtgccgccgccggctgtcagtcctagacccgccggccagcgaggggtggggcccgcagccagggcctcgcgggtcccctcgtttctccctcctgggactggggcgggggcgcgggcccgagattcaacccccaaccctcccagcggctttctccgcgcgacccctcccggcccttcccccactacggtgggcagcgccgcccaaagggcgctggggacggtcgtcttgggggtggtccccgggcccgacccatccggctttcctttccctccgcgcccgtttttgccagtcggtttggggacccaggggccgagctcggggactggcctggcaggggagctagaaaagagaagcgctcctggtaggtttgacaagatcgctgtgacaacattctgcccagggtgtgggtggggaaagggaagaatcggactctgaaaatgggaacctacagtggggctttcatttgaccacccaccttctcctttcgactcctggtcatttccatctccctctgcgttttaaccggtgaaccaagtcacattttaattcgagggagaaagatgtcatgtgttacttctgtagcctcaaaaaagtcccccagtgagcaagcgcgctgcaacttccttagttttgtcaaagccgcttcctgctttcagtcttttatacccttataaggtagtttttagtttccaacctgagcacatcttactagaacttttaagcaggttttaaagagactgaattaccggtgcttggtgtccatttatatgacttaaaaaaatgtacttatgtttcatggagtgggggaaaggaagcaccctggaaaataaactaatttaagttgtattcgttcattctgtgatggtatcttgaaggaagcaggaaggtatagaggtatataggagggtgtttaagttgcaaatagttactcgtagatatgtagggtagtttgcgaaaatgtagagtggctttaaagtgtggtcgttcattttgtattaatagacgttttagagagttgtaccacactcataactgcatagagaatagactacccttatttttatgtagaatcactgcttcaggatgacatataggaaagtggtttttttttctgtgctgatgacatctctccaattcccagaacactcccagttttttttttttgagggggaagtc

SEQ ID NO: 19 - DNA, 26803 bp, Homo sapiens
gccgcacctaccgctggcctcagacatcagcaccccaaagggtatgttggagtcccatggtggaggtgccggccgctcctccacgcacttgatgtataccgaggatcccatgcttgacgtcgcagggggcattagccaggagcacgttgctgggatgccagtccaggctgaggatggtggagccaatgggcttcttgatgtacttgcacacccaccagttattctcccgctggaaataacagatggcgatgacacacagctgccgcccacagcaaacttgtcctgtgggcccagcacacacagcaggcagtgggtgcgggcttaccctcctggcccgtcagcgtccacacagaggccttgtggcctgtgccataggtcacgatgaggttactcttggaggcccagttgatgccttttacctgcccgttgtgctccttgagctcgggcaccttggcccacttggccccactcttacagcttcgtggttgttgaggcagatggtggccatctgggtgcggcccttgctccaggtttggcagcaatgggttcctgcagtcagctgtgggaggctgtagttgctctccttttcagagtaccccagctgcagactctgggcaggacgcacccaaccagtgctctggttttttgaagtaaaaaatgcataatgcaattttaccatcttaaccattttttaattatgaaatccggtagtgttaagtataattgtgttgttgtgaaacagatctccacaactttttcattttgcaaaactaaataactcctctttccccctactcccaagctccaggcagctaccatttctgtttctatgaatttgactacttatattacctcatataaaggggttcataagtatttgtcttttcttgcttggttacatcacttagcatgatttcttaagtttcattcatgttgtagcacatgtcaagatttccttttttttttttaaaaaaaaggatgaagactattcgtttgtatgtatatgccacattttgtttatccatccatttttcttcaaatgtttgagttgtgtgatgtttaattatgtgtcaccttgacggggcaaagggttgcccagacagctggtaaaacattatttctgggtatgttagtgaggctgtttccagaagagattagcatttgaattggcaggctgaataatgaagatctgccctcatcaatgtggatgggccagaacaaaccaaaaaggtggagaaaggaccagttatctccccaccacccctgtgccctttagctgggacatccatcttctgccatcagacatcagagcttctggttctcaggccttcagactccagaagttataccagtggcttccctggcttttggactcagactggggtttcactgtatgtttccctgattctcaggcctttggacttgaattgaattacagcatgaactttcctagttctctagcttgcatatggcatattgtgggacttcttgacctccataatcatgtgagctaattcccataataaatctcctcttatgtatctataattcatatagatatgatatctatatatcaatcccatagataaatagatgtctcatatatatatcaatgtctctatatgtagatgtctcatatatggtatctatgtatctgtatcatctctatatatctaatcatctaatatagatgtctcatgatatctatatagatatatctatatcatagatgcagagatatcatatatatgtctgtttctttggagaattctgactgatacaggttgcttccgccttttggctatcatgagtaatgccgctgtaaccatgggtatgcaaatacttctttgagaccctgctctgagttcttttgggtaaatacccagaagtggattgctggatgatttggtggttctacttttaattttttgaggaaatgccatactgttttccataatggttgcaccattttataatctcaccaagagtgcacagggtttcaatttctctacatccataccaacacttattagtgtgtgtgtgtgtgtgtgtgtgtgtttaatggctgtcctaatgggtgtgaggtgacatttcactgtggttctgatttgcacatctctgataattgctggtgttgagcatccttccatatgcttgttggtcatttatatatcatctttggaaaaaatgtctattcaagtcttttgtctattttttttccttccaacttttattttaggtctgggggtacatgtgcaggtttgttacatggataaattgtgtgtcatgggggtttggtgtacagattatttggtcgcctaggtaaatgagcatagtacctgataggtagttttttgaccctcccccttctcccaccctccaccctgaagtaggccccagtgtttattgttcccttcttagcatctgtgtgtagtcaatgtttagctcccacttataagtgagaaaatgtggtatttggttttctgttcttacattaacttgcttagaatgatggcctccagcagcatccatgttgctgcaaaggacatgatttcgttcttcttatagctgtggtgtatatgtaccacattttctttacccagtccactgctgatgggcatctaggttgattccatgtctttgatattgtgaatagtgctatgatgaacatatgtgtgcatgtgtctttgtggcagaacaatttacatttctttgggtatatatccagtaatggggttgctaggtggaatgattaattcacttttaagttctttaagaaatctctaaacctctttccccagtggctgaactaacttacattcccaccagcagtgtccaagtgtttccttttctgcacaaccttactaacatctgttattttttgactttttaatgatagccattctgactcatatgagatcgtatctctctgtggttttgacttgcatttctctgatgattagtgatgtagagcattttttcaaatgcttgttggccgcatgtgtcttcttttgagaagtgtctgctcctgtcatttgcccactttttaatgggcttgtttgttttttgcttgttaatttaagtttcatgtagattctggatattagacctttgtcaaatgcatagtttgtgaatattttctcccattccataggttgtttactctgttgatagtttcttttgctatgcagaagctctttagtttagttaggtactacttgtcaatttttgtttttgttgctttgtccattttaaaaaatagagtaatttgattattttgttgttgaattgtaggaattctttatatattatggatgctaacatcttatcaaatatgatttgcaaaacattttccctcattctgtaggttgccttttcactattgtgtccttcaatgaacaaaagtttttatgtttgatgcagtcccatttgtccattttttttggttgcctgtgattttggtgtcatatccaagaatgtggaatgtgtcatatccacattcaatgtcctgacgatttttttctatgttttcttccagaagttttattgctttgggtctttggtttaagtctttagtccattttgagttaatttttgtatgtggtgtaagaaacaggtccaactgcattgttttgcatgtaaatatccagttttcccagcatcatttgttgaccagactgtccttttcccatttagtgctgttggagctcttcttggaggtcagttggccatgtgtacacaagtttatttctgggctctttattctgttctattgatttgtatatctgtctttattccagtaccacactgttttattcttctttttcaaaattgtttgactcttagggccctttgagattccatatcaattttaggatgaattcttctatttctgcaacaaatgctattggaattttgataaggattgaattgaatctgtagactgttttgagtgatattaacatcttaataatattaagtctaatccatgaatgtgagatgtttctatttatttatctcttctttgatttctttcagtaatgttttatagttttcattatataagtttttacttccttagtcaatttctaagaattgttttctttttgatgccattgcaacgggaatcattttcttaattttttcagatgctttcactatttgtgtatagaaatgtaactgattttttgtatgtgtgttgattttgtatctggtaactttactgaatttttaaatttgttctaacctgttttttttttttggtggaatctttaggattttctgcatataagatcatgccatctacaaacagaaatttttacttctttcttcccaatttggatgccttttattgctttttcttgtctaattgctttggactggagttccaatactctgttgaatagaagtgtccagaacagacatttttgccttgttcttaatcttagaggaaaagcttccagtttttcactgagtatgccgttagctgtggacttttcctaaacaacctttattatgtgcaggtaatttccttctctttccacttttgagtgttttttttcttttcttttctttttttgtgtgtgaaaggatattgaattttgccaaatgcttttcctgcatcagtggagatggtcatgtgggttttgtcctttattctgtaaatgtggtgtactacattgattttcatatgttgaaccatccttgcatcccagggataaatcccacttgatcatggtgaatgatcttttgagtgtgctgttgaatttattttgctagtatttttttgactacgttcatcagacatattgggtaattatttattttttcttgtagtatttttgcctagctttgatatcacactaatgctgcccctcaaagaatgaccttggaagtattcctttctcttcagtttttgggggattgatgtaaattcttttttttttttttttggagacagggtctcactgtcacccaggctggagtgcagcggcacaatcatagctcactgcagcctctaactcctgggctcaagcaattctgcttcagcctcctgagtagctgggactataagcatgtgccaccatgcacagctaatttatatatatataatataatagataaatatatatatatatatatatatatatatatattttttttttttttttttttttttttttttttttttgcagagacaaggtaggtcttgctatgttgcccaggctggtctcagactcctaggctcaagtgaacctctcacctcagtctcccaaagttctgggattacaggcatgagccaccacgtctggccagtgttaattcttcaatatttggtagaattcttcagtgaagtcttctagtcctgggcttttctttgttgggaggtttttaattaccaactcaatttccttactagttattggtctatttatatcttctatttcttcatgattcagtcttggcaggtttggtgtttctagaaatttatccatttcttataggtcatccagtttgttggtatagttcatagtcttctcttataatcctttcttatctgtagctcagtacctcctatctggagatgcagaattaggaattgaaactataataggccccccttttataatggggtgtccttatttttaccttctcaccttgcaatacccttgtcttgctagtaaagaaagaagggaaatttgattcaggaggtaatcatacttttcaatttgtacaagatctaatagccatgaactcctatgtcattcctcaccatcccataattcttagcccagccatcatccttacctcaatccctgctggtgcagcctggtttattctgttaatgtgctgtactgcattgaggtaaggacttctgctcagctttcttcttgataccattgtaccttgattcacacttcctcttgtgaaataaagtttagcatgaagctgctttcttacatattttaagttcggcttaaaggtttttctgtacatcgtgaactgtaacaagtggaatataaccagaccgtagcttacacttgtgccatttaccaagttttggccaatcaaatgtagccaactgtttgaactgtattcaaataagggaaatgctcagctgtaaccaagccaactgtttctgtacctcacttctgttttctgtatgtcactttcctttttctgtccataaatcatcttccatggcgtaggtgtgctggagtctcagagtctattctggctcaggaggctgcctgattttgaatcattcatggctcaattaaacttctttaattttttttttttttgagattgagtttcacccttgttgcccaagttggagtgcaatggtgcagtctctgctcactgcagcctctgcctcctgggttcaagcgattctcctgcctcagcctcctgagtagctgagattacaggcacatgccaccatgcccagctaatttttctatttttagtagagacagggtttcgccatgttggccaggctggtctcgaactcctgacctcagcctcccaaagtgctgagattacagatgtgagccactgcacctggcttcactccttcaaatttaattcagctaaagtttttatttttttctctttcttttttttttttttttttgagacagagtcactgtcacccaggctgaagtgcagtggcacaatctcggctcactgcaacctccgcctcccagactcaagcgatttctggctaatttttgtgtttttagtagagatgggttttcaccatattggccaggctgatcttgaactcctgacctcaggtgatctgcctgccttggcctcccaaagtgctaggattacaggcatgagccactgtgcccagcctcaaatttaagaagaaacagttaacatggacttgcatacctccaggatattgtgaatacctctcaatatttttctaagttctcaaagtcaaattagactctatgacaatcactcaaggttccctttgtttccaatatgttgatgacctgctactttgcaaccaaagcaaacagggtgctcttctggactcccttactcaccttaaggcactgactgactaaggttataaatcttccaggtccaaatgccaacaggtacaaaaaattcttacctacttaggccataaaatattttagggtactcaaaaactcgtcccaaaatgccttgaatcaattttattcattatctctcaaagacaaacaattacgtgaatttttaggagcaactggatattgccaatggattcccaattttgctgcccatgtctaacctttatatgctgtcctcttagatacaaccacagagcactttacctggtactctgaggcaccagcctccttggaagcattgtccacaccccagcccttcgactacccaactttgacaatcttttttacctatattactgtgaaaatgatgggattgttgtgggtatcttaggacaatctttttgtcccataacatatttctcatgtcaacctagatatgtcccacagtacctttctcatgttaagtagcatcaggcattcctccatgcttatatgcaatagacttagctgccatcctaattgacaaagcaagtattcttatactgccccaccattcacctctctgttctccatgctgttcctctacattggtatccctttcaaagtggatcttgcctcaactaacccttaactgttttttttttgtttttgttttttgttttttgacaattctggcactaccccaacacctgcttgttccaatctttcaaagcctggccaccttaaatagttaatctggttactggttaggttaacatctacataatgcagaagagtttttgttcctaccaatgtaaatatacctggtgaacccattctggacaatggatatataaaagcatatggtatccataagcaggaagacaaagtcactctgtctcctcctctggtagattaatttggcactgggaagcctccatggaagctcaaggtcagtgctttacccaagtaagactattggaaggaaatctctctacattgaaaataaatacagtactggaccttttctgggtaacatttcaaaaatgtattgcaatcaaattctgtgatttggcttcacagatggcactaaacaaccctccactgtcattgttacttggattataactaagtatttcaatgtgagtgaatgtcagattacaggataatattcctggtttgtaggaaaaagtagtgggatatggaatagctcaagtgttcccctagttggcttgaccagcacccatgactatagttggatggatggaccttaacttggtcaataaataaaatacatttctatagtaaccaaggctaaattaaagggtttctctgccaggtgtttcacaacctgttttaccctcatagcctaacagaagcacattggaagtgaagatgtgcagatgccaacatgattgatgataagggttgtgaaagacacagaattccaacttggttgttcacaggttccaccactatgaccttgtctgtaaacaacactggtctctctctctttttttttttttttagaaggaatctcactctgttacccaggctggagggcagtggcacaatctcagctcactgcaccctccaccttccggttcaagcgattctcctgcctcagtctcccgagtagctgggagtacaggtgcccaccaccatgcccggcttatttttgtagttttagtagagacaggatttctccatgttggccaggctggtcttcacctcaagtgatccgccagcctcggcctcccaaagtgctgggattacaagcgtgagccactgtgcctggcctggtctcatttttatgtagcaataagatatataaaaggttcccacctaagtggtcagagaaatgtgaagttggatatctggtgccttcccttaccagatatcccactttgaatgctagccacattacaactggggttcttttatatataaattaatgccatgtagatgcacctgatgagacatcatagacaacgcacttatgtattgcaaccctaagttctcagtaatgagaatgcttttccaaagcctggcaatgtacgatgtagaaagaacaatcctaagcattccaaagtaatgaacaagcatctggtgccactatacagactgggaagcctgccatttacaagttagcagtgtagcctctgttgcactccaaaattgtgtcctagatatgctgactgcccaacagagaggagcttgtacaatcactggcaacaatgctacttctatataaattagaaaggaaaaattgtgtctaatctatatcatttaaaaagaaaggttggccgggcacggtggctcacgcctgtaatcacagcacttcgggaggccgaagcgggcggatcatgaggtcaggggatcgagaccatcctagctaacatggtgaaaccctgtctctactaaaaatacaaaaaattagccaggcatggtggcgggcacctgtagtcccagctacttgggaggctgaggcaggagaatggcgtgaacatgggaggcggagcttgcagtgagcagagatcacaccactgcaccccagcctgggcgacagaacgagactccgtctcaaaaaaaaaaaaaaaaaaaaaaaaaaaaaaaaagaaaggtcaacattctacgttaggtaaataaggcatagtccaattaactgaactgaactgacctattcccacgactgggagactggttcaacagaatatggaccagtgtgttcagatttttctctgttgtaatctatgttcttctttcattttgcagatctcttacctcccagcacctaatatgagtcttttctacataggaaataatccaaatatttgtgaaacttcatgtgaagtttcaaatgggggaagtgaaggaacgaacaacccacctcctaaccccaatttatacccacctgtgttagttcatttgtattgctatgaagagatacctggaggctgggaaatttataaagaaaagaggcttaattggctcacagttctgcagggtgtataggcatggcatcagtatgtgctcagctcctggtgagggcttcagggagcttacaatcatagctgaaggtgaagggggagcatgcatcttacatggtgatagagggagcaagagagagggtcggggggtgccaggctctttaaacaaccagctctcatgtgaaataccagagccagaactcactcatcaccatggggatggcactaagccattcatgagggatctgcctcatcacccaaacacttcccagtaggccccacctccaacttggggattgtatttcaacatgacattttgaggggacagatatccaatattcaaaccatatcaccaccagaaaggcataaagattactttaaactgaaaatattggaacaaacaatcgctgcggaaagcagccttatctgaccgaaagcagacctgtccaagagttctgctatcatcaactccttctgagggactttccagacagcgaggtgacagatgtttacaaacgtgacgttaaaaaataaagttgtgtaaatgagtcttatcagaaccttttatactttctcactgaagcctcagttggtatataaacccttaccactggctgtttgggaagtgactccttacagagtgctccctcaggcatggagaataaacttttctcctgttaatgtattttcaactaattcgcaggccctagaccactcagatctaagttgacagatgaaatgttttcctcccaacatgaccaagcttatagtgcttttatggtatatctgtagagattgcggtcaggcataacattgtttgttagggttgcagtacctttcaggaaatgctcaaagtttaattgatttaggggactttcactggatgagatgcctctctgagtcatcataggttgcaaagtattagttttttgccactcactgtgtgttgtgatatgacatactcataatggggtaggacaagatgtcagttttgcttccaaactttccttacttgtttcctttttggttcaccactaatgttgaagaaatgcaagatggaaaatctcaatagttgacactgattgattgattgagatggagtctcactctgtcacctgggctggagtgcagtggcgtgatatcggctcactgcaacctccacctcccaggttcaagcagttctcctgcctcagcctcccgaacagctgggattacaggtgcccgccactactctcagctaattttttgtatttttagtagagatggggtttcaccatgttggccagactagtctcgaattcctaaccttgtgattcgcccgcctcggcctcccaaggtgctgggattacaggcatgagtagttgacatttattaagtgtttatatgtgataagcactgttagattatcccatgtaatacatcacttgattgatttaagagattgtcatttgaaagattaaagaatatttcccagaaaggatgcttggtcaagcctcatcatcctgggatggatgggaccttggttttgggcaagtttattacaatttaagactattctaggtcatggaagtgtgtgttaggacatataagtagttttcttgtccagaatactttgtaataatataccctaagtttgatcagctttttggcattcacttaattaaaatgttcacaagtaggtacatttttagaattgttaagtaatatactatttgtagtagcaaaacactacaaacaaatacctaatataataagagggagtggttgaataaactagggcatgtcaactaaaaaacatatttgaaatgcagggaaaatgcttactctaggcaatagttacaacttttgtccattataggtacataaaggaaaagagtacacaaagaattctattaatgatgaaattaggaacaatgttcccatccccaatttatacccaaaagaaaatatgttctggctgggcgcggtggctcatgcctgtaatcctagcagtttgggaggctgagacaggtggatcgcctgagctcaggagttcaaaaccagtctgggcaacatggcaaaaccccgtctccaccaaaaatacaaaaaattagccaggcgtgatggcacatgcctgtaggtccagctacttgggaggccgaggtgggaggatcgcttgagctcgggatgtggaggctgcagtgagcaaagctcacaccactgcactctagcatgggtgacagagtgagaccccgtctcaaataaataaataaataaatgaaaacttatattctataacatgtattcttatgtctttggctaaaacaaaagagaagaaaaataagtagagagctaagtgaagtgaagtgtcttgaaacagataagccataaagtgagatatatgagtaaatgagtagttgctggcctaggaattgtttctgatgttttcacctattgaaagaatttttttctttttgtaaatcttttttttggtttgttaaactgaaaaataaaagcaatgaagagataatattgctgtagtaatgtcccttagtgcatccttggagttagttgtcttgaatttggcctgctctgattgtcatttgctgtttgctgcattgaaaaaatttcagatttacaaaaatatgtgtgccagggtggaggaaatttttaacttgatgaattctcacctttaggacactgtctgctcttatatggcacttagcaagatgctgcaacaattgtccctgctcatactgttggaggaagagggtatttgcagggagattgctggagtcaagatgatccaaatttaaattgcagtggtgagcagtggccactagagggctgtgaagtacttaattctaaaatttccacattttaatctggagcagaggaaactctggaaggaccactgggactaagggagctcaatcccaaacatctttatctgagccctaaatgtcttctacgttattctttgacaatactttgttacatctcagaatttgtagttttgaggtggaggtttaagttagaaatagtttaatatattctattccagaatataattcgcttttttccaaatgaaactggcactaaaagctttttacttgaaagcaaatacacttcatatgctttatgtatttttgtccctatatcattgaaatagtagattcaaggctgtttgtaaaaataagtgactatactgcatataggaatagccccaccttaaagactttgattttaaggacattaagtgggagggtcttttttgcctttttttttttgactatcaaaatactttcacatttcttcaattcaaagaacaactgttctaaatttagaagacagacaagtgaaagagaatatgctgccatttccgatggttcttttttactcttgatccatcactctcctgtctttggctgactctttctccaaaaagtaccccttatttttcctatgcctttaacttctgttttacttactctattgtagaactttgagaagttgtacaccacattcactgctacctcacattaactctgcttactcattgcagtctgccttctgctcctcaatgattgctcctgtgaaggtcatctttggtttagcacttgtttgaaatctaatagcctaaatgcacatcgattactgtttagaattcaaacgacatttatttatttactttgagatggagtttcattcttgtcgcccagctggagtacaatggcatgatcttggctcactgcaacctccacctcccaggttcaagcgattctcctgcctcagcctcctgagtagctgggattacaggcaccctcaaccacgcctggctaagttttgtattttttttagtagagatggggtttcgccatcttggccaggctggtctcgaactcctgacctcaggtgatctgcctgcctcagccccacaaagtgctgggattacaagcgtgagccaccacgcccggcccaaatgacatttatttttaaaagcaactaaaccaggaaagaccttcactcattcaatcaaaaaacatgcattgaacacgtattcttggctagatccggtgctgcaaagatgaaagacgccactcctagcctcaaggagcttgcagtttagtggtggcactggatgtaaaataatcataagatgtgaggtgaagactgatgaggtctattttgttgacacaggtaaacattctcagagaatatttaattagcaacatgacaaaaattagttgatttatttgaaggatatttaagtgaatttagagatgagatttgtttttacttttttaatttcagagagttatgttggttgcaaaaatctttgttttctagtatctattttataagccatctgagaccaggatgttttctttttaacatgtaaacttgatgcagtctctttgtaaagtaatgaatccccccgtgaacctcaaggagaagaaagtttagcttgaacacttaatttcaagtaccttgagaagggaacaggctgtattgctcagagaagaaggctctattagctaaggtagaaggacaatgtaaaactcttgtgaagacacctaaatgtcattccactcaaagcccattattaataatttgaaactgtctgctctgtgaaggcaacgacctatctttactcatttttgactctgctaacatttctttttatagttgaactagaggcaaggcaaggaacttgacatgcttgttttccctttagaataaagtggccagaagcagtttcttctgtgtgatccaacactttcttatccccagagcaactctgcatagtctagatgtaccagagcccagcagcctgtgaggtgatgtgatgtgatgtgatgtgaacagaaaggctccatgttggatgatgcctatgaatctaatcagattctctttcttggtcattttgatttccagagaaggcagtagaagcaggttctgtgtgtataaccagagactagagggaggaactgacagggaagctgggtcatgagagtggtgtgctcagcagagtagggagtaagagagagctggctccagagaggatgacaaaatgcccatgtctccagcacttctttagcattctgagttcccatcctatcatgaataggaagagttttctagctctccatgaagccgaaataggtttcagactttcctttctttcccacacacataataaatacccatcaggtaacctgggcatggccttttatttaggcactaacaattctaaaaggaattaataaatgcttcactgccatttcacagtgtaacagcatgccagtttaccataccattaacatttagcctcgtggtatttctgtgttttttcagtcagtaatgatggcatttttgccaagataatatagtgttaaactgtattggttgaaatcctaggctttttaaatgtaaactagcactttacaaagtattacaaaggaaacgaaccagggaaacttgagaaggaactttcttatccacattgttataggttataaaatagttcctatttaaattaaaatacctactgttgcacttttatgtgtgtttttatatataaataacatctgggttggcaaatatgtgattttcgtcaaataggctttgattgaagatgaaatatttttgtaaaactagtccttttttaaagttaaaattttatgttaccacatgaattgatcagcagaaatttatttacattatgtaaattgatttttaagagtatccacaaggttttagctattatttttgaacttgcttcctagcccacacaattaagtaataagagtaagaaaaaagaaagcacacatccaaatcatctatcaaaacccagcttctacccaatgacacatcattttatttcttgatcttgtaatgttgagcacatgccttggacatattcctatatgtgggctctattctctgcagcacgtcactccctcttttatccgcccctcttatgtgctcccactcctatcctcttcaattaaaaatgcctctttcttttttttttaagttaattaattaattaatttttttttattgatcattcttgggtgtttctcgcagagggggatttggcagggtcataggataatagtggagggaaggtcagcagataaacaagtgaacaaaggtctctggttttcctaggcagaggaccctgcgggcttccacagtatttgtgtccctgggtacttgagattagggagtggtgatgactcttaacgagtctgctgccttcaagcatctgtttaacaaagcacatcttgcatggcccttaatccatttaaccctgagtggacacagcacatgtttcagagagcacagggttgggggtaaggtcatagatcaacagcatcccaaggcacaggaatttttcttagtacagaacaaaatgaagtctcccatgtctacttctttctacacagacacagcaacaatctgatttctctatcctttccccacctttccccctttcctattccacaaaaaccgccatcgtcatcatggcccgttctcaatgagctgttgggtacacctcccagacggggtggtggccgggcagaggggctcctcacttcccagaaggggcggccgggcagaggtgccccccacctcccggatggggcggcggctgggtggaggcgggcccccacctccctcccagacggggcggctggccgggcgggggctgaccccccacctgcctctgggacggggcggctggccgggcgggggctgaccccccacctgcctccgggacagggtggctgctgggcagaggggctcctcacttctcagacggggcagctgccgggcggaggggctcctcacttctcagacggggtggccgggcagagacgctcctcacctcccagacggggtcgcggctgggcagaggcgctcctcacatcccagacggggcggcggggcagaggcgcttcccgcatctcagacgatgggcggccgggcagagacgctcctcacttcctagacgtgatggtggccgggaagaggcgctcctcacttcccagactgggcagccaggcagaggggctcctcacatcccagacgatgggcggccaggcagagacgctcctcacttcccagacggggtggcggccaggcagaggctgcaatctcggcactttgggaggccaaggcaggctgctgggaggtggaggttgtagctagccgagatcacgccactgcactccagcctgggcaacattgagcactgagtgaaccagactccgtctgcaatcccggcacctcgggaggccgaggctggcggatcactcgcggttaggagctggagaccagcccggccaacacagcgaaaccctgtctccaccaaaaaaatacgaaaaccagtcaggcgtggcggcgcgcacctgcaatcccaggcactcggcaggctgaggcaggagaatcaggcagggaggttgcagtgagccgcgatggcagcagtacagtccagctttggctcggcatcagagggataccgtggaaagagagggagagggagactgtggggagagggagagggagagaaaaatgcctctttcaatatgtaaggtaagattgatagatgattgccttccgtagttcctcccaaaattcataggttgaaatcttagccctcagagtggtggtattaggaagtatggagcctttgggagataattagctcaggagggtggagccctcccgaataaatttaatgcctttataagcaagaccccagagagccctttcacccttttctaccctatgaggacacagcgagaagacagctgtctgtgaaccaggaagcaggccctcactacataccgaatctacaagcaacttgatctcagacttcccagtctcctgaactgcgagatataaatgtttgctgtttaagtcacccagtctaaggtatttttgttatagcagcctgaatggactcaggcggtaggcaagaggaggacagtgcacctgagttatacattgggcaagtcatttaccttcattggagcctcggtttacttgtgttagatatgggaataatgatagttacactgcagggtggttgtgaagattagagaaagtgcatatactctgatcagcacagtgcatggtacttcagtacacagtgttaactgaagacacagtgttaactgaagacacagttgaaaactaaagatagctagtgaaacacatgttctctgcacatcatacagtttcttgggcagttttcaaagtgtgactctgcagttcataccaccattatcacttagtctctaacaaataatcatatttgacacatttggctgggacttaataattttatttgggcagcagctggtttctggaagtgttcatgggaagaaaatgtatattaataaagttagcaggtaatgttctttgttgaaatgttggatattgtgggacacaaaagagtcagggtaaatgtacatttacagaattgagcgtcagagtgtcatagttctctaatgatttacaaagaaagaattcctggaacaagtgaaatacttaataattaattcagcctgtatttctgcaggtaatcaactgcagtgataaaaaaataaaaatggaactgtcttttgctcattggaaagatatttgctgcattcaaagtcatcaaaaaggcgaagcaatgaaacttaagacttttgggttttaataattaaaaatccatcttaaagagaaccttgggctctggcacggtggctcattcttgtaatcctagcactttcggaggcccaggtgggcggatcacttgaggtcaggagtttgagaccagcctggttaacatggtgaaaccccatctctactaaaaatacaaaaattagctgggtgtggtggtgtgcgcctgtaatcccagctacttgggaggctgaggcacgagaatcacttgaacctgggagatggaggttgcagtgagccaagattgtgccactgcattccagcctgggtgacacagtgagactctgtcttgaaaaaaaaaaaaagagagagagaccgtttgtgaaggtgtgttacacagagaattcctgattcctaatctccagaatagaaaaattcaaaggctcagaatcatcccaaatcaattatccagtggcatctgcattttccgatttcattctcactagccgtgtgaacatgggcatgaccccaggagccaaggaattctctaatgcctaaggacagccatgaggtcaatgaataacatgtgtcaggtttccctggcacagaggagcttcccagtaaatgttattttccttagctatttcccatttaacatgtcaattattcttagtgagtttccattcaatatgagagtttatataatttgtcatattgaataggaacttgctaaggaaagctgtgtagcagaggaagcagccccaagtgacaggacataaactttaaattcacaagatgcttgtatgtgaattatgatggtatctgaattaacagtgatatttacagtttagtaatacatttttcttcccttgtcttgggctttataaaaaccctgtaagtcatgtatgtcaggaattttatcctcataattgagagaaaaatactccatattttattggaaataagatcagtagattctctgtatatcatacaatgtcttgcctacttaaattatcaccccccttcctatttcaacaaagactttctctaagtacccctggcctcttgccctgatccatactgttctccttggtaatggagtgagtttcctgcctggtgggtgcagccattggccacatttctctagtgtatggaactcaccggataaaaggcctcagatgtaggtctctttctgctgtcttcacccaggtgttgtggagtgtgtctgtccttgagcactagctttcccctgtgtgggctgcctcaaggcctgcattcatcaggtagggactgttagctggtagacctaagccaccactccagtactgactgtcagtaaggaaggtgacatgctgacctccatctgctacatcattgtgtatatgtcttcattagttctgcatattggtgagaaaatggatgctctgattcctcttgaaccccaagagaatgaaggtaaaaaaattgaggtcctaatgcaaattttcttagtacacccaaatctttggatagagtcctgcactctttgagatatatcacacaatctgtctcactttcttttcgcatatgttatatattttaaaacttttgtttttggggccaccacttactggctctgtgattttaggaaagcttttcagaccctcagaaccccagtctcttcatctctaaagtaataaaatatatgtaaagaacctatttcagcatgtgaattctgttttcctttttcctctagatgtatcatatccagttaaaaaaaaatctacttgaactttgcaggtatcttcagtgtttattacttctcatttttaacatttattggaaattagcatattgtcagaattgatataatacaatatgtaacctctttcattaagcttatcatttttaaaatacaaataactattctttacttaaatttttatttctagacacagggtcctgctctctcgaacccaggctggagtgcagtggcacaatcatagctcactgcagcctcaaactcttgggcttaagtgatcctcctgcctcacactctggagtagctgggattatagacctgagccatggtgtccagcatgacttaaattttgaataagttgcacttactaattacacttacactgctgcatctgaaagagtaatacaacaatagaagccttttatagtaattatttgtggcaggtagactcctaaaatgactcccaaatgacccacacccttgtacaatcaataccctgtcccttgagtgacagtgacttgctctaatcagttggctttcagttaatcaaaagagagattatcttgggctgaactaaactaatcccagcaagataacagggacttcagtcttgcaaacagatatcatataaagggaatcatatctgcacatttgattcttggaccctgggtaggaatttgttagagagcaaggatgtgaataaaggtgggaaataaaggtgtatctggtgtctctgctcaaaagctcacatgtagctacaaggcagagatttaggggagtggtatccacagtcaagaagaattaatacatagtgtttgagtctggcttcttccaattagcataatgcttttgaggttcatccatattgttgcattaccagtagtttttatttatttattttatcagtagtttctaaattgttgagtagtatattacattgtgtagatatatcctgtgtgtttatccatacacatttatggatatttgggagttgctagtttttagctattctatgagcattcacatacatgtctttgtgtggaaataggttttcatatctcttgggtaaatatacgggagtggaattgctagatcatatggtaaatactctgtatacttaaaatgaagagaaactgtcaaactattttccataatggctctaccatacttgatgttttagaaaagaggaaaaacactagcaattttgatgctgtatgtctacaacctaagagaatctaataatagcgtcctggtctgtcagtgtaggaattgcctaggtaatacatggaaggtgtggagggagcaggtacacagaaaatgtgcgtcagaaagttttgcttttcctatcccacgtcatttctgagtctgatcctccctactcctcacaaataaattggtagattcatctgtttttggacccttttctgctctagttactgaactatcagagacttcaggaagagcttaagctaagctattccagggaagttttggtgttactctgtacttacggactcctgcgtgtctgtctctgtcaccccagctgccaactcaacttagagtttattagcctggcattgaccagcacactgtgatattctctgaggcacactgcatgctgctagtgtgccctggttcataaagctgggccttcagcattgatcccactccaagttccttgctctgtcttcccacagctgtccccttgggggatgtggggggtctgacatcatttgcattattagtctattccaagaaatgcacctgtgcactaatcagttcactttttctgtcttagtcggcagatctagccatagcccaatccctcaatttctatactaagccttttatattagtaaaactgttatgttatctagaaattcatcagtgggaaaactacttcaagggaggtagttagaggctgcaaggtgctaaatatttttctttctttctttttaaatgtaacttggatctaaagtaaggacgaatttccttttattatttgttcagaatataccagctggtcctgtgggcagaagtttgttaaggggcctggatgtgaaataacagtgtatctcgtgtctctgctcaagagctcacatgtagctacaaggcagagatttaggggagtggcatatacggccaactgagaaataacaatattgtcagggactccaaggcactttggaagatataaagaatttcttaaattttcttgtagaattgttgcaaaaggcagacatgcttaaatgtttaaataagcttcttgaaaactcatggaacattcaatcacaactccaacagttctccaaaatttgatttattctggccatattatgcagcaaagaaacacttggctatttatctaaatctcttctgtcttgtaaatgatcctagaaaataatctagaaatacattttattaaagtaatgcatgaggtacatatcgattaccagccaatagttgaacttaaacataatgcatgggtgtgagggctggcattgatgattcacaatgaacacagttgaatatcacttccctgctgagactcgggtatcatcgcaaaaccacagtgagcatcagtggggatctgcatgctctggtcaagacagatctccatgctgagtgtctgtttgccatgatgaagagaacagtcaacaggagtgtttgccatgatgtagagaacagtccgggaggagtgaatggaggatgggggcatgaggaaagatgaggctttctctagttatgaccctttgtgtagaagttaggagtaggggataaatgtttctgcctaatatttaacttggaagagaagatgtccatgtgaaaaactgctaaatactgaaacaagagagcatgtgactaagcaataccatgtgtggcacagaaaacaagtgcaatagcagtttagcaaagtgagttcagtgtaggctgaactggttagagcaggtttccgggtgaaggtgaggattggtgagggtttggattggtagaaagagacggggaggacatctcacatcaagaagttatgccagtggatttcaggagaattgagtgtttgtgtctgaaaagcctgtaagaatagggcatgacagtgtggagaaatgcatgaaagtatgaaggatcgtgatatccagtttgaggagtgctaactagaggctctgaagatttgagaagaaacataatgaaaggtgttctcagcctgatcttggtatgcaggactggtaaaccccaaacaccttaccattctattacctctccctcaaggaatgggtcccttgataagaatttagtgtaaaaaagattgtcaattcagtgctgctgctgagtgctagtttctttaaacacacacagttttcttttgagaattttttttctattagatagacgaactgttatttaaatgaaaaaggcacatagtcccataaaacaattacacattcgggtgataacttcaaaaggagaaattaaaatgttcttatgttttgagcaagcatttccacttccagactttgctgcataaacatctgtggtcatctagggaatgcctgacctggttcagaggtgtcagagcaatgtaaagtcacggaagtgctgcagttctattctgggctctcatctttttgcagcggtccattctctaattttcaaccacatattaccagacaatctcttaagtcatacacaacaaactgattctgtttcaatgcttagaattagaataaaaaagcctaagcaaaaatagcacaaacatttgaaaaacactccttttttctaccactcccttcttagaacagaaataaaagccctgtactttaagaaaatggatggaagaattttctttgtacttcttattctccaagttacatttactacctgatagtgttaatacctttttgtagtacctttctttaaaatatacagggaaatgatctgttccaagaaactgtgtttttaaatttaattatagtgtgctatgatgatttaaaaaatggccttttgagtaaaggacacgaacaagttatttaaaaagtgagcagtaagtgtggtcagtaaacacatcaaaaagttcccttcactaatattcaaagaaatgcaaattagaataataatacccttgttgcttgtcaaattaatactttaacaattattatgtaaattttatggataggattgcaaatcaacacacctttcctggccactggtgtacataatagaaattctaaaaatgttcttaggcttgaccaagcatttccacttctagactttgctgcacaaagatctgtggtcatctaggagaaggcttgacctggttcagaggtatcagagcaatgcaaagtcatgaaaatgctgcaattctatcctggactgtcatcttttttgtagtggtccattctctaatttttcaatgacgtagtaccagacagtctcttaagtcaaatgtatttgtagggctctggatttgaaattcaatctggctttcagccttgatgtggccactcccaacttgtaaaggacctgtgaagacttagacacagaataaaacacagaagataagaaaaccaactttgaaagaaaatttattgtcaaaattgtactgggtcaattgagcaaaaacttcaaagagcgttttcatattaaccaaagcatccctcctcaattgaaacatataaagatattgttcacccctatcctgactcagagatccacaaatctgggcattcatcatcaccatattctgctggcaatagttttaagcagctaaattactgttctctactcttgagtttcctccatctcttcagatacagaaagttctagaatatattcaaataatcaaatctttaattcattccatatatctggctcaagacagtgtcccaataaccttattctagagaaagtcagatttagacttgtgctcatcatcatactcatgttcttgacatcattttaagctctgaggagacatctcacataactctcattgatacgtgtatacatctgtcactctgtgtttgtgctgtgatggatggacttggatgtagatatgcatagatgatgaagcagatagctatatatatggtattgatgtagattcagtacagctgtataattgcatctgtgtttcacatatcttgtgtactgtatcttgactgtatctgtgtcaatacctaattgagttataaggcataaatatgtggagctcttagcacaatacctggcacactgcaatcagtcgatgtatgtgtttgtgtgtgtgcgtgtgtgtgtgtgtgatacagacagaacctgctaatatgcataatagtcaggttgggttgttataacaaaatactatagactgtgtggcttaaacggcagacatttgtttctcacagttctggagtctgggaaatccaaggtcaagattagtttctggtgagagcagtcttcctcttttgcagctccccatggtttgcaaatcacagatttctcgctgtattctcacatagtgtaggaggaacagagggagggaagggaggaagtgcctaaggacactaatcccatgatgagagttctatccaccatgacctaattacctcctaatgccaccatctccaaatactatcacactgggaattaggtctttaacatgtgaatcatttggggtggagaagacaaacattcagctcataacaggtaaggtagaaaatctcaagaatttatattttgtatatgaaagatcattaatgagcagaattttaagtttaatgccaattttaatctatttttatcttttctacgattcttttttactttttaatttttaaactttcatatacaaagggataatatttggctaaatgttctcttctttttgagctctggatcattgttacgatcaccccataattgtatgtgtgcagagatagtgctttatacatttttaaaacaattttatatacagtattaaattttatttttcaataaacaatccatgagatagaaagaacatatattttgttttacagataagctccagggagagtctagggtaccttagattgtatgggtaaaacatggtttatttaaatcataaataaacagtcttatttccctaaatgcacatacaggcatccacatcaaatgaaatcacatcacatgaattgaacaggcagttactgacttagaactttgcactcacaaaagacacactctcctaaatgtctccatcatactatactttttgtccccaaatgcctaatcactgaagcttcagactttgttgctttgattcccttaggaaaaattcctggtgtttcagaaaaaaagagccatttaactacattagaagttaaccctcctttaaaaatgtg

SEQ ID NO: 20 - DNA, 26803 bp, Homo sapiens
cagttaaggtggggcaggaataaatcacaatggtggaatgtcatcagttaaggcaggaactggccattttcacttcttttgtgattcttcacttgcttcaggccatctggatgtatatgtgcaggtcacagggcatacattggcttagcttgggctcagaggcctgacaaggcacagaaggagctgggatagaggtgcaaagtactcatgctgacctgacatcccatgcccacggcagacatgactacttgatcggacaatactttcttggaatcaaagacacaacttcacagtcctcagcatcatagttcaggcagcctgtatcagtagatcagagtgggcacatggcctggtgctatcactccatcctgtgaggggagatgggattggaatggaggtggaggagtcacaggtggtcctgatatcacaggcctgggagtctgaaagaagtgcagtaggtagtattatggccctcaaagacatctgtgtcctactgtctagagtcaattaaagtgttacctaacatagaaaaaaggattttgcaggtgggattaaactaaggatctcaagatagaaagactctcctggagtatccagttgtgtccaatgtaagaacaagcgttctcaaaatagggacacaggagattgaattgcaaaggagatgtgctgataaacggagaggttggagtgatgccgccatgaggcaaggaatgtgggtggcctctagcagctagcaatgattcggaaatggattctcccccagagtccagaaagatcacagcagtgctgacaccttgatttgagcccagtgtcacctctgtcagacttctgccctatagaactgtaagaggataaatttgtgttttaaggcacaaagtttatggtaatttgttatagcagcaatgggaaactaatacaagaagggttgtgttatcaacagaaatacagcaatcagaagaaagatggttggggagagcagagggtggggtgggaaggtgatggattctgtttgggacattctgggtgtcatatgaatattattggggaactgtccatcaaaagctcagacttcaaagaaagaaaggaaggagcaacaatattttgaaagggagaaagtaggtaatattcaatatgtgttgagtacctacaaggtttttagttctttcaccaagttattttatttaatttttatggcatcaaggggtgttttttttttttcttaaaccaaattttctcagttaagcatcccatgtaagtggccaggggttaagagatgtgactaagactagacagagtgattttcatcattacatggtactatggttctactgaagcactgaggaaggaagtcaagagagttcctgagaaatgtctggagtcttagtaacatgcaaagtgaggcagaggtattgtcagtgttagctggtcactttgaaaggttagaggtaaataaagttcagggcaatggtacttggagaggagtgaatctttggtaacctggaggagatgcttctcagaggaaaatttcttcacagcatgaagtcaccagctctaagactagtgggtgttctgggggatgttagcagtgactcactgactgttggcccagtgaggggagggatgaaaggctgggtagtgggtagagaatctgactcctcctgcccccacatgtctattcctgggccttctcttggtgggggcaaaaggtatgcaaagggatttccgcagtgtctgagtgctcccaggagacggaaaagtaactgatgacttggagttggagtcttgttggctcaggcagctggggcgttttgggatttcaacacctccctttagtttctatgtatggtgctgagcaagtagtcaaagactttggtcttgctttaccccagtagcccacaagcctgagtacatggctaacatttattgggcacttagtgtgtgccaaagagctttatgagacaggttctttttgagtcccattatactgataatgggactgataagaaacagaaggtcagaaaggcccagtaacttgggcaaggtcatgtagctagtaagtggtccagctgaaatttaaaaccaggtttatccaactccaaatcccacatctgatttattttgccatgaattaaaacatagttctgattttgagaaactcccagtcccagtgggaaaacagatggaatcacaaattaccataacacagtgtagtgatgtagatataaaaacaaagacatgggaaccctgaaaggaagttgtaacaccaatagaggaatgcatggaggagatctttcagaggaggtagcctcgtagctgggctcaggggtggatgagtttctggctagaagcgcattgtgggtagagggagaacatatatagaaaggcatgaagatggtggacatgtttggaaagagtgagtactagactgatgaacacgatgagtcaggagcttatgacgtcaggggctactgctagcctagctaatgactgaagattctgtgaaaagaaaaccctaacatttccagctgagtactagggccatggtgattatatatcatctctcatgacaacacaaatgtttgggcttacttatcatcctgctcagtaatcattatgtcactcattaaagatgtatcagggtaaattttaggtgagaattgattagaaatgtaaactctatatatgtagttacaggcttcacagtttgccactcaaacaatatggtcatccaatcatgaggcacaaccttctgctcagaacttttttataattgggagaaagtgacatccgagttccatctcttctgagaactgtgcagctcagaaatcttcttcccttttttgatcccccagttgggtgagatgacattaacagtgtgttataagcacttttcatgtttactaccccatattcaaaattaagcatttcaaacaactgtataattgtctataaatgtagcattattagttaattttccttttaacacattgaggttacctctaatgttttgctatttttaactatgttgaaataatcatgtggtttttattctttgaattattttatattgtaatgttccctgaaatgaaattagttgatcaaaagatgagtaatcttttcatgacttttgatacatgtcactcaatcaccttctggaagagttggaacaagagcctattgctggcatcccatttcatagccatctcaccaatgttggaaaatgggcttttcctattttctgctaattcattagttgttaatggcttattttaactattaatcccttgttattgatgaaagttaagcattttctgtatttttattttctgtctaaattctactttttgcacaatttcctttgctcacttcttcactggaatttagtatttttctttccaatttgtatgactccaaaatcagtgataaaataagcaaagggtctttcttagaggctaaacaagggaatgaataaggaacaagaacagcaaagggatagtgaataaagatacaaaataataacttatttttatttttgaagctttccccaggcagtaattcttgacctttttaagattataaattattttgagatatgcattcttatcctcaaaatgaattagtacataaaatttaaatgggttgatagatcccctgaagtgtatccacaaaatgctctcaggttaagcaacattgttctataataactgctttaaccaaaatgtttaattattgcttgtgtttacctgtcctagcaaagagctaattgttaaattttgtgttagagggtcaatattataaataacttaatgtggcctctctttcctttcctttttttgagagttttgaggctatcactaagtgggctttagagtaccaggtgggaatctgacctcactgctcaaactttcaacttcaggcatgaagtggtcccagtgatgtgggaacctcagagtctaaaacaaaaatagtagactgaggccctcagaaaccagacttatcagattcagaatttaatataactatgtttgaaagatttaaagaaaataaatcaaattaaaaagtgagcaagaagcaagaataacaaatgaactggcatatttgagaaagaattttgagcttttagaaataatacatacacttattgaaataaaaactcaagtcaataggtttaaacagcaaaatgaatatagttaaagaaaactattgtgctgaaagatttaaaaaactattacacagaatgcaaaatgatgaaatagggtaatttaatatatggcagatatgttaagacactatgaggatagtatgagaagacctgatagacatctaatcacagcaccttaaggtgaaaatagagagagtgcaccaatattgaggagttaatgtctgagactattccagaactgataaatagatgaatctacagatctcagaaacacagcttttacaaaggataaatgaagagaaattcaccagagatacattgtaatgaatctgtaaatcaccaaagctaaagatattatttcacaagtggaatgacagctgacttctcaacaacaacgaaagcaaggagacagttgaaagacatcttgaaaatggtgagagaaaaactaactgttaatataaaattgtgtacctatcaaaaatatcttttggccaggcgtggtggctcacgcctataatcctagcactttgggaagccaaggaacgtggatcacttgaggtcaggagtttgagaccgagaccgtcctggccaacatggtgaaaccccatctctactaaaaatacaaaaaaaaaaaaaaaatagccatgtgtggtggtgtgcacctgtaatcccagctacttgggaggctgaggcaggagaatcgcttgaacccaggaggtagaggttgcagtgagctgagatcatgctgctgcactccagtctgggtgacagagtgagactgcctcaaaaccaaaccaaaccaaaccaaaccaatctttcaagaagtacaccataaagacatttccggataaacagtgaatgagattacttcctaaacgaatatgtaaggatgtttctttttaaaattttttttgggtgtattcatcacctcaagcatttattcttttgtgttgttacaactgataagaatatctaaggatgtttcaaaaggaagaaaaatgatccctaaagtctggtatattagtttcttattagttgctctaagaaattactgcaaacttagtggctttaaaaaacacgaaattatctttcagttctgtaggtcagaaatttaacctcctgatttctggtcagaagtcttactgggctaaaatcagggtatcagcagggctgctggaggctctggagatgatgtttctctaatttctagaggcatttgcattccttagctagtggcttcttcccacatcttcaaagctaacagtggcagtcgagtccttctcttatcttttttttttggggggggttataaattttttttattattattatactttaagttttagggtacatgtgcacaacgtgcaggtttgttacatatgtatacatgtgccacattggtgtgctgcacccattaactcatcatttagcattaggtatatctcctaatgctatccgtcccccctcccccaccccacaacagtccccagtgtgtgatgttccccttcccttctcttatcttatcactctgacctcttctgcctcctttctctacttttaaggacccttgtgattagattgggtccacctaaataatccaggataatctctttattttaaggttagctgattagcaacctcaattccatctgtaaccttaatttcttttttgccatgtaacctaacatagtcacaggcccaagggaataataggatgtgggaattgcgggtggtggagtaggggcattattctgcttaccacaggggaccttggatgtcagtaaaaaatggtgaggaagaaaacaggaaacgtagaataatctaaacaaatctttgaaaaataagttgaaatgtggggttagaaaaagggcagaactaaaatgttaagacaaattaaaatgttaagcctataagttgagagggagatgatcaaggttaaaaatactcataaatcatatttttttgggtagggggttagatatttattaattttagaccctgagaagtaaaatagtcatgacaaaaatttaatagtaaccactaaaacaagagaaacagagtatataacttctaaatcaatatgggaaggggaatggaataagaaaacaatagcaaccaccaacaccccacccaaaataaataataaggtgagagagaaaaagaagcattgaaaaggggctaaaataaaataaaaaattaagtcatgcccgtaatcccagcactttgagaggccaagatgggtggatcacctgaggtcaggagttcgagaccagcctgaccaacatggggaaaccccatctctactaaaaattcaaaattagctgggtgtgggggtgcatgcctgtaatcccagctactctggaggctgaggcaggagaatcgcttgaacccaggaggcagaggttgtggtgagcagagattgtgccattgcattccagcctgggcagcaagagcgaaacgccatctaaaaaaaaaaaaaaaaaaattaagatagtaaaacaaatccaaatacattaaagattacaaaaaatgaaaatgaactaaacttcctagttgaaagacatattgtcagattggattttaaaatctggcaatgatatttccaggacacagtcctaaaatattaaacacagaaaagttgaaagtaaagggatggaagaacacagtcaaactaactagaagagagctgggttcacccttttatatcagagcagaatttcactgagaaaacactaacaggaagggggaaaggcacaacatagtgatgaagcacttaattctcaacaaatgtatgacacttctaaactattatgactgcaaaaaaaaaaaaaacctcagcatatataaaattttggaagagccatggctatcagctgacatgcacttaccatatttgcattgtcctactacaaactttacccatatgaccaaggtgctgtcttcatccccattttacagatggggaaatttccccatagagaaaaagatttgggccatgccttggtttcttcttgactctgcttcctgctgattgatcctcacacctcacctggagacctacttcacattatccatcaggatgagaactggtgtgcctttaccaaaggaccacagtcaccttcaaaacgtgtttagatagatctggatggagacttatgtggttgcagatgaaaaaaaagtccccatggtatatctgactccatgtcattcactgcatgaacactcacacacatgcacacgtacacaggcaaacacaatcctgttctggtccggcagtagtgccaacactcaaatcccaggtcctactctgaagcctttgaggaaaccattgtcattctggggtttatgggaatatttcttcttggtgccccttgttcctcacagaagctttttttctgtgctgtgggcttgctatcctagctttccaagctatcctagttttgcaaatttctctgatcaatcacatcaggttcttggatcatcccaaaattaaagaggtacgttttgctgcaagagacaaagacattcacctctcacacagtttgaattcctgggtagaaacagatttcaatgctggccagcctctgtagctcccagtgccccctcaattatgactcccgaggcattggagcaggatcctcaccttgcgcaaagataattaggtgtgctgaagaaagccagacactgctctttcttagctctgcatccttaaaaagttaccactactccttctctttgaatctttgacttgtcaatggtaaagtgcctatgattcttaaagggataaaaacgcaacctatataaagcacctggcatagtgcctggcacaggtgggtgtttaacaaatgttaactcctttctatcccactgtgggtgtccatatcctcttgggtaggctgcctctggtttccattgtgtcatcagagccatactaaatcgatgtgttggacatggatcccaagaactaatttctggaatgagttatgcctaccaacttccctgatacttacttctgtctctccatttatcaaatggaaatgtttgcatttggcctctgccagttggagtaaccaaaaggcttagaggttttggagaggtcctacactgccatctgtttgaccacatactgcctttcacgtgtaataagcattgtttcttacatttgtctaggaattagcagttcacaaagcacattcgcatataagggcttgttttgaattgatcttggcagcaattctatgagacaagtaaaaggtaggtcaagcattataatcctcattttaaatctgggaaaactgaatctcaaaaaggttgaaagacttgtctaggggacagtgtgtgggtaaatgagaagttaagatttgctgaactggcatttcctgactacatatctagtgtttatttatggagaaggcactacggtggccaagtggctcagagtcacacagctctgtgcctcagtttatttgtctgtaaaatgaagataataatatattctgaatactgttgtggaatttcattgagatagttcacataatggcatggatactgtagtacaccgcctagattcacaaccccacgactatccatgagaatggcccatagctcaagaggtcacattctttccccaggtgaagcccgcatccaatgactgctcagtgtgggtatataaaggcctggctcccttgccagtgccaccctacctcctggcgaatggactgaggcttgcattatgactgcattgcagctcaactgttctttccattcagtctttcctttacactcacacaggtgaggacccagccattaaatgcctcacatgatgacctctattgcatgctaggcttcgtgtgcacacacaaaaaccatcctctatcagtcaggccccttacttgcagaggcaaagaggccagtctgggttagatgtgcaccctgtttttacaacagaacgagacaaacaggtcctccttaggtgtaagttcatggccttggccccacccctgaaactcagccatctgagacagttttaggactgaggcaaccccagactttgggttgttgtttgctgggcacagcctccttttgccaatgttgcaatcctttgtaagagaccacaggttgatcacccgttcctgttactgagcacagagaggtttgtaggccagtctctccaggaattctgacgcactgcaaaatcccatggtctgaatgcttctaccttccctgtgaaagcccctggcctcagaaaaggaagctggtttaagtgaccaacatttggggtggagcttccgagggcccagccaccgtgttacatgcaacaatcaacagagatattctttggctagagttgtttttctgggtataggaccctataattaaaatcagctctccaacttcccttcctccaaaaagtatacaatgtaaggaggaaaatgcaaattgaaaagttgctagcccttcccgccagaatgccaccccaagcctcccctgcaggaagttctggagtccccaactctgccccaagcctgaggcccttgataaggtaaagggatgtgagtgtggaggccggagcccccctcgccctgtaggctgctccccttgcttttccctttgaatgttacagtttagttctgtgacttacttataattgcctgaattccccgcccacgctttctcttactttggggcttctcaccgttcctcttcctccatcttcctcctctgaccccactcccaagcctgaatggggtgttcctcttccgtgctcccacaaaaccctgtgcctctttcatcgttgcatatattatgctgtaatgtagttttctggaggtgtgaagactatgaatcctatgaagacaaatacacacctaccttgctgaccgttgtatcctcagaatctaatactgcacttggcacacagtggttgggagtaaatattcatgaggcaaacacacaggaaggactcttttgttatggttgtttgttgttgttgcaagtaacataaccccaccttgatctagctgactgacggctctaccaccttgtcttttgcagcacaagaggaataggaactgcacctcttccttcagtttcagcttgaataatatcaggaagattcgtatcggtctgagttgggtcacgtacccgacgtgctatagctgaggatggggtaagctgattggagtttgcaacactgttcacatagccaagatatggaaagaacctaaatgtcaactggtggatgaatggataaagaaattgtggtatatacatacactggaatattattcaaccttaaaaagaaggaaatcctaacatttgtgacaacatggatggacctggagggaattatgctgagtgaaataagacagacacaaaaagacatttcttgcaggagctcacttatatgtggaatctaaaatagtcaagcttaaagaagagagtagactactggttgtcaggagcaggagaaaagtggaaatgaagaggtgatagttaaagggtacaaagtttcagttatacaagataaataagttctggaggtttactattaatatatcacatagtacctataagtaacaatactgtattgtatacttaaaattgctaagagggtatatcttatatgttcttaccaataataataataatggtaataattaaggggcaggaggacacttcaaaaggtgatggatatgtttatggccttgatggtggtgatggtttcatgagagtatacttatccccaaactaattgagatgtaaatattaaatatgtacagctttttgtatgtcaatcgtacctcagtaaagtagtttaaaaatggttggactgagaaaaggaggagctgctcagcaacatgaggctgggtgctgggcagacaaaacctcacacatgcattactgaacccacggactcatgtctgtgagctttgtggctgtggatgcaccatgccaatgtagtcaaggattcttcaatgtgtaccttactggattagttccctctgtttatttgtattgactcctcagttcccttatgggttgcttgttggctcttgtggaattatttaagtaaggctttggttgcaggagtcagacatgcttaagctggttttggctgtaatggggaatttgtgagatgtgacacagtgacaggaagtgcagccagacgttgtgagaggcagtaactgggaataggaaagttatgagaagttaaggcagtagtaattgtttctctatcgaaggccataatgttatcattcctgcctctatctgtttgcttgttcttctctctcagcagaatggtcttctctgcttctctgtgcacctgcagaaggtgaccaccctaaggcttatggattcaggagtcctcagtttgagagcagttaccaaatgcctcgcccctgtgaactctagtcccagtttcttattcctggtactggcttagtttgaggcagctgcccaccgtaagtccagtgagccatggcctggggacaaggtcaggtacatgtgtaatcagctgggtctatgagttgtggtggtggcgatggaggtagctcccagaaaaatggattacaggttaagaagagtctatatatcttgaccacatttgatgtgacttggaagtttcaatgtgtgaccacttacaaagttatgatcaggtgtctcatttatttatggtgatgtatgagtccgtgtgtgagtgtgtgtgtgtctgtgtttgtgtgtgtgtgtgagagagagagagagaatgagaatatgagtggtggtttcccatttatttttctatgggccaaatcctgggctatgagctggagatataagagtaaacaaaatagacacggtgcttgctgtgacctgccctgggagacagatattacacggaggatcacataaatgcagagtctgagctgaggtcttaagggtgaggataagtaactagtcagtggagcaggggagggaagggtgttccatgcctgtgtcaaggtcctgaggtgagagaaagaggtgaatttgaggaaccaaaaggagttcagggaacaagaggggctgtttcacaagctgagtctggaagctgagcaggctgagcagattcttaggaactctgcaaaaacttaagggcttgtctatgaccgtaaacaactacggtcgtagataaacaagttggcaaacaactcaaggatttacagtcatcagaattgtaaaactgatcccatgtattttcaaacctcaaatcccttgctctgaccttgtgtgtctaagctagaaggaagcaggatgcacctctcccctggctggaatgaagggattcacccaagctctcagtcttctcacggcatccagggcccccctgcttgtgtgtggtctagatttccattcccatagtaggaattcctttgggagccttggggtctctcctgctagagggcttcacctgtgactgtctcaattcaagggaggggttctaataacattaaacctcaatatcttgctcttccattcctgatgcctccctttccttctacccttcccctacctccttctttcctatgccacaggctggcaggttagtgccagagcaagtggccagtcaccatcattggggttgtggatcctcagggttcttcagaagccccttcaccatgatcaagagtctccagtcactcagaattccacggttcccaaatgccagctctcccactactcccagcgttctccatctctgggatgttgggctccaggcttctcagatgcactgagtaccctaggctaagccactgatccatcagaacttcatagcctgagaggagagggagacaggcttgcaaaggagagttctgactagacactggggtgctacagatgcccgtaagttgtccctttaccctcgatgtccccagtgttgggaccacctgggaatgcccagccttgtgtgctgattgacttgtagtcccctggccctgactggaagcctagttttctctctcatgaccagctaggcccctagctccccagggaagaaatccaatctatttcctctgatagtaatggctaatacttaaataatgccaaccacatgccaagcactttacagttgttagcccagtcttcacaagcaccttgtgaggtgggcaagagtcttatcttactctcattttatagatgtggcccaggatcccacagctatagttcatggtgctgggatttgaacctctggccaccagagcccaccttaatgtgtcctcctcctgttgtcataacagaaaagtacaacaccatgatgacacatcaggctatcctggcaggttcccaggctgccccaatgcccaactttctaggtttacaaagttgacatttacgaagtttccaggtttacaaatctagtttctgattctttagtcagcaggaatttctctacaaaagctgcttcgaaaatttccagccaaaccttacacaccttggcattacatcttggtgagccaaggcggaagagaacaggaagtgaaggccccatgggaagtccctgcggtcgggagcacccaggcggggcggggggtggggggctttcctgtggccggctccctgcccctcccacccccattcaggccctgtgagttgaatgaagagaccctgggaatgagtccaggtctgcagggttagaggaaattgaaggcccttaccagatccctgttgagaagtttatgaattatgagcccttctgcaaatgagagggttcttccctgtcaggagggacagattgtaggtggcaagattggtggcagccagtaggctggtctgctccttcctctctatttcatatgtgtatgaaggcattacctgcagcaagggcctgtgtaaatgcatgtgatttacagagcattttatgtactgcgtgtcattcatgcttccggtgagccctaagtctaagatagggcagatagcatcaggtccattttgcagctgtcaaaatgaggtctgaagggcagaagtggtgtgcccacacacacacaactggttggctgcagacctggggactagacccgggacttcgtcctgcccaggggtctcttgccactgctccccatcaacttggatggctttaagcatttgtgagttgtctgctccctgatggcagaatgcagagacatgaagctacaagcaggttcgctcccaacggcaaaaaggaggaggggtgttcagaacatcaggtgcttctagagaaagcagggagagagtatctggccttgtggacaatgtcacggcagaggccaggtatagggcatgggggtaactggaagcgggatggaccctgttattccctaagacatggcttccacgtagtgctcaaacaaggcctttgcccttgctgttccctccacctggaatattcttccccttccttgacattgctcaggtctccactcttatgtcaccctctcagagagggcttccctggccactttccctaaaatagccacccactcctaggtccctcaaaagcatatcctgctttggattttccctatagcaatatgccctatgaagttattttatttgctaacttgtttcttgtctgttttcctttgttagagcgttggggaccttgtctggcttgttcccaatgcctggaagagtgcctggcacacaggattaagccaacacatatgttttgaatgaatgtgtgcacacatgcatgagctggcggcagtcggggttggggtaagcacgaaggcccagctcagttctctgcatgtgacctcccatcttacgcagataagaaccagtttggtttctgctagcctgagtcaccctcctggaaactgggcctgcttggcatcaagtcagccatcagccggcccatctcctcatgctggccaaccctctgtgagtgtgtgggaggggaggctgggctcctccttgtactctctgaggtgctctggaaggaggggcagctccaccctgggagggactgtggcccaggtactgcccgggtgctactttatgggcagcagctcagttgagttagagtctggaagacctcagaagacctcctgtcctatgaggccctccccatggctttaggtaagctccttccactctcattttttcacctgagaaatgagagaggaaaatgtctacaattggtgtttatcaaatgctttcaggctctggtgagcaagcgtccaggaaaatgtcaagcgcatggagctccaggcctgtctgggggatctgggcacggggaggcatccatgggagaccatgcaggcactctgaggcaggggctgcaagcctagtgcctgctggggcagcaggtgaacagagaggtgtaactgctgtgacagaagtcatggagtccttggagtgtgagggtcattttccactgttgatagaatagggaaattggtgaaatagccctgttaaatgagagaaagaacagtgtgagctcaatgagaaatactaatagaatgtggcactgagccacaaggtctgaggcttgattgataaggaagggtggggactgtggagaattaagggcttggcacaggtcagttccaccagttgtcacaagagaatgcaggctcaggtggccagaacttctcgcttttccagaagagtccgatattctgatttcattatatatagtattctgattaaaccagacaataaagcaagcagataaaatatttaaagtataagctgccagtttgcaacctccggttaggatttgtgtggggcaaagaaaaaaactctcaggatcattggtatgtagactctaattttaagtttctaatttaaaattggcccctgaggctgggcgtggtggctcacacctgtaatcccagcattttgggaggccaaggtgggtggatctcttgaggtcaagagttcaaggcctgcctggccaacatggtgaaaccctgtctctattaaaaatacaaaaattagctgggcatggtggtgcatgtctgcaatcttagctacttgggtagctaaggcaggagaattgctggaacccgggaggtagaggttgcagtgaatggagatcacaccactgcactccagtctgggcaatagagagagacgctctctctaaaaaaaaatatgtaaagataaataaaatgaaataaaataggcctctaatgagcaggccattctcctttctgggtcttactttccttgcactcctttctgggtgttaagaggaggtctagaggaagctggacaactcttagcttgtagtaagcacagtggaagtatcagctcttaatgggtcatggacacgttacaagctaggcgccgtgctgagcactttacatggtttatcccactgaaccctctcaataaccctatgaggaagggctattattgctcacattttcagaagaggaaatggatatagagagattagataatttgcccatggccagacagctagtataagaggaggaggtggattgactgcagacattctgtcttcaaaccactacactatgctatggaggcacagagacttaatgaaatcatggagaggggaattgctttgtcaaccacaagcagttattccgggggcagcagatcctcccctgtcccccagtgggtacaatggtccctggtgggttgtgctacaatgttagcccatggtcttatgtgtttttcaaatgtgtaaagtaggatgctggaaccactcttagaaccagataccaatacattgtgaagaaataaatctctgtgcttaaaactggttcatcccaaaatattttgaactgacacacaataggtgctaaataaatgtgtgttaacttgaattggattgaattcgggaaaaaagtgcaataagcttagtgaagacaccatgttccctgggtagaggaaccacattctccatctaaggccaggagtatgggaggtatcaatgtttgcccagcacagaacagggtgccaagaagagaaaagttgacggggtgcatactctgactggaaactggaagggtgagaacagagggtaaaggatagagatggaaccatgtgcatacactttgtgttaccttggacaagtcattcatttctctggacctctgctttctctctacacaatggggtcccaccacttcccttacagctgacttgtatgaagaaggaggtggaggaggaggagaaggtgaagacaatgctgactcaaagggtaaattatttttaggatccaagtttgaaaacaattttaggctactagatatgaacaacatcttgattatgtagttgaaggaaattaaagatgaatggtttaattaaaaattaatcagaatgaaaacgattgattactaatatatctgcaatggtttattttcctgagtggcagactcactaaggtttttgaatactcctgtgtgattgctctatgtatgtatgtatgtatgtatgtatgcatgtatctatctatctgttgtctaataaaatggatcacatctctgctaataaaaacactacactggcagggtacaattataatcattaactgtgcctggaatttgcagcagcagccaccagaggtaccagtgccctttaagggttcataatttagaataatccaattatctgagtttttcagggactgaggggtttggcaaggtgtagaactttcagtaataaagtcaagaaagtcctggacaaaccaaggtagttggtcactctagtccataaccaggtaaagagctttccctgtaacctgtgtaaggttttagaatcatttctttccttattaccaaaaatcctccccaaattttcaagaaattatgaactaaatagttactctatgagataggagttcagcccaaaagaaacaccataagaacaaatataattcttgcttatgttaaccatgcaatgaagcagagagaaaaagtcagtggcctctttaggaggactgtagtgtgggaagaaataactaaactgggtttcaatcctggcctggccaggatctggagcaagtgagttaatctttctaagccttgagtagtttcttcttcttcttcttcttcttcctcccccttctcctcttcttcttcctcctccttctcctcttcttcttcttcttcttcttcctcttcttcttcttcctcctcctcctcctcctcttcttcttcttcctcttcctcttcctcttcctcttcttcctcttcctcttattcttcttcgtcgtcttcgtcttctttttattttcaaagtgaaagcaagtttattaagaaagtaaaggaataaaagaatggccactccatagacagagtagcctgaaccttgagttcttctataaagtcactatgaatttatactcattttgaaagtgggtgtcaatatgtctgtccactttgcacagctgttatgtggacaaaaggagatctgtgtgaaagtgtaacacagagcctaaactataacaggtaagcaacacagttgtccccttccccatggtgtctgttcttctccatttcctcctgtctgcagggggattataaaactaatcatcaaagccaagaaggcaagagcaagcatgtaccgctgaaaacacaagataactgcataagtaatgactttcagtgcagattcatagctaacccataaactgctggggcaaaaatcatcttggaaggctctgaacctcagaaaggattcacagtaagttaaccatgtagatctgagaggagagtagcttcttgtagataacagttggattatataccatgtcctgatccccttcatcatccaggagagcagaggtggtcaccctgatagcagcaagcctgggggctgcagcttggtgggtagaggtactcaggggtacagatgtctccaaacctgtcctgctgccttagggagcttctaataagttgatggatttggttaaaattaacttggctacttggcaggactgggtcagtgaggaccaacaaaaagaagacatcagattataccctgggggtttgtatttcttgtgtttctttctcttctttgtactaaaatatttacccatgactgggaaagagcaactggagtctttgtagcattatcttagcaaaaatttacaaagtttggaaaacaatattgcccatattgtgtggtgtgtcctgtgacactcaggattcaagtgttggccgaagccactaaatgtgagatgaagccattacaaggcagtgtgcacatctgtccacccaagctggatgccaacatttcacaaatagtgcttgcgtgacacaaatgcagttccaggaggcccaaatgaaaatgtttgtactgaaatttgttaaagcttcccgacaaactagatttatcagtaaggattgttttctgcaagggggatgaaacttgtggggtgagccatttgggctgaggaggagggaggttggagctgagaaatgtggagacaatttccctttagaaggactgaatctccctgcctctctggggtgcggcagccagcaggatccaatggtgtatatgtctccccagctccccattcagtgatatcatgtcagtagcttgaaattatccgtggtgggagtattatgtcatggaaattggcaaatggaaacttttattggagattcaattgttaaacttttaccagcacaacactgccctgccttcagagtcaatgaccctatccaagtttaatccatctgtccactgtctccaacacgatctttataaaacacacctgacaacattacccttttattcagttttttaaaagataagtttccagctcatcggggtggctttaaaggccatttctcctctggacctcacccaacttttcaaatcacttttcctacccctacctctaaatgctactcaaactccagccatcctgaataataagacttttgaaaagtagattatgggctgggcacagtggctcacacctgtaatcccagcactttgggaggccaagatgggtggatcacctgaggtcgggagttcgagaccagcctgactaacatagtgaaaccctgtctctactaaaaatacaaaattagttgggggtggtggcacaagcctgtaatcccagctactcaggaggttgaggcaggggaattgcttgaacctgggaggcggaggttgcggtgagcctagattgctccactgcactccagcctgggcaacaagagcgaaactccatctcaaaaaaataaataaataaataaagtagattacatcagatacctctggcctaggttgtttatgaccaactctcctgctgagaataactagaaaagctagacaaaacatatttccaaaagatctctttggaggcatcagagaatggccaaggctgtaaggaactgcctgagcccagagaggtggagcccagcactggtgccctttactcctggggacatgtgctggtttcaaaaacttcagctgagcttttgagcattcatggaacttggtgggggagatgaaatttgtaccttaaatcctgcctacagggagggtccctgataatccccacccaatttggaaatctgggtcagccttcacaggtactgaagccctcctctgaatgatctcaagtcctgctagggtagaggttacctgcttttgaaaggctcctggcctacctgtgcagcaggagcaaaagtgaaccatctcagggtacagataacaatcatccagagccttgaatgacctctactgtgcttaatatatagtattcagcagtcagtaaaaaggatttaggcacatgcaagatgacctgtgtatcagggagaaataggcaataaattgagatccagcagggatttgaatcatggatttgaatcaggggcagccttcgaaagaactatggagaatatactcagatttaaaacataagattggaatttttggcagagaactaacaactgtacaaaaaaggaaccaaatggaaatcctagaactgaaagatgcaattaaccgatgttgagaaatagccaacatctattgaacacttcccatgtggacagctgtgctaaacactttacaggcatcaacataagatgtgtccccttacagcagtgcagtgtccctcctaagacatggacagcctggtttccctatctctctgcttcatcaaaacccctttacgtggggcttagacactcctgttgtctctagtgtctagtagcacagggctcagcacatggaagccactagatacaatttgatgaccaggacctccgatgaaagccatgggtgctgattgggaaggcattgtcttttatgtgctatggtcttaaagcttcatccaggaagcagaactcggggggtgctgaggacccagaaccgagaataagattagtcagagatttcctgtgggcagaaatcataaggacgccaactgtttgggtgagataagacgaaaccaagagtggacttgtggccagaagcgtgaggaagagggagagagcttcccttgtcccctttcttcctctccctaagccacagtgattgacagccccccccctttggagtcagagcaggcttgagactggactgggaaaggagggtgggtcaggatacagagcaggaaggctgggagtgcagggcaggagcaaggggctggggcattcattgtgcctgatctctcccactttacctggggtaaagaagcatatgcaaaagccacggtgtgagtatttcccaagtgccagggtcagggcatgattcatcacgtgcagcatttcattcaatccttatagtaaccgatgatgtggcttctattattagctctatcagataatgaaactgagaccaagacaggctctgcacattgtgtggggtaatgacacagggggattcagacctagactccataactcctgccccagggaccacccccaccctcaccctgtgcatgtcgacaaaggacagactgggccacttctcaggacacagcggggaaatgacacagagcagggaggttccaggagccccgagcgtcttttctccaggagaatactctctgaattcagactggggtcagagaaacatttacccaggagccgcagtgtgggtggggctttttacttgaaacgctgtctgaaggcagtggccaggatggaactctccaccctaccttggcaagccacttctcttctgcaatctgtaaggacattgttgagagaattatggtcttccaattccggagggttgaagaaagacaaataggagagaacctatcatagtcaggtgctagctgccttctctttcagagagtgtgagaataaagtgatacacttgattattagcaaatactttggaaattttaaacgctaatattcaacacactctggaagaggcaaataagtagacaggttcatatacatcatctccttcagctagtcctcacaaaaacaaacaaatgaataaacaaaattcttctttggccctcataggaagacactgtttcttgaacgtgtttcaaaaaggatgggtgactcactcaaggtcacactgtttatgaggacagtacaggaatacagacatgccattttgcctgaaaaaatccatcacccagggaggtgacacaattttgcagaaatgttctatttcctctgaaggatacattctttaaacctttgggaaattcattcatagtcttcctcctttgaaggattaactctctggacacaaagtgtttgattctgatttgttggttggaagatgtgttggttgagagaaagattctgatttgttggttgaaaatagactcatcaagatcaactgctgtagtagtaaatattttgacattttgtctgtattcctgtgctgccctcacaagctgcatcaccttgagtgagtcattcatacttttttgtttgtttttgttttggagatggagtcttactctgttgcctaggctggagtgcggtggcgtgatcttggctcactgcgacctccatctcctgggttcaagtgatcctcctgcctcagcctcccgagtagctgggattacaggcacatgccaccatccctgctaatttttgcattttcagtagagacggagtttcaccatgttggtcaggttggtcttgaactcctgacctcaggtgatccgcccacctcagcctccccaagtgctgggattacaggtgtgagccaccgtgcccagcccagccatcatttttgaaacacgtttgagaaacagtgtcttcctttgagggccaaggagacattttttttgtttatttgtttgtttttgtgaggactagctgaagggggtgatgtatattaacctgcctacttatttgcctcttcccagagtgtgatgaatattagggtttaaagtttctgaagcatttgttaataaagcccggggctggaggtcagaagacctggatttctctgcatacttttgccatcagcaagctgtgtgaccttggacagatcccttttttgtctaaatctttctgagtcttcttgaaaacaatgccaggttgggacaggatgattgccaagctcccgtccagctctaaaacactgcaacgtatgcttctgcaccagcactgtccatcctgtagatcatgcagaaattctcttcaactttttcctacccataaaataggagcatgcttacctttttcctaatgttccaggccccgggtctagaatattgtaagtaaggaagttaatgtgtatcagagcccattatgggccagaagttctcctcttccttcctacacctgcttcctccctccctccctccctctttcccttccttccttccatccatttgtgaagaagacatgatcaccctcattctgagagtgaagagacagaggctcaactaatgaaatgatttgttcaaggtcacacgggtggcacaaggcaagtggcagaggttgaatttagacccattcctgtccaaatgctgagtttatgtcatcgtcccgagaccataactttaaagatgtaagatagtgggaaaagagttgatttcaaagcacctctcagaaggactcactttacatcaggggtcagcagactcaggccaaatccggtccattccccgcttttgcaaagaaagttgtagtggaacacagctaggcttattgatttatggattgccaacgtccttttgtgaaacagacagctgagctgagtaatcgtggcgcacaaaacctaaaatatttactatctcgtcctttacagaatgtttgccaatctatggtccggagtccaaggctgtccatttttcaaagaacacaaagtgacatgagactgtcccatgtgcagggagccctatcattttattatgaaaaaacggcctttctgctcaaatctgttttttaaaaagtcaacaaacagactctgggtacctgtcaggaacagtagggagtttggtttccattgtgctcttcttcccaggaactcaatgaaggggaaatagaaatcttaattttggggaaattgcacaggggaaaaaggggagggaatcagttacaacactccattgcgacacttagtggggttgaaagtgacaacagcaagggtttctctttttggaaatgcgaggagggtatttccgcttctcgcagtggggcagggtggcagacgcctagcttgggtgagtgactatttctttataaaccacaactctgggcccgcaatggcagtccactgccttgctgcagtcacagaatggaaatctgcagaggcctccgcagtcacctaatcactctcctcctcttcctgttccattcagagacgatctgccgaccctctgggagaaaatccagcaagatgcaagccttcaggtaaggctaccccaaggaggagaaggtgagggtggatcagctggagactggaaacatatcacagctgccaggggctgccaggccccagagggcctgagaactgggtttgggctggagaggatgtccattattcaagaaagaggctgttacatgcatgggcttcaggacttgtgtttcaaaatatcccagatgtggatagtgcgaccggagggctgtcttactttcccagagactcaggaacccagtgagtaatagatgcatgccaaggagtgggactgcgattcaggcctagttgaatgtgctgacagagaagcagagaggggcaccaggggcacagcccgaaggcccagactgatatgggcaaggcctgtctgtgctgacatgtcggagggtcccactctccagggaccttggtttccccgtctgtgacatctgtgacatgagagtcacgataactccttgtgtgccttacagggttgttgtgaaaattaaatgcacagataatagcgtaacagtattccgtgcattgtaaagagcctgaaaaccattatgatttgaaaatggaatcggctttgtgagaccatcactattgtaaagatgtgatgctgatagaaatgacaggactgcttgtgcatgccctctgcagtgtgacattccagcagtgaaatcatgttggggtgacttctcccccactctgacctttatgtttgtctgggccgaggctgcaagtcgggctctgtgggtgtatgagtgacaagtctctcccttccagatatggggactgtctgcttccctaggttgcctctccctgctctgatcagctagaagctccaggagatcctcctggaggccccagcaggtgatgtttatccctccagactgaggctaaatctagaaactaggataatcacaaacaggccaatgctgccatatgcaaagcactttggtttgcctggccacccctcgtcgagcatgtgggctcttcagagccacctgatgaggtgggtacagttagccacacttcacaggtgaagaggtgaggcacaggtcccaggtcaggctggccggagctctgtttattacgtctcacagctttgagtcctgctctcaaccagagaggccctttaccaagaagaaaggattgggacccagaatcaggtcactggctgaggtagagaggaagccgggttgttcccaagggtagctgctcctgcaggactctgagcaggtcaccagctaatggaggaaaggctctagggaaagacccttctggtctcagactcagagcgagttagctgcaaggtgttccgtctcttgaaacttctacctaggtgctatggtagccactagtctcaggtggctatttaaatttatacttaaatgaatgaaaatagaagaaaatttaaaatccagacccttggtcacactatccacatttaaagaggtcaatagccacatgtggttagtggccaccctattgggcagtgcagctacagaacatttttgcatcccagaaagttcttttggatgttgctgctctacagcatgctttgctgaaacagaagtgccttccctgggaatctcagatgggaagcaagtaaggaggggagtcaaatgtgggctcactgctcaccagctgtgagggttgggcctgcctcttaaccattgtcagcctcagtcttctcatccatgcatgccgtgggtatactaaaatactatacccctggaagagctggatgcaaatttgacaagttctgggggacacaggaaggtgccaagcacaaggctgggcacatggtggctgtgcactacagctgagtccttttccttttcagaatctgggatgttaacc

SEQ ID NO: 21 - protein, 177 aa, Homo sapiens
MEICRGLRSHLITLLLFLFHSETICRPSGRKSSKMQAFRIWDVNQKTFYLRNNQLVAGYLQGPNVNLEEKIDVVPIEPHALFLGIHGGKMCLSCVKSGDETRLQLEAVNITDLSENRKQDKRFAFIRSDSGPTTSFESAACPGWFLCTAMEADQPVSLTNMPDEGVMVTKFYFQEDE

SEQ ID NO: 22 - protein, 159 aa, Homo sapiens
MALETICRPSGRKSSKMQAFRIWDVNQKTFYLRNNQLVAGYLQGPNVNLEEKIDVVPIEPHALFLGIHGGKMCLSCVKSGDETRLQLEAVNITDLSENRKQDKRFAFIRSDSGPTTSFESAACPGWFLCTAMEADQPVSLTNMPDEGVMVTKFYFQEDE

SEQ ID NO: 23 - protein, 180 aa, Homo sapiens
MALADLYEEGGGGGGEGEDNADSKETICRPSGRKSSKMQAFRIWDVNQKTFYLRNNQLVAGYLQGPNVNLEEKIDVVPIEPHALFLGIHGGKMCLSCVKSGDETRLQLEAVNITDLSENRKQDKRFAFIRSDSGPTTSFESAACPGWFLCTAMEADQPVSLTNMPDEGVMVTKFYFQEDE

SEQ ID NO: 24 - protein, 143 aa, Homo sapiens
MQAFRIWDVNQKTFYLRNNQLVAGYLQGPNVNLEEKIDVVPIEPHALFLGIHGGKMCLSCVKSGDETRLQLEAVNITDLSENRKQDKRFAFIRSDSGPTTSFESAACPGWFLCTAMEADQPVSLTNMPDEGVMVTKFYFQEDE

SEQ ID NO: 25 - DNA, 3804 bp, Homo sapiens
taatttcagtgaaattatataacttggttacatttaggttacttattacaaatgaaaataaatatactaacagaagctgcctcatatgcaaatgagtaacatgttagagactaaaatacacaaaaaaatgcatgtgctttagctcatataaacaatatacaggacaacttaccgggtagcataaacaaccaacaacggactatcaaaaggaacctcgtcatctagtaactttaaccttgttggtagatctcctttttccatctccatatacacaggattggaacttgccatttctgaaatataaagcatatccttttccaaactttatctcttaggcggaaatattcaatttatgaacatgttcattcagcaatcattagtcacgtacctactgtgtggacctattatgtgcaaggcccaatattaagcattacaagagaaacaaataaaagtacaagagatgtaatttctacttttaagaaccttaaaatctaattgggaggcaaagcatattaaaagttttaaataagacgaaggaacatataattaatacatcagtgactattactcttaaaataatgagtatctaggcctatatatagcaactgtccatataagcacacatcaaaaaccaatatacatagctatcatcaatgccaagttgctcagttttttctagaactagtattcctactccatcttttagaattaaattcaatgaaattaattttaaaatatttgacctttttttaaagttaccagtatagcaaatactcattctctgaagaacagaagatttgactttttggaatagccaaaagtcacttaaaatcaagtctggtgaaaggagtgatgatctaaaactatttgtggtttaaaaaaaaaaagtatgaatctaaagtaaagtgggtttttttccaagtagttttcttttttagttttttagaaacagggtctcattctgttgcccaggctggagtgcagtggtgatcactgcaaccttgaactcctggctgtgtgtgtgtgtgtgtgtgtgtgcagcgacggggtcttcctacgttgcctagctgcagtgcctgtgtgcacacatgcgcacatgcgtgtgtggagagacagggtcttgctacgttgcctagctgcaatacctgggtgtgtgcatgtgtgtgtgtgtagagacaaggtcttgaaacgttgtctaggctggcatgtgtgtgtgtgtttatatgtatgtgtgtgtagacagggtcttgctacattgcataggctggtgtgtgtgtttttgtgtgtgtagagacggggtcttgctacgttgcctaagctgggcaagtatttttcaactgcctctgaagacaaatcccaaataacagttccaaaagctgtttcccataattatcacatcattagaagggtgaggcctactcaccaggttctaagagccaacattcattttctgatacatgcttttttaaaaaagtcattttttccccagtctcattgtttcccatttgactgtgtcaggcaataagtactttaaaggaattcagaggaggaggccattcagaggtttggggaagcctgatgactgcgcgggagctaaaccagacatatccacctaaattcaagtaagcagccatatcactcaaattgcccaccatgcttcctctagccagcactggtagtaacaactatcactctggctgatggagactcttttctgctcttctgtgactgggtatgatcacataatagagacagatacagtaaatttccaatgagtaataatgtcacacatttgaacttacctgaggagaaatagcttgtttcttatttcacacaaaagacaatctacctcaactcagaaaaaaaaaaattattatgcttttaactgctatatttgaattaaagcagatctgtaactatagatccatgtttctagaaagctaaaatatctttaagtaagatgacataaaaatgtatctctattcacttttggtaatgaatgaaaagttgcttaaagtctaaagtattagaaatatggcatctgttattcaagtaggatttggaattaagaaaattcacttcttcaaaaacatgggactatggctgcagaaagggcaatgcatatagtttttagggtatgatagctggtttctattatatgtcaggatgacatatgcgaccttccgccaaggtagatactgcgggctatgcaccaaagtctctgaggcagacatgtaagcgagctcttcacctatattcattcttttcctcctggacaggttacatttcccagtttcctttgcagttagttgtggctatatgacagaattctcatcaatggaaatgtacacagaagagaggtaagccactaccaggccaggcctataagacagcactttctacatgctttccccagacatagcaacccaaacatgaccacatcccttaagggaagatggagctgaaaataatggaaggaacttggaatgctagaatgctgaattaccacctgggagacagctacccactgacctggaatacctgtcctggactgttacatgagcaagaaatacacttctatttatgtatgagttacttcattatcagatatttattacagcagtttagctacctaagatctctctctgcctcagactgcttatctataaaatggaataacaccatctactccaaacattattgtaaggatgaaatgagacaatgctgaaaagtgtttaccataatatctgccacacaataagtaccccatatagtatttctgtattagtaagttacatgagagattttcttcttttaatacatctgcatttataaacattttactttaacctcaacttccccagcactgctctaccattttctgaatgtcattatgagagaaataaaactaatttctagggccaggcatggtggctcacacctataatcccagcattttgggaggccaaggtgggaagactgctttgaggtcaggatttcaagaccaacctgggcaacacagtaagaccccatctctataaaaaaatgaagaaatcagagggtacagtggcacatgcctgtaatcccacgactcagaaaactgaggcaggaggatcgcttgaacccaagggatcaaggctacagtgagccatgatcacaccactgcattccagcctgggcacagagtgagaccctgtctctaaaaataaaaaatagggccaggcacagtggttgatgcctgtgatcccaacactttgggaggccaaggcaggtagatcacttgaggtcaggcgtttgagaccagcttggccgacatggcaaaaccctgtctctactaaaatacaaaaattagctgggcgtggtggtgcacgcctgcagtcccagctacttgggaggctgaggcaagacaatcacttgaacccaggaggcggaggttgcagtgagccaagatggcgccactgcactcaaacagaatgaaactctgtctcaaaaaaaataaaataaataaaaatttaaaaactaatttcttataatccagttgtgaatttaaccaatgtctgaaagaactattaaaagttaaaatgaatggaaaacagaataaagggttgaccagaacagatgtgattttctacttaaatcttttttttaaaccccaaaattcaaaactgctaatgttttttaatacgaatttctatctttgataaggcaatctgagtattacctttcaatccttcaataaaagtatcccaaacagaagggctattactgtaactaagcttgatactctccttcgctcttttcaag

SEQ ID NO: 26 - DNA, 3804 bp, Homo sapiens
  misc_feature (2122)..(2131): n is a, c, g, or t
ggcttctggctctgagtgaggtcctgctgcaaggtttcctagatgagccactgagactctaataagatccagtggaaataaccaggctctcgtcggaatataagtcccaagggaagctgtgccagtcttgtgggcgactgcctgacttctcctttcatttcagcaccatgaagcttctcacgggcctggttttctgctccttggtcctgggtgtcagcagccgaagcttcttttcgttccttggcgaggcttttgatggtaaggcttcagaaggtttgcaggatttctgaagagaaacatcaccctggacctgataaactggggaaaatgatgctttcggaaggctgcttttgaaccacagagttgctagtgtctgcgttgctgaggcctgccaggaactagggtttgctgggttgcctgtctcgagtctttcagagctgctgggaatatcccctttccccgtagtgcagcttctcaggatgtgttaagtggatggatcacatttcagaagccgctgcaaggtgtatcaaaaacacatctcctgagccgtaagggacggggcatccagtaacaacgcacacggggtatttttgggcttccttaagatttgagccgctgccttaggttgtgctgcccaatgtgcctggggagctgctaaacagattagagagtcgaggattgttgtcagttactcagagaaagaacaatcatcctttccaggagcacctgagctgtttgttttgcgtagaagatgcaaaataaggcctgcaatgggtataaaatgtccctcagcataaatcgcataggagtatgactaaggctgttgactcttctgtcttctttctccttcctccttcgatttcctagttggataatgtacagggctctttagcctcgctctgtcaggggctcccttcctggtttgttctgtttccattcttccttctccagccttcttgacaagagctgggaactaacgtgcctcaagcccccacaaggaccacagcattttctcatttagtttcagaatgactctgtgacgcaatcttcctctcttggaaggtgagaaagctgatcttggaaggtgagaaagctgagacttagagcagctgaagccaatgcccagggacttactgccagtcagcaggtggcagggcagaggtttgagcccggctgtgcttgaggtcagggctcttgccaggtagacgcatcactgaccacctcctagaggttgatggttatgaatctcaggcacaccttggcatcacctgaaatacccatgccttcaactccccagcagagtctgcagaaactggcctggggtgtggcctgggcactgggactttcagtttctctctgggtgattagaaagtgcagccaaggctcacgcctgtaattccagcactttgggaggccaaggtggatgaatcacttgaggtcatgagttccggagcagcctggccaacatggtgaaaccccgtctctactaaaaatactaaaatgtagccaggcgtggtggcaggcacctgtaatcccagctactcaggaggctgaagcacgagaatcacttgaacccgagaagcagaggttgcagtgactagagatcgcaccagtgtcctccaacctgggtgacagagcgagactccatctaaaaaaaatgaaaaagaaagtgcagccaaggcagagcaccactgccctattgcttcctcaagcaacccacagcatcagtacagcctactaagaaagtatttagggacttttatgctcctaacagtcactggaactcacgtcacaatgacgtgtattccatttgcaagaatatatactttaggtcggggtgcggtggctcacgcctgtaatcccagcactttgggaggccaaggcagggggatcacgaggtcaggagttcgagaccagcctgaccaacatggtgaaatccccgtctctactaaaaatacaaaaattagccaggcgtgatggcgcatgcctgtaatctcagctactcaggaggctgaggcagaagaatctcttgaacctgggaggtggaggttgcgatgagctgagatagcaccactgcactccagcctgggcgacagagcaagactctgtctaaaaaaaaaannnnnnnnnnaaaaaaaaaaaaaaaaaaaaaaaaaaaaaaaagaatataaactttagtagtcagggcagaagtactctgtgtctgccacctttctcagcatcagtattccatgtcactacctcattcatacacactcctggatcttatcataggcagcttcattctatagcagtggctcttcaccagggcacttgaagaagccaactaggataaaggaatgtgcttctcaacccatggtatccaaggctgctatgatcacaggctgaaagcttgaagtcagtggaagatttgtccttcctcattcccctctaaggtgttgttggagtctttatgttctcctgatgtcccttctgcctttcctttcctttccaggggctcgggacatgtggagagcctactctgacatgagagaagccaattacatcggctcagacaaatacttccatgctcgggggaactatgatgctgccaaaaggggacctgggggtgcctgggctgcagaagtgatcaggtaactggagctcctgggacgttagggctgggtgagcagagcttgcctgccttggacagtcaggagggagacgagctccttgtggagaagttagaggctgcggcccctcctcctcttgccctctctctgcctctgtgctcagtgtgaggtctgagtggatggtaggagtgagtgattcctcatcctccctctctgggtgctgttcatccagcctaggggtgcccagcctggctgaatggggtggtgcccagtgttttcatccctccttccttggcctttctgggctcctctctgagccctcccttggaacagggagaatgggagggtgggctattgctcactggcctgattattaatctccttcttgcctgccttgattacagcgatgccagagagaatatccagagattctttggccatggtgcggaggactcgctggctgatcaggctgccaatgaatggggcaggagtggcaaagaccccaatcacttccgacctgctggcctgcctgagaaatactgagcttcctcttcactctgctctcaggagatctggctgtgaggccctcagggcagggatacaaagcggggagagggtacacaatgggtatctaataaatacttaagaggtggaatttgtggaaactgggtgttatactttgtggtatagactgcctgtttagtatgaaggggcgatccatgcacatctaagtgaacgtggaggctgggtgggtgggagacgactcctgggcacacagggcatcctgggcatccctgaggcaaggacatgatgagttcagtggccacccccacaggatcccaggggcttcagcagatcccaccccttaccccatgtgagcagctgcccagtgagtctgtaggaacccgagccacattcccagtgagttcaactgcaccccggcacgttttgctagcacctcaatggagagctccttgcttgcagctttggcttgtggcacccagcaaaagcttcctgccacccagtggctacagccacacactctccagcaagatttaatctcagccttgtgaggagccctttcccaaatttatttctttctgtgttttttatcccttagtagctaatctcatgttagccattaataactctctatgttaaacccttccttttgtatctgcggctacattga

SEQ ID NO: 27 - DNA, 3804 bp, Homo sapiens
gtataaatgcagaggtgcagtaactgggcttttcaggatatccagatggagttgtggtgttgttttgcttgtggtttttaacgttaacttttttttcccctttattttaagagaagcacaaaatgaacaaactagtgagcccagcaacatggatggaaattccggagatgcagactgctttcagccagcagtcaaaagggtatgggcaaaaaaatatgaaccatttggggctcaagtttctccaaatactttatgtgactgcaagtactgtatacgcttatttcctgtgactcagttcttctaactaagatgttaagcatttggcttaaagtgtatagcattacaaagagtatttccccagctttggcttgccagccaactttccattgactctagcctgttagccatttttattgttttttgtttgtttgtttgtttgttttcctcacatgtacacatacatacagattgttcttatatgtgattttgttctctgggaataaaatcttcattcaacagaggcaatatgacagaaaaaccgaagtttcatgtatatgatttttcaaagaaagtgaattggccctcatgttaaacctagcatttcagagctgaaagtgtcttctcattaaatattgaagaaatcatttgagggtgtggagaaggatggacagaattagctgcttgtgtatttattcttctcctgcaactttgccacgctattttgtacctcccttcctaattatgataaagctttcttagagagcagtcaggcaatgtgtattaaatgtttaaagctttacacccttagttctacttgtggacatttatttcttaagaaagatgtatactaagatttagatagaaatattcattacagtatcataataaagacagtagcaaggattctgttatctgtgttgcattaatacaatagagattgatgcaactgttcattattttgaaagcattaatgataatattgcatcaaagagttcactgaacagattgtacagtacagttttacacacaaaaaaaatagtttgtgagctttaaaagggccttcaaatgaatatgctaaacggttatctttcaataaagagagtatgggtaagtcttaatttctttcatttatttcagtaatttaatgtttttgttgttgttattgtttgtttttttgagacagagtcttgctctgtcacccaggctggagtgcagtggtgcaatctcagctcactgcaatctcggctcactgcaacgtctgcctcctggattcaagcaattcttctgcctcagcctccggagtagctgggattacaggcgtgcaccaccatacctagctaatttttgtatttttagtagagacggagttttgccatattggccaggctggtgttgaactcctggcctcatgtgatccgcccatctcagcctcccaaagtgctggggttacaggcatgagccactgtgccagcctatttcagtaacttaatgtttttacaggcatgtattacctataaaattaataaagccagtgaggtatttcttttttgaactaaagcaaagctaataataagttatagagaagttagagaagaaatctattaagtgatactttctttgtatactgttgggctgagtacccttgattcttggtggtgaacaagttatcagaaatttcttggccaggagccgtggctcacacctgtagtcccagcactttgggagtccaaggtgggtggatcacttgaggtcagaatttctagatcagcctggccagcatggtgaaaccctgtctctattaaaaatacagaaattagccaggcatggtgacgtgcgcctgtaattccagctacctgggaggctgaggcagcaaaatcacttgaacctggcaggcggagttcgcagtgagctgggatcgcgtcgctgcactccagcctggatgacagagcaagactccatctcaaagaaaaaataaaaaagaaatttatttacttgtgtgaatttttacaatacagatgcttctcgacttaaatggggctacatcccaataaactcataagttgcaaatactgtaaatcaaaaatgcattgaatacacctaatgtatggaacaccatagtttagcctatcctactttaaatgtgttccgaacacttagattagcctgtagttgggcagcattacctactataaagtgtattttctaataaaatgttgaatatctcatgtaactcattgaatactgaaagtgaaaaacaatgtatgggtactcaaaatatggtttctctactgaatgtgaatcactttgacaccatcataaagttgaaaaattccaagtcaaaccattgtaagtcaggggctatcagtattcagtggtaaatgctggctctaactattcttccaagtcagtggttgactgctgtttattctataaagggttacaatttatagattctctcacttgtagaatgagagattcagaattaatagcagacagagtccctaccttgatggagctttcatttaagtgtgaaagtcaggtgacctaacaaggccttggcataagtttaggatttggattgttatgggagcttgggtagggacatgtcataggtaaggcaacagcaggggtagagataagcttgacatatgtcaaaaatcatgaagacatcagtaatccttgaagttggctgaaaggtatagagttgagaaagtagttaaaaaaaaaaaagtcaggctgagtctaggtaaggatgtgtttctctgaggtcagatttgttcctgtaccataaagggactatttagaatcttaaagctggagcaatttaaaacgttaagttttcagattgaggtcagatttgtgacttcatgtgaggtcagatttgttcctgtaccataaagggactatttagaatcttaaagctggagcaatttaaaacgttaagttttcagattgacgttttttgaggtatagttaataacctgaatgttctgattctagtcttggtagtcaataagagttgaccagatgaatttcatagctttgtagaggatgaaatatttcaaggctgatttgcacaaatgtttacatagatcatgtatctttcataagtaatatgtttgtattattacaaggctgtaaaaatttaagcaggttgttaatagcacagggggtaacagattaataaaattaatgaataaaattactaaaagagtccagaagtaaacccaaatacgtggaggaattaagcatatgtatgatacacatgacattttaaaaatcagtgggaaaaggtaaattattttacaaatggtgttagaagcactgattgataattttgttaaaagaaacttagattccctattttactcctaatccaaaataaattctgagtggatctaagattaagcaaaaattaagccggaagctgagcatggtagcatgtgtctgtaatctccgcaatttaggagactgagtttggctggggaggtggtgatatgcgcctagaaaaaaaaaattttttaagccacagatgtataagcaaaaagcgggcaaagaggcggaatttttttttttttttttgatgaagtctcacttgtcgcccaggctggaacgcagtggcgtgatctcagctcactgcaacctctgcctcccgggttcaagcgattctcctgcctcagcctcccaagtagctgggattacaggcacctgccgaggagaggatttttttataattaaaacaaaacaaaacaaaaaaacaccaaactggaagataaagtatttacaacatgtaaaagactgttt

SEQ ID NO: 28 - protein, 662 aa, Homo sapiens
MVVSEVDIAKADPAAASHPLLLNGDATVAQKNPGSVAENNLCSQYEEKVRPCIDLIDSLRALGVEQDLALPAIAVIGDQSSGKSSVLEALSGVALPRGSGIVTRCPLVLKLKKLVNEDKWRGKVSYQDYEIEISDASEVEKEINKAQNAIAGEGMGISHELITLEISSRDVPDLTLIDLPGITRVAVGNQPADIGYKIKTLIKKYIQRQETISLVVVPSNVDIATTEALSMAQEVDPEGDRTIGILTKPDLVDKGTEDKVVDVVRNLVFHLKKGYMIVKCRGQQEIQDQLSLSEALQREKIFFENHPYFRDLLEEGKATVPCLAEKLTSELITHICKSLPLLENQIKETHQRITEELQKYGVDIPEDENEKMFFLIDKVNAFNQDITALMQGEETVGEEDIRLFTRLRHEFHKWSTIIENNFQEGHKILSRKIQKFENQYRGRELPGFVNYRTFETIVKQQIKALEEPAVDMLHTVTDMVRLAFTDVSIKNFEEFFNLHRTAKSKIEDIRAEQEREGEKLIRLHFQMEQIVYCQDQVYRGALQKVREKELEEEKKKKSWDFGAFQSSSATDSSMEEIFQHLMAYHQEASKRISSHIPLIIQFFMLQTYGQQLQKAMLQLLQDKDTYSWLLKERSDTSDKRKFLKERLARLTQARRRLAQFPG

SEQ ID NO: 29 - protein, 662 aa, Homo sapiens; identical to SEQ ID NO: 28

SEQ ID NO: 30 - protein, 508 aa, Homo sapiens
MVVSEVDIAKADPAAASHPLLLNGDATVAQKNPGSVAENNLCSQYEEKVRPCIDLIDSLRALGVEQDLALPAIAVIGDQSSGKSSVLEALSGVALPRGSGIVTRCPLVLKLKKLVNEDKWRGKVSYQDYEIEISDASEVEKEINKAQNAIAGEGMGISHELITLEISSRDVPDLTLIDLPGITRVAVGNQPADIGYKIKTLIKKYIQRQETISLVVVPSNVDIATTEALSMAQEVDPEGDRTIGILTKPDLVDKGTEDKVVDVVRNLVFHLKKGYMIVKCRGQQEIQDQLSLSEALQREKIFFENHPYFRDLLEEGKATVPCLAEKLTSELITHICKSLPLLENQIKETHQRITEELQKYGVDIPEDENEKMFFLIDKVNAFNQDITALMQGEETVGEEDIRLFTRLRHEFHKWSTIIENNFQEGGQQAHLQPHPFDHPVLHAPDVRPAASEGHAAAPAGQGHLQLAPEGAERHQRQAEVPEGAACTADAGSAPACPVPRLTTLCPAP

SEQ ID NO: 31 - DNA, 5687 bp, Homo sapiens
ctctctggttgcccttaacattttttccttcatttcaactttggtgggtctgatgattatgtgtcttggggttgctcttctcgaggagtatcttagtagtattctctgtatttcctgaatttgaatgttggcctgtctttctaggttggggaagttctcctggataatatcctgaagagtatttttcaacttggttctattctccttgttactttcaggtacaccaatcaaacgtagatttggtcttgtcacatagtcccatatttcttggaggttttattcgttcctttttattcttttttctctagttttgtcttctcgctttatttcactaagttgatcttcaatctctgatatccttgcttctgcttgattgattcagctatcccccgctcgatattacaaaccatgtcacgaggcgtggacaccccccatgatatggggagtattatcacccccctcttcccccactggatattacaaaccatgtcatagggaggtggacatcccccacaatatgaggagtaatatcacacccctttccccgcagtggatattatgaaccatgtcacaggcggttaaacacccccaacgatatggggagtaatatcacactcctctcccccctggatattacgaaccatgtcatggggggtggacaccctttgcaatatggggagtaaaatcacccccctctcccccaactggatattatgaaccatgtcacagtgggggaaaaatcctctgtgatatgcagagtaatatcaccccactctcaccacctggatattacgaaccatgtcacaggggggtggacaccccccaagatgggggagtaatatcacctcactctctgccaccagatattacaaactgtgtcacaggggggtgaacaacccccacaatatggggagcactatcacccccctcccccagggtattatgatccatgtcacaggggggtggataccacccactatatggggagtaatatcacctttctctcccgccctggtttttatgaaccgtgtcacaggggggtggacaccccttgcgatatggggagtaatatcacccccctctccaccatctggatattacgaaccatgtcacaggggggtggacacccctgcgatatggggaggaatatgcccctctccccacctggatattacaaatcatgtcacgggggacggacatcccccacaatatggggagtaatatcaccacactctcccctgctggatattacgaaccatatcacaggcggctggagacacaaggcattaacaatatttcgagtaatattatctttccctttgaacattatgaacaatatgacagaggggtgtacacctcctgcgatattgggagtaatgtcatcccctcccccactggatattaggaaccatattactgggggatgtattcccccttctagattgggaggaagatcatacttgccctccctgaatatttgaaacaatatcataggggtttgtacacttttacgatattgggagtaatatcatcctttctccccctggaaattaggaacaatatcacaggggtggtgtacacccctgcaatatttagggtaatattattgtcttctcccctcgatattaggaacaatattacaaggacggtgtaaagtacctgccaaattgggaaaaatactatcctctccctcttgtatattagaaacaataacacagggggaatgtacacccactgccatattgggagtaatatcatactcgccccatcccccagatattaggaacaatatcacagcaggggtgtacacttttacgatattgggagtaatatcatactctctccccctggaaattaggaataatatcacagagatggtgtagaccctctgcaatacttaggataatattatcatctcccccctcgatattaggaacaatattacggggagtgtaaattacctgccaaattggaggtaatcctctcctctctctccctgtattttagaaaatataacacacaggaaatgtacaacactgcgatattcggagtaatatcttcttctccccacctggatattaggaacaataacacggacggggcgtacacccctcgcgatattgaatgtaatgtcatcctctccctccctttatattacgaacaatatcacaggggggtgtacaacccctgcaatattggaagtagtatcatccattctcccatgaatattaggaacaatatcacaggggtagagtacaccctctgcaatttcgggagtaacatcatcctctcgttccctggatattataaacaacaccacgggggggtgggggtgtacacacccttcgatattgggagtaatataatcctttccctccctatatattagaagcaatatcacaggggttggtgtaaacttcttgcgatatggggattaatatcacccccctctcctgccctggatattatgaaccatatcacagggaggtggacacactttgcgatatggggagtaatatcacgcccctctcccccccgatattacgaaccatatcacaagggagtggaccccccccacgatatggggagtaatatcacccccctctcccgccctggatattacgaaccatatcacagggggatggacaccccccgcgatgcggggagtaatgtcacccccttctgccccctaggatattacgaaccatatcatggacaccctccacgatattggaaataatatcatcctctcccccttggatattaggaacaatatcacagggggttgtacacctcctatgatattggaagtaatatcatcctctccctcctggatattagcaacaatatcacagggagtgtgtacaaccccagcgatatttggagtaatatcaccctctcaccccatggatatgagaaacaatatcacaggggaggtgtacatcccacgtgatattgtgtgtaatatcattcttccccaacccctgcaatattgtggtgtaatataattctctcccttcctggacattatgaacaatatcactactaggtgatacattaggagtaatgtatccataggatattatgaggaatatcacagggtgtacacccactgtgatattagaggtaatatctccctaaaatattaagaagaatatcttacacccactgtgactttagaagtaatatctccctaaaacgttacaaataacatcgcagggtgtacactcacagtgatattaggagtaatatctccctagaatattacaaatacacatggtgtaaacccactgtgactttagaagaactatctccctaaaataatacaaaaatatcgcagtgtataccataatatcccctagaatatcataaataatatcacagggtgtacacccactgtgataataggaataataccaccccaggatattatgaataatgtcacaggctgtacacccactatgacattaggagtaatatctccctaggacactatgaataacatcacagattttacacccatggtgtgcacccactatgatattaggagtaatatctgcacaggatataacaaataatagtacagggtgtacacatatgatatacacccactgtgatattaggagaaatatatccctaggatattatgaataacctctcagagtacacacacatggtatacaccctctgtggcattaggaacaataactttctaaaacattacgaataacatcacagaatgtacacacatggtttacacccactgtgacaggtgcaatatctcccttggatattatgaataacaacaaactatcactgtcatattaggagtaatttctccctagaatattacaaataacatcacagggtgttcatttatggtgcacacccactgtgatattaggagtaatatctccctaggatattacttttcatataaaagtgtgtacatccactgtgatattgggaaaaatatttctctaggatattatgaataatatcacagagcgtacacccactgtgatattaggagtaataattccctgggttattatgaataatatcacaggatgtacaaccactgtgatattaggagcaatatcttcctaggatattacaaataatatcacagggtgtacacccactgtgatattaaagtaatttttaggttattgtgaataatatcaccaagtgtacaaacatggtgtacactcactgtgatatcaggagtaatatctcagtaaaatattatgaataatatcacagggtatacacccactgtgatattagcagtagtatctttgtaggatattacaaataatatcacagggtgtatgcccactatgacattagaagcaatatctccctaggatatcaaaaataatatcacagggtgtacaacttctacatcccaggttctaagggattctcctgcttcagcctcctgagtggctgggattacagatgcccaccaccacacctggctaatttcgtattttcagtagagatggggtatcaccatgctggtcaggctggtctggaacttctgacctcaggtgatccaccagcctcggccttccaaagtgctgggaatacaggtgtgagccaacgtgcttggcagagagttatatattaaataaatctggaaacatagctcccatgtttgagtgtgcatttacttttatgaagaaattatgtcagaaaacctaaggatgataataaatatgaaaagtaactggcatgtaaaaaggtcttttgattaagaactataaggttcgatttcatttttagataacgtgatcctagctcttgtatagtgcttataaatattctacatcaaaggaatttgttgcacagtgtcagaataaaataaagtgtatttcactgcttcttaatttttaaattagactgagtttgttttcctagagagagaagaacattttttattttttctgaaaagagtaggccatattttactgagatcttagatttgttatatattaggttttggtcttctaacattctccagtggattttctctaaagtaggtatgcacagaaagagttgaatagcaaaaaagtaaatcatgtaataattctgagatttttgggtttgtcacaactgagaaatattgctgagggtgtatggtcctcaagtgtgaaaatgttccttgtgaattgcttgtatccgaaatatacacacaacattaagtcctggtttttatcttttattttttccaatccttttttcttctcaaggtgtccaagtcacacagagccacagaatctcacaggtgtctcagaattcctcctcctgggactctcagaggatccagaactgcagccactccttgctgggctgttcctatccatgtgcctggtcacgatgctggggaacctgctcatcatcctggccgtcagccctgactcccacctccacatccccatgtacttcttcctctccaacctgtccttgcctgacattggtttcaccttggccacggtccccaagatgattgtagacatgcaatcacatagcagagtcatctcccatgcaggctgtctgacacagatacctttctttgtcctttttgtatgtatagatgacatgctcctgactgtgatggcctatgactgatttgtggccatctgtcaccccctgcactacccagtcatcatgaatcctca

SEQ ID NO: 32 - DNA, 5687 bp, Homo sapiens
attgaattttatctcagagcccacatgaagcaggatcaaagtcagtacacatgaaaactagagcccaaagactataaagcatgaaataaggatttaagctaaccctatcttgtaaggggtttgtaaagcccagcttgcatctgagctacactagcaccaggacagccactcagtaatggggtttctcaaggttattgcttttcattcagttgaaatgagagtcatttcttacccttatgccctgtgagatttcactggaggttgttcactgaaacattttcatatcattgcatcaaccctcttgaactcactgtgcctgcccccagttcagtctgtgactcacaagtaccctgcagcaaaagaaatccaatagagggcaaatccctcaccttaccttcctttctaagacctttgatgttctcatgtgtcatttcataattgggattgtcaattagtcgcctcatctctggtcctcactttcctctctcccagccaaactcaaccttcagcccacacaatggaattcaacaaaatgaggtaacagttttctgtgtgagtcactctgggcaactctgttcacagagcactgtgaggtgagcagccagaacccaggcaagtgtttcagccatccaagaactggcaggcagcccaagagacactctcacctgatgacagactagcaggatgagtcctggaggaaatggttcccaacagctgcagaaggagtctcttggctcatgcacagcaatgctcttctcaattaaaaacgttgtcattattgacactgcagtgtaaaatccttttacactgtgctcacatttctacaggccttcacctgctctgcccattaaagacaagacccttccatgagatgatgacatctctaagttactgttccacccaaacagtcctatataatgaagagaaaaattttgctggccctcaaaaggcaaacacaaggagaaagatttccacaagctgtttctctttgctgagcacttagaggaaaactgtaagtggttggaagaaggctttgttttctacaagacttttagttattcctcagaaattttcctgcttattcccagaggaggtcatctcttagatgctgtcagtcagatagggattggcagccaagcagaggtgctcagagaggtttccaactaatgtggccagcggaaaactgccaaagaagcagggatccttaggacaaataaactggaagatattttggggataaaaataaatccttttgaaaatgaaagatggagagatgctgtatatacaaattgccctgttctgaacaatgttgtcactaggactggccctggagaccaatgatacaaaccaaaatgttctcagacatgctttgatggtctttttctccaaagttatctattctgtttccatttcattctcacaggacttgccatggggttctcataagatttcacattggtcataatccaggtggccctggactgcaacctctgagttggcaacatcagaataggaattacgaaaaaccaatttaaagttaaatacagacacaggcaaaagagagatgggttgtcgaagctagtgcctaggtggacactgcctcacatttttaattccagaagccatcagtactgagtgtcagatctcattagtcaaacacagtgatcaggaatcctgttttcctggaggatttccttgagggagggaccactcaagagtctgaaatatttcacgtcatagagtatggatctcaccccaacacccaatcagaaaatagggagaactggaaaccaaaattccccctcccgctgtggaaggatgaaaaccagagtgttggagttctgtcctgataatggagcagacagctaggcagcaatcaatgagggccagtacaggaattcagtgctaagtattgggtcataacagaagtagggaaggtattaatccagtgctatatgaggatcctgggacactggctcctagtaatctagttataactattagcaaaaaagaaaaaaaaaatcagtgatgtgaagagatggcctaaaggagctccagcaatatagctaagcagctggcaagtggtctgaggagcattgcaattccaggcctcctaaggtggcagtacgggcactggtaagacattctgctgtggtgaaactagtttaccatagaggattcacaattaaaataggcaaacaggaaatgcaagacagaggctaacaaagggttttttttttggtgggggggagttgtttgtttgtttgtttgttttctgagacggagtcttcctctgttgcccaggctggaatgcagtggcacgatctcagctcactacaacctctgcctcccaggttcaagcagttcttctgcctcagcctcccaggttcaagcagttcttctgcctcagcctcccaagtacctgggactatagctgtgtgccaccacattgactaatttttgtacttttagtacagactgggtttcaccatgttggccaggctggtgtcgaactcctgacctcaagtaatccccccgccttggcctcccaaagtgctggaattacaggcatgagccaccacacctggccagtttttggtaattcttaaagaactcaatgagcaacactcaaacaaccataaagactatagagctcatggttgaattttagatagctaaacagacaggagtttttgtaagttttgtaagtcttgctcatccttccctcttccatcctctatctcaactattctgtctaccattaaagcaccttagaccttgagtttggcaatgcaacaagtgtgtgctcaacacgaaataggtaattcaatagcaaagccctaaaacagcctggcttgattatttctcagggcatgcagttcctttgaagcaggatcattttaataataataataatagaaataataatagaaattgaagacaattatttcacaatttccatacacctaagagctatacatatgaatgataatgcataattgtaaagcatgcatattacaggtaataaatatgttagctaattataaacaatgcccattttcatatagtttatccttgccaaataaaactgtaaaaaaaagacacctttcaaatgctgctaaggagtaatacctgaatgaggttgatttaatggagtcttagttcctgcatgtgttctaattgaatagactatgtagtaattcccttacatacccatccatgtccaagaacagtgaagatctttatttaatatgaattattgcagatgattagcacagtctagccaaaccattccagtaattgtttttacttgttatattaatatataaattctcaaaggatataacagtgatgttgggtgaatttcactgaatgatagctcaaacacctgaaatattgactaagaaaactaatttatcaatactgataatcaattttaatatgttaattgattgtaatacaggattctgtggttcaaaaaaaaagaacaagcaaaaaaactttcttccatttccaaataccaattaatagatctctacttccccttggatttcttcttaccacctaccacctccaatcttcattctttcctcacaaactaaacataaaagttacctacaaagcatagaatctgtgttaaaggatattcttgcttgttttaagtccaaaattaaacagctctgaattattaaaaagcacatgaattcaaatgtcctattctaataagaaaatggtttacatttctctatgttcaaggaaaaaaatagtcaagggtgtacaagtggggtaaaaattatttccagtaggttatgtgatttaagttatagaaacgaaccaggcaattcaattaaatgtcatggaaagtaggttttttcttttcctctttttttctaatatgtacactttgtgagaagataaatccatagtgtgataatttgtccactgggtccatcagacactggagacagcttcctaagaattataaggcttctaaaggcttctaaagcctaaattgcctagagcattttgtgtgccaggcactttgctaggtgccctagggatgcaagaagtataaatgttttatgagaatacaggctggaaatgtattcttgattattcctgtggaatttctaggcagaaaagagtctaatggggtataggtatattttctcaacacaattttctgagcctttaccagatgcagttctatggtttgaatgtgtccctcagagtttgtgtgttggaaacttaatccccaatgcaataatgttggtgaggcctaatgaaagcctaataatgtaggtgaggcctaatgagagctgtttagaccatgaaggctcttccctcatggatggattaatgctgttatggtgggaatgggttcattattactggggtgggttcataataaaaagatgagtttggcctgctattctctctctttctcatcctctcttccaccatgggatgacacagcaagaaggcccctgcaagatgccctcccctcagtattggacttcacagcctccaggaccataagccaataaatttttgttcattataaatttcccagtctgtggtattctgttatagcaacactcaatttatgcattacttccagattcttatggctatacctacttctcacagtttgtattcacccctccttcaaccaagtacccttaacacagttcccatagtcacaaagccaggtcactgaagctgccctctctccaaccacacacatatagatcaaatgaccccagacatagagctgattgagaaggagggaccagtacgagctctgcttccccagcagcttcctggaaagaagaggcaatacaacccaacccaaaagtgcaagagaagtaacacctcatgggatgagcttaattaatcaatgggagaggacactagaagacactagaggatctcccttcctccctttctttcccacttcaccccctccagtctctgaaccatgagctatttcaaaggtgcagtaatgctatatttggcttctctgaagatatcctatgaggccaagtcatcagctttgttcattatctaagagtggtggccagctcaccagcacttcccatcatgtttgccctccctctttcccttgtgttacttcccattttcccttacttctgctttcttggcattaaattctactctgcaatgttaggatataagtttttgcctcagattctgttttctaggaaacccatgctaagacaacactggcagtggccctggaaaagtaaacctcatgatggatttggagttggattgttcactgatctgaaggacagaggactccacttaagtggtaagcagtgtagctatgaactctgccacgcaggcctcacaattactgaggcttcttttacctgtggttaactgggacacagaacagcaggaaattgagtgtagaggttatcaagtagctgcttcacttaattggtataattttatggagttaacctggtttagagtccagagaacattccacatagcctagaaagggtagttatttgtccttaccataatcaagtcatactttgaatatgagttttccttccctgttcagcaccacttctcttagacttaagaatgcctgatctgttgatattatgtcccatgtaacattgcctgagacaaagatatccatgtaccttaaa

SEQ ID NO: 33 - protein, 140 aa, Homo sapiens
MGFQKFSPFLALSILVLLQAGSLHAAPFRSALESSPADPATLSEDEARLLLAALVQDYVQMKASELEQEQEREGSSLDSPRSKRCGNLSTCMLGTYTQDFNKFHTFPQTAIGVGAPGKKRDMSSDLERDHRPHVSMPQNA

SEQ ID NO: 34 - protein, 128 aa, Homo sapiens
MGFQKFSPFLALSILVLLQAGSLHAAPFRSALESSPADPATLSEDEARLLLAALVQDYVQMKASELEQEQEREGSRIIAQKRACDTATCVTHRLAGLLSRSGGVVKNNFVPTNVGSKAFGRRRRDLQA

SEQ ID NO: 35 - protein, 141 aa, Homo sapiens
MGFQKFSPFLALSILVLLQAGSLHAAPFRSALESSPADPATLSEDEARLLLAALVQDYVQMKASELEQEQEREGSSLDSPRSKRCGNLSTCMLGTYTQDFNKFHTFPQTAIGVGAPGKKRDMSSDLERDHRPHVSMPQNAN

SEQ ID NO: 36 - protein, 116 aa, Homo sapiens
APFRSALESSPADPATLSEDEARLLLAALVQDYVQMKASELEQEQEREGSSLDSPRSKRCGNLSTCMLGTYTQDFNKFHTFPQTAIGVGAPGKKRDMSSDLERDHRPHVSMPQNAN

SEQ ID NO: 37 - protein, 187 aa, Homo sapiens
TSEETISTVQEKQQNISPLVRERGPQRVAAHITGTRGRSNTLSSPNSKNEKALGRKINSWESSRSGHSFLSNLHLRNGELVIHEKGFYYIYSQTYFRFQEEIKENTKNDKQMVQYIYKYTSYPDPILLMKSARNSCWSKDAEYGLYSIYQGGIFELKENDRIFVSVTNEHLIDMDHEASFFGAFLVG

SEQ ID NO: 38 - protein, 168 aa, Homo sapiens
VRERGPQRVAAHITGTRGRSNTLSSPNSKNEKALGRKINSWESSRSGHSFLSNLHLRNGELVIHEKGFYYIYSQTYFRFQEEIKENTKNDKQMVQYIYKYTSYPDPILLMKSARNSCWSKDAEYGLYSIYQGGIFELKENDRIFVSVTNEHLIDMDHEASFFGAFLVG

SEQ ID NO: 39 - protein, 662 aa, Homo sapiens; identical to SEQ ID NO: 28

SEQ ID NO: 40 - DNA, 3444 bp, Artificial Sequence
  An exemplary cDNA sequence of human MX1
cgagcagaaatgaaaccgaaactgaattgtccgggaaattcgcggtgggggcggagagcgcagggagaagtaagcccagtgcaggatcctgaggcccgtgtttgcaggaccagggccggccttccgattccccattcattccagaagcaccgaaccacgctgtgcccggatcccaagtgcagcggcacccagcgtgggcctggggttgccggttgacccggtcctcagcctggtagcagaggccaggccagtgccacaaggcacctaagtccacctgggcctggagcaggacaggttgcaaaagaaaatatctcgggacccccaaactccttatgctaagggaaacatcgagcctgggaactgagccatcaacgctgccattctttttcccaaacagaaccctgttgtcagaggtacacccagagcaactccacaccgggtgcatgccacagcaactccatcttaaataggagctggtaaaacgaggctgatacctactgggctgcattcccagacggcatagcgaggaggtgctgaagagcgcaggtttggagaatgatcacctggattggaaccatagctctaccaatatggaacccagctccttaggcctcggtcttctcatggagaacatggtgtgataatcctactcctctgggagggtggctgttaagccttggaccgcagttgccggccaggaatcccagtgtcacggtggacacgcctccctcgcgcccttgccgcccacctgctcacccagctcaggggctttggaattctgtggccacactgcgaggagatcggttctgggtcggaggctacaggaagactcccactccctgaaatctggagtgaagaacgccgccatccagccaccattccaaggaggtgcaggagaacagctctgtgataccatttaacttgttgacattacttttatttgaaggaacgtatattagagcttactttgcaaagaaggaagatggttgtttccgaagtggacatcgcaaaagctgatccagctgctgcatcccaccctctattactgaatggagatgctactgtggcccagaaaaatccaggctcggtggctgagaacaacctgtgcagccagtatgaggagaaggtgcgcccctgcatcgacctcattgactccctgcgggctctaggtgtggagcaggacctggccctgccagccatcgccgtcatcggggaccagagctcgggcaagagctccgtgttggaggcactgtcaggagttgcccttcccagaggcagcgggatcgtgaccagatgcccgctggtgctgaaactgaagaaacttgtgaacgaagataagtggagaggcaaggtcagttaccaggactacgagattgagatttcggatgcttcagaggtagaaaaggaaattaataaagcccagaatgccatcgccggggaaggaatgggaatcagtcatgagctaatcaccctggagatcagctcccgagatgtcccggatctgactctaatagaccttcctggcataaccagagtggctgtgggcaatcagcctgctgacattgggtataagatcaagacactcatcaagaagtacatccagaggcaggagacaatcagcctggtggtggtccccagtaatgtggacatcgccaccacagaggctctcagcatggcccaggaggtggaccccgagggagacaggaccatcggaatcttgacgaagcctgatctggtggacaaaggaactgaagacaaggttgtggacgtggtgcggaacctcgtgttccacctgaagaagggttacatgattgtcaagtgccggggccagcaggagatccaggaccagctgagcctgtccgaagccctgcagagagagaagatcttctttgagaaccacccatatttcagggatctgctggaggaaggaaaggccacggttccctgcctggcagaaaaacttaccagcgagctcatcacacatatctgtaaatctctgcccctgttagaaaatcaaatcaaggagactcaccagagaataacagaggagctacaaaagtatggtgtcgacataccggaagacgaaaatgaaaaaatgttcttcctgatagataaagttaatgcctttaatcaggacatcactgctctcatgcaaggagaggaaactgtaggggaggaagacattcggctgtttaccagactccgacacgagttccacaaatggagtacaataattgaaaacaattttcaagaaggccataaaattttgagtagaaaaatccagaaatttgaaaatcagtatcgtggtagagagctgccaggctttgtgaattacaggacatttgagacaatcgtgaaacagcaaatcaaggcactggaagagccggctgtggatatgctacacaccgtgacggatatggtccggcttgctttcacagatgtttcgataaaaaattttgaagagttttttaacctccacagaaccgccaagtccaaaattgaagacattagagcagaacaagagagagaaggtgagaagctgatccgcctccacttccagatggaacagattgtctactgccaggaccaggtatacaggggtgcattgcagaaggtcagagagaaggagctggaagaagaaaagaagaagaaatcctgggattttggggctttccagtccagctcggcaacagactcttccatggaggagatctttcagcacctgatggcctatcaccaggaggccagcaagcgcatctccagccacatccctttgatcatccagttcttcatgctccagacgtacggccagcagcttcagaaggccatgctgcagctcctgcaggacaaggacacctacagctggctcctgaaggagcggagcgacaccagcgacaagcggaagttcctgaaggagcggcttgcacggctgacgcaggctcggcgccggcttgcccagttccccggttaaccacactctgtccagccccgtagacgtgcacgcacactgtctgcccccgttcccgggtagccactggactgacgacttgagtgctcagtagtcagactggatagtccgtctctgcttatccgttagccgtggtgatttagcaggaagctgtgagagcagtttggtttctagcatgaagacagagccccaccctcagatgcacatgagctggcgggattgaaggatgctgtcttcgtactgggaaagggattttcagccctcagaatcgctccaccttgcagctctccccttctctgtattcctagaaactgacacatgctgaacatcacagcttatttcctcatttttataatgtcccttcacaaacccagtgttttaggagcatgagtgccgtgtgtgtgcgtcctgtcggagccctgtctcctctctctgtaataaactcatttctagcagacaaaaaaaaaaaaaaaaaa

SEQ ID NO: 41 - protein, 715 aa, Artificial Sequence
  An exemplary amino acid sequences of human MX2
MSKAHKPWPYRRRSQFSSRKYLKKEMNSFQQQPPPFGTVPPQMMFPPNWQGAEKDAAFLAKDFNFLTLNNQPPPGNRSQPRAMGPENNLYSQYEQKVRPCIDLIDSLRALGVEQDLALPAIAVIGDQSSGKSSVLEALSGVALPRGSGIVTRCPLVLKLKKQPCEAWAGRISYRNTELELQDPGQVEKEIHKAQNVMAGNGRGISHELISLEITSPEVPDLTIIDLPGITRVAVDNQPRDIGLQIKALIKKYIQRQQTINLVVVPCNVDIATTEALSMAHEVDPEGDRTIGILTKPDLMDRGTEKSVMNVVRNLTYPLKKGYMIVKCRGQQEITNRLSLAEATKKEITFFQTHPYFRVLLEEGSATVPRLAERLTTELIMHIQKSLPLLEGQIRESHQKATEELRRCGADIPSQEADKMFFLIEKIKMFNQDIEKLVEGEEVVRENETRLYNKIREDFKNWVGILATNTQKVKNIIHEEVEKYEKQYRGKELLGFVNYKTFEIIVHQYIQQLVEPALSMLQKAMEIIQQAFINVAKKHFGEFFNLNQTVQSTIEDIKVKHTAKAENMIQLQFRMEQMVFCQDQIYSVVLKKVREEIFNPLGTPSQNMKLNSHFPSNESSVSSFTEIGIHLNAYFLETSKRLANQIPFIIQYFMLRENGDSLQKAMMQILQEKNRYSWLLQEQSETATKRRILKERIYRLTQARHALCQFSSKEIH

SEQ ID NO: 42 - DNA, 2961 bp, Artificial Sequence
  An exemplary cDNA sequence of human MX2
aagagatgatttctccatcctgaacgtgcagcgagcttgtcaggaagatcggaggtgccaagtagcagagaaagcatcccccagctctgacagggagacagcacatgtctaaggcccacaagccttggccctaccggaggagaagtcaattttcttctcgaaaatacctgaaaaaagaaatgaattccttccagcaacagccaccgccattcggcacagtgccaccacaaatgatgtttcctccaaactggcagggggcagagaaggacgctgctttcctcgccaaggacttcaactttctcactttgaacaatcagccaccaccaggaaacaggagccaaccaagggcaatggggcccgagaacaacctgtacagccagtacgagcagaaggtgcgcccctgcattgacctcatcgactccctgcgggctctgggtgtggagcaggacctggccctgccagccatcgccgtcatcggggaccagagctcgggcaagagctctgtgctggaggcactgtcaggagtcgcgcttcccagaggcagcggaatcgtaaccaggtgtccgctggtgctgaaactgaaaaagcagccctgtgaggcatgggccggaaggatcagctaccggaacaccgagctagagcttcaggaccctggccaggtggagaaagagatacacaaagcccagaacgtcatggccgggaatggccggggcatcagccatgagctcatcagcctggagatcacctcccctgaggttccagacctgaccatcattgaccttcccggcatcaccagggtggctgtggacaaccagccccgagacatcggactgcagatcaaggctctcatcaagaagtacatccagaggcagcagacgatcaacttggtggtggttccctgtaacgtggacattgccaccacggaggcgctgagcatggcccatgaggtggacccggaaggggacaggaccatcggtatcctgaccaaaccagatctaatggacaggggcactgagaaaagcgtcatgaatgtggtgcggaacctcacgtaccccctcaagaagggctacatgattgtgaagtgccggggccagcaggagatcacaaacaggctgagcttggcagaggcaaccaagaaagaaattacattctttcaaacacatccatatttcagagttctcctggaggaggggtcagccacggttccccgactggcagaaagacttaccactgaactcatcatgcatatccaaaaatcgctcccgttgttagaaggacaaataagggagagccaccagaaggcgaccgaggagctgcggcgttgcggggctgacatccccagccaggaggccgacaagatgttctttctaattgagaaaatcaagatgtttaatcaggacatcgaaaagttagtagaaggagaagaagttgtaagggagaatgagacccgtttatacaacaaaatcagagaggattttaaaaactgggtaggcatacttgcaactaatacccaaaaagttaaaaatattatccacgaagaagttgaaaaatatgaaaagcagtatcgaggcaaggagcttctgggatttgtcaactacaagacatttgagatcatcgtgcatcagtacatccagcagctggtggagcccgcccttagcatgctccagaaagccatggaaattatccagcaagctttcattaacgtggccaaaaaacattttggcgaatttttcaaccttaaccaaactgttcagagcacgattgaagacataaaagtgaaacacacagcaaaggcagaaaacatgatccaacttcagttcagaatggagcagatggttttttgtcaagatcagatttacagtgttgttctgaagaaagtccgagaagagatttttaaccctctggggacgccttcacagaatatgaagttgaactctcattttcccagtaatgagtcttcggtttcctcctttactgaaataggcatccacctgaatgcctacttcttggaaaccagcaaacgtctcgccaaccagatcccatttataattcagtattttatgctccgagagaatggtgactccttgcagaaagccatgatgcagatactacaggaaaaaaatcgctattcctggctgcttcaagagcagagtgagaccgctaccaagagaagaatccttaaggagagaatttaccggctcactcaggcgcgacacgcactctgtcaattctccagcaaagagatccactgaagggcggcgatgcctgtggttgttttcttgtgcgtactcattcattctaaggggagtcggtgcaggatgccgcttctgctttggggccaaactcttctgtcactatcagtgtccatctctactgtactccctcagcatcagagcatgcatcaggggtccacacaggctcagctctctccaccacccagctcttccctgaccttcacgaagggatggctctccagtccttgggtcccgtagcacacagttacagtgtcctaagatactgctatcattcttcgctaatttgtatttgtattcccttccccctacaagattatgagaccccagagggggaaggtctgggtcaaattcttcttttgtatgtccagtctcctgcacagcacctgcagcattgtaactgcttaataaatgacatctcactgaacgaatgagtgctgtgtaagtgatggagatacctgaggctattgctcaagcccaggccttggacatttagtgactgttagccggtccctttcagatccagtggccatgccccctgcttcccatggttcactgtcattgtgtttcccagcctctccactcccccgccagaaaggagcctgagtgattctcttttcttcttgtttccctgattatgatgagcttccattgttctgttaagtcttgaagaggaatttaataaagcaaagaaactttttaaaaacgt